European Patent Application EP 4 681 734 A2, published January 21, 2026. Title: EXPRESSION OF NOVEL CELL TAGS. Applicant: PRECIGEN, INC. Application EP Not yet assigned, filed June 6, 2018. The sequence listing filed with the application follows.

SEQUENCE LISTING (240 sequences)

SEQ ID NO: 1 - DNA, 66 bp, unidentified
  misc_feature 1..66: note = Description of Unknown: GMCSFR alpha signal sequence
  source 1..66: mol_type = genomic DNA
atgcttctcctggtgacaagccttctgctctgtgagttaccacacccagcattcctcctgatccca

SEQ ID NO: 2 - protein, 22 aa, unidentified
  REGION 1..22: note = Description of Unknown: GMCSFR alpha signal sequence
MLLLVTSLLLCELPHPAFLLIP

SEQ ID NO: 3 - DNA, 60 bp, unidentified
  misc_feature 1..60: note = Description of Unknown: Ig Kappa signal sequence
  source 1..60: mol_type = genomic DNA
atgaggctccctgctcagctcctggggctgctaatgctctgggtcccaggatccagtggg

SEQ ID NO: 4 - protein, 20 aa, unidentified
  REGION 1..20: note = Description of Unknown: Ig Kappa signal sequence
MRLPAQLLGLLMLWVPGSSG

SEQ ID NO: 5 - DNA, 54 bp, unidentified
  misc_feature 1..54: note = Description of Unknown: Immunoglobulin E signal sequence
  source 1..54: mol_type = genomic DNA
atggattggacctggattctgtttctggtggccgctgccacaagagtgcacagc

SEQ ID NO: 6 - protein, 18 aa, unidentified
  REGION 1..18: note = Description of Unknown: Immunoglobulin E signal sequence
MDWTWILFLVAAATRVHS

SEQ ID NO: 7 - DNA, 63 bp, unidentified
  misc_feature 1..63: note = Description of Unknown: CD8-alpha signal sequence
  source 1..63: mol_type = genomic DNA
atggcgctgcccgtgaccgccttgctcctgccgctggccttgctgctccacgccgccaggccg

SEQ ID NO: 8 - protein, 21 aa, unidentified
  REGION 1..21: note = Description of Unknown: CD8-alpha signal sequence
MALPVTALLLPLALLLHAARP

SEQ ID NO: 9 - DNA, 63 bp, unidentified
  misc_feature 1..63: note = Description of Unknown: TVB2(T21A) signal sequence
  source 1..63: mol_type = genomic DNA
atgggcaccagcctcctctgctggatggccctgtgtctcctgggggcagatcacgcagatgct

SEQ ID NO: 10 - protein, 21 aa, unidentified
  REGION 1..21: note = Description of Unknown: TVB2(T21A) signal sequence
MGTSLLCWMALCLLGADHADA

SEQ ID NO: 11 - DNA, 72 bp, unidentified
  misc_feature 1..72: note = Description of Unknown: CD52 signal sequence
  source 1..72: mol_type = genomic DNA
atgaagcgcttcctcttcctcctactcaccatcagcctcctggttatggtacagatacaaactggactctca

SEQ ID NO: 12 - protein, 24 aa, unidentified
  REGION 1..24: note = Description of Unknown: CD52 signal sequence
MKRFLFLLLTISLLVMVQIQTGLS

SEQ ID NO: 13 - DNA, 84 bp, unidentified
  misc_feature 1..84: note = Description of Unknown: Low-affinity nerve growth factor receptor (LNGFR, TNFRSF16) signal sequence
  source 1..84: mol_type = genomic DNA
atgggggcaggtgccaccggccgcgccatggacgggccgcgcctgctgctgttgctgcttctgggggtgtcccttggaggtgcc

SEQ ID NO: 14 - protein, 28 aa, unidentified
  REGION 1..28: note = Description of Unknown: Low-affinity nerve growth factor receptor (LNGFR, TNFRSF16) signal sequence
MGAGATGRAMDGPRLLLLLLLGVSLGGA

SEQ ID NO: 15-16 - skipped (2 entries)

SEQ ID NO: 17 - DNA, 12 bp, synthetic construct
  misc_feature 1..12: note = Description of Artificial Sequence: Synthetic oligonucleotide
  source 1..12: mol_type = other DNA
agtggcagcggc

SEQ ID NO: 18 - protein, 4 aa, synthetic construct
  REGION 1..4: note = Description of Artificial Sequence: Synthetic peptide
SGSG

SEQ ID NO: 19 - DNA, 45 bp, synthetic construct
  misc_feature 1..45: note = Description of Artificial Sequence: Synthetic oligonucleotide
  source 1..45: mol_type = other DNA
ggcggaggcggaagcggaggcggaggctccggcggaggcggaagc

SEQ ID NO: 20 - protein, 15 aa, synthetic construct
  REGION 1..15: note = Description of Artificial Sequence: Synthetic peptide
GGGGSGGGGSGGGGS

SEQ ID NO: 21 - DNA, 60 bp, synthetic construct
  misc_feature 1..60: note = Description of Artificial Sequence: Synthetic oligonucleotide
  source 1..60: mol_type = other DNA
ggtggcggtggctcgggcggtggtgggtcgggtggcggcggatctggtggcggtggctcg

SEQ ID NO: 22 - protein, 20 aa, synthetic construct
  REGION 1..20: note = Description of Artificial Sequence: Synthetic peptide
GGGGSGGGGSGGGGSGGGGS

SEQ ID NO: 23 - DNA, 54 bp, synthetic construct
  misc_feature 1..54: note = Description of Artificial Sequence: Synthetic oligonucleotide
  source 1..54: mol_type = other DNA
ggcagcacctccggcagcggcaagcctggcagcggcgagggcagcaccaagggc

SEQ ID NO: 24 - protein, 18 aa, synthetic construct
  REGION 1..18: note = Description of Artificial Sequence: Synthetic peptide
GSTSGSGKPGSGEGSTKG

SEQ ID NO: 25 - DNA, 78 bp, unidentified
  misc_feature 1..78: note = Description of Unknown: Glycophorin A (E91-R116) sequence
  source 1..78: mol_type = genomic DNA
gagataacactcattatttttggggtgatggctggtgttattggaacgatcctcttaatttcttacggtattcgccga

SEQ ID NO: 26 - protein, 26 aa, unidentified
  REGION 1..26: note = Description of Unknown: Glycophorin A (E91-R116) sequence
EITLIIFGVMAGVIGTILLISYGIRR

SEQ ID NO: 27 - DNA, 69 bp, unidentified
  misc_feature 1..69: note = Description of Unknown: Glycophorin A (I92-I114) sequence
  source 1..69: mol_type = genomic DNA
ataacactcattatttttggggtgatggctggtgttattggaacgatcctcttaatttcttacggtatt

SEQ ID NO: 28 - protein, 23 aa, unidentified
  REGION 1..23: note = Description of Unknown: Glycophorin A (I92-I114) sequence
ITLIIFGVMAGVIGTILLISYGI

SEQ ID NO: 29 - DNA, 69 bp, synthetic construct
  misc_feature 1..69: note = Description of Artificial Sequence: Synthetic oligonucleotide
  source 1..69: mol_type = other DNA
ataacactcattatttttggggtgatggctggtgttattggaacgatcctcttagccctgctcatctgg

SEQ ID NO: 30 - protein, 23 aa, synthetic construct
  REGION 1..23: note = Description of Artificial Sequence: Synthetic peptide
ITLIIFGVMAGVIGTILLALLIW

SEQ ID NO: 31 - DNA, 63 bp, unidentified
  misc_feature 1..63: note = Description of Unknown: CD3 zeta (CD247) transmembrane domain sequence
  source 1..63: mol_type = genomic DNA
ctctgctacctgctggatggaatcctcttcatctatggtgtcattctcactgccttgttcctg

SEQ ID NO: 32 - protein, 21 aa, unidentified
  REGION 1..21: note = Description of Unknown: CD3 zeta (CD247) transmembrane domain sequence
LCYLLDGILFIYGVILTALFL

SEQ ID NO: 33 - DNA, 84 bp, unidentified
  misc_feature 1..84: note = Description of Unknown: CD8-alpha transmembrane domain sequence
  source 1..84: mol_type = genomic DNA
atctacatctgggcccctctggccggcacctgtggcgtgctgctgctgagcctggtcatcaccctgtactgcaaccaccggaat

SEQ ID NO: 34 - protein, 28 aa, unidentified
  REGION 1..28: note = Description of Unknown: CD8-alpha transmembrane domain sequence
IYIWAPLAGTCGVLLLSLVITLYCNHRN

SEQ ID NO: 35 - DNA, 81 bp, unidentified
  misc_feature 1..81: note = Description of Unknown: CD28 transmembrane domain sequence
  source 1..81: mol_type = genomic DNA
ttttgggtgctggtggtggttggtggagtcctggcttgctatagcttgctagtaacagtggcctttattattttctgggtg

SEQ ID NO: 36 - protein, 27 aa, unidentified
  REGION 1..27: note = Description of Unknown: CD28 transmembrane domain sequence
FWVLVVVGGVLACYSLLVTVAFIIFWV

SEQ ID NO: 37 - DNA, 63 bp, unidentified
  misc_feature 1..63: note = Description of Unknown: Cytotoxic T-lymphocyte protein 4 transmembrane domain sequence
  source 1..63: mol_type = genomic DNA
ttcctcctctggatccttgcagcagttagttcggggttgtttttttatagctttctcctcaca

SEQ ID NO: 38 - protein, 21 aa, unidentified
  REGION 1..21: note = Description of Unknown: Cytotoxic T-lymphocyte protein 4 transmembrane domain sequence
FLLWILAAVSSGLFFYSFLLT

SEQ ID NO: 39 - DNA, 66 bp, unidentified
  misc_feature 1..66: note = Description of Unknown: Low-affinity nerve growth factor receptor (LNGFR, TNFRSF16) transmembrane domain sequence
  source 1..66: mol_type = genomic DNA
ctcatccctgtctattgctccatcctggctgctgtggttgtgggccttgtggcctacatagccttc

SEQ ID NO: 40 - protein, 22 aa, unidentified
  REGION 1..22: note = Description of Unknown: Low-affinity nerve growth factor receptor (LNGFR, TNFRSF16) transmembrane domain sequence
LIPVYCSILAAVVVGLVAYIAF

SEQ ID NO: 41 - DNA, 57 bp, synthetic construct
  misc_feature 1..57: note = Description of Artificial Sequence: Synthetic oligonucleotide
  source 1..57: mol_type = other DNA
gcaacgaacttctctctcctaaaacaggctggtgatgtggaggagaatcctggtcca

SEQ ID NO: 42 - protein, 19 aa, synthetic construct
  REGION 1..19: note = Description of Artificial Sequence: Synthetic peptide
ATNFSLLKQAGDVEENPGP

SEQ ID NO: 43 - DNA, 60 bp, synthetic construct
  misc_feature 1..60: note = Description of Artificial Sequence: Synthetic oligonucleotide
  source 1..60: mol_type = other DNA
cagtgtactaattatgctctcttgaaattggctggagatgttgagagcaaccctggacct

SEQ ID NO: 44 - protein, 20 aa, synthetic construct
  REGION 1..20: note = Description of Artificial Sequence: Synthetic peptide
QCTNYALLKLAGDVESNPGP

SEQ ID NO: 45 - DNA, 54 bp, synthetic construct
  misc_feature 1..54: note = Description of Artificial Sequence: Synthetic oligonucleotide
  source 1..54: mol_type = other DNA
gagggcagaggaagtctgctaacatgcggtgacgtcgaggagaatcctggacct

SEQ ID NO: 46 - protein, 18 aa, synthetic construct
  REGION 1..18: note = Description of Artificial Sequence: Synthetic peptide
EGRGSLLTCGDVEENPGP

SEQ ID NO: 47 - DNA, 66 bp, synthetic construct
  misc_feature 1..66: note = Description of Artificial Sequence: Synthetic oligonucleotide
  source 1..66: mol_type = other DNA
gtcaaacagaccctaaactttgatctgctaaaactggccggggatgtggaaagtaatcccggcccc

SEQ ID NO: 48 - protein, 22 aa, synthetic construct
  REGION 1..22: note = Description of Artificial Sequence: Synthetic peptide
VKQTLNFDLLKLAGDVESNPGP

SEQ ID NO: 49 - DNA, 570 bp, Encephalomyocarditis virus
  source 1..570: mol_type = genomic DNA
ccccctctccctcccccccccctaacgttactggccgaagccgcttggaataaggccggtgtgcgtttgtctatatgttattttccaccatattgccgtcttttggcaatgtgagggcccggaaacctggccctgtcttcttgacgagcattcctaggggtctttcccctctcgccaaaggaatgcaaggtctgttgaatgtcgtgaaggaagcagttcctctggaagcttcttgaagacaaacaacgtctgtagcgaccctttgcaggcagcggaaccccccacctggcgacaggtgcctctgcggccaaaagccacgtgtataagatacacctgcaaaggcggcacaaccccagtgccacgttgtgagttggatagttgtggaaagagtcaaatggctctcctcaagcgtattcaacaaggggctgaaggatgcccagaaggtaccccattgtatgggatctgatctggggcctcggtgcacatgctttacatgtgtttagtcgaggttaaaaaacgtctaggccccccgaaccacggggacgtggttttcctttgaaaaacacgatc

SEQ ID NO: 50 - protein, 1210 aa, unidentified [sequence omitted]

SEQ ID NO: 51 - protein, 1255 aa, unidentified [sequence omitted]

SEQ ID NO: 52 - protein, 1342 aa, unidentified
  REGION 1..1342: note = Description of Unknown: Receptor tyrosine-protein kinase ErbB3 (HER3) isoform 1 precursor sequence
MRANDALQVLGLLFSLARGSEVGNSQAVCPGTLNGLSVTGDAENQYQTLYKLYERCEVVMGNLEIVLTGHNADLSFLQWIREVTGYVLVAMNEFSTLPLPNLRVVRGTQVYDGKFAIFVMLNYNTNSSHALRQLRLTQLTEILSGGVYIEKNDKLCHMDTIDWRDIVRDRDAEIVVKDNGRSCPPCHEVCKGRCWGPGSEDCQTLTKTICAPQCNGHCFGPNPNQCCHDECAGGCSGPQDTDCFACRHFNDSGACVPRCPQPLVYNKLTFQLEPNPHTKYQYGGVCVASCPHNFVVDQTSCVRACPPDKMEVDKNGLKMCEPCGGLCPKACEGTGSGSRFQTVDSSNIDGFVNCTKILGNLDFLITGLNGDPWHKIPALDPEKLNVFRTVREITGYLNIQSWPPHMHNFSVFSNLTTIGGRSLYNRGFSLLIMKNLNVTSLGFRSLKEISAGRIYISANRQLCYHHSLNWTKVLRGPTEERLDIKHNRPRRDCVAEGKVCDPLCSSGGCWGPGPGQCLSCRNYSRGGVCVTHCNFLNGEPREFAHEAECFSCHPECQPMEGTATCNGSGSDTCAQCAHFRDGPHCVSSCPHGVLGAKGPIYKYPDVQNECRPCHENCTQGCKGPELQDCLGQTLVLIGKTHLTMALTVIAGLVVIFMMLGGTFLYWRGRRIQNKRAMRRYLERGESIEPLDPSEKANKVLARIFKETELRKLKVLGSGVFGTVHKGVWIPEGESIKIPVCIKVIEDKSGRQSFQAVTDHMLAIGSLDHAHIVRLLGLCPGSSLQLVTQYLPLGSLLDHVRQHRGALGPQLLLNWGVQIAKGMYYLEEHGMVHRNLAARNVLLKSPSQVQVADFGVADLLPPDDKQLLYSEAKTPIKWMALESIHFGKYTHQSDVWSYGVTVWELMTFGAEPYAGLRLAEVPDLLEKGERLAQPQICTIDVYMVMVKCWMIDENIRPTFKELANEFTRMARDPPRYLVIKRESGPGIAPGPEPHGLTNKKLEEVELEPELDLDLDLEAEEDNLATTTLGSALSLPVGTLNRPRGSQSLLSPSSGYMPMNQGNLGESCQESAVSGSSERCPRPVSLHPMPRGCLASESSEGHVTGSEAELQEKVSMCRSRSRSRSPRPRGDSAYHSQRHSLLTPVTPLSPPGLEEEDVNGYVMPDTHLKGTPSSREGTLSSVGLSSVLGTEEEDEDEEYEYMNRRRRHSPPHPPRPSSLEELGYEYMDVGSDLSASLGSTQSCPLHPVPIMPTAGTTPDEDYEYMNRQRDGGGPGGDYAAMGACPASEQGYEEMRAFQGPGHQAPHVHYARLKTLRSLEATDSAFDNPDYWHSRLFPKANAQRT

SEQ ID NO: 53 - protein, 1308 aa, unidentified
  REGION 1..1308: note = Description of Unknown: Receptor tyrosine-protein kinase ErbB4 (HER4) isoform JM-a/CVT-1 precursor sequence
MKPATGLWVWVSLLVAAGTVQPSDSQSVCAGTENKLSSLSDLEQQYRALRKYYENCEVVMGNLEITSIEHNRDLSFLRSVREVTGYVLVALNQFRYLPLENLRIIRGTKLYEDRYALAIFLNYRKDGNFGLQELGLKNLTEILNGGVYVDQNKFLCYADTIHWQDIVRNPWPSNLTLVSTNGSSGCGRCHKSCTGRCWGPTENHCQTLTRTVCAEQCDGRCYGPYVSDCCHRECAGGCSGPKDTDCFACMNFNDSGACVTQCPQTFVYNPTTFQLEHNFNAKYTYGAFCVKKCPHNFVVDSSSCVRACPSSKMEVEENGIKMCKPCTDICPKACDGIGTGSLMSAQTVDSSNIDKFINCTKINGNLIFLVTGIHGDPYNAIEAIDPEKLNVFRTVREITGFLNIQSWPPNMTDFSVFSNLVTIGGRVLYSGLSLLILKQQGITSLQFQSLKEISAGNIYITDNSNLCYYHTINWTTLFSTINQRIVIRDNRKAENCTAEGMVCNHLCSSDGCWGPGPDQCLSCRRFSRGRICIESCNLYDGEFREFENGSICVECDPQCEKMEDGLLTCHGPGPDNCTKCSHFKDGPNCVEKCPDGLQGANSFIFKYADPDRECHPCHPNCTQGCNGPTSHDCIYYPWTGHSTLPQHARTPLIAAGVIGGLFILVIVGLTFAVYVRRKSIKKKRALRRFLETELVEPLTPSGTAPNQAQLRILKETELKRVKVLGSGAFGTVYKGIWVPEGETVKIPVAIKILNETTGPKANVEFMDEALIMASMDHPHLVRLLGVCLSPTIQLVTQLMPHGCLLEYVHEHKDNIGSQLLLNWCVQIAKGMMYLEERRLVHRDLAARNVLVKSPNHVKITDFGLARLLEGDEKEYNADGGKMPIKWMALECIHYRKFTHQSDVWSYGVTIWELMTFGGKPYDGIPTREIPDLLEKGERLPQPPICTIDVYMVMVKCWMIDADSRPKFKELAAEFSRMARDPQRYLVIQGDDRMKLPSPNDSKFFQNLLDEEDLEDMMDAEEYLVPQAFNIPPPIYTSRARIDSNRSEIGHSPPPAYTPMSGNQFVYRDGGFAAEQGVSVPYRAPTSTIPEAPVAQGATAEIFDDSCCNGTLRKPVAPHVQEDSSTQRYSADPTVFAPERSPRGELDEEGYMTPMRDKPKQEYLNPVEENPFVSRRKNGDLQALDNPEYHNASNGPPKAEDEYVNEPLYLNTFANTLGKAEYLKNNILSMPEKAKKAFDNPDYWNHSLPPRSTLQHPDYLQEYSTKYFYKQNGRIRPIVAENPEYLSEFSLKPGTVLPPPPYRHRNTVV

SEQ ID NO: 54 - protein, 1298 aa, unidentified
  REGION 1..1298: note = Description of Unknown: Receptor tyrosine-protein kinase ErbB4 (HER4) isoform JM-b (isoform X7) precursor sequence
MKPATGLWVWVSLLVAAGTVQPSDSQSVCAGTENKLSSLSDLEQQYRALRKYYENCEVVMGNLEITSIEHNRDLSFLRSVREVTGYVLVALNQFRYLPLENLRIIRGTKLYEDRYALAIFLNYRKDGNFGLQELGLKNLTEILNGGVYVDQNKFLCYADTIHWQDIVRNPWPSNLTLVSTNGSSGCGRCHKSCTGRCWGPTENHCQTLTRTVCAEQCDGRCYGPYVSDCCHRECAGGCSGPKDTDCFACMNFNDSGACVTQCPQTFVYNPTTFQLEHNFNAKYTYGAFCVKKCPHNFVVDSSSCVRACPSSKMEVEENGIKMCKPCTDICPKACDGIGTGSLMSAQTVDSSNIDKFINCTKINGNLIFLVTGIHGDPYNAIEAIDPEKLNVFRTVREITGFLNIQSWPPNMTDFSVFSNLVTIGGRVLYSGLSLLILKQQGITSLQFQSLKEISAGNIYITDNSNLCYYHTINWTTLFSTINQRIVIRDNRKAENCTAEGMVCNHLCSSDGCWGPGPDQCLSCRRFSRGRICIESCNLYDGEFREFENGSICVECDPQCEKMEDGLLTCHGPGPDNCTKCSHFKDGPNCVEKCPDGLQGANSFIFKYADPDRECHPCHPNCTQGCIGSSIEDCIGLMDRTPLIAAGVIGGLFILVIVGLTFAVYVRRKSIKKKRALRRFLETELVEPLTPSGTAPNQAQLRILKETELKRVKVLGSGAFGTVYKGIWVPEGETVKIPVAIKILNETTGPKANVEFMDEALIMASMDHPHLVRLLGVCLSPTIQLVTQLMPHGCLLEYVHEHKDNIGSQLLLNWCVQIAKGMMYLEERRLVHRDLAARNVLVKSPNHVKITDFGLARLLEGDEKEYNADGGKMPIKWMALECIHYRKFTHQSDVWSYGVTIWELMTFGGKPYDGIPTREIPDLLEKGERLPQPPICTIDVYMVMVKCWMIDADSRPKFKELAAEFSRMARDPQRYLVIQGDDRMKLPSPNDSKFFQNLLDEEDLEDMMDAEEYLVPQAFNIPPPIYTSRARIDSNRSEIGHSPPPAYTPMSGNQFVYRDGGFAAEQGVSVPYRAPTSTIPEAPVAQGATAEIFDDSCCNGTLRKPVAPHVQEDSSTQRYSADPTVFAPERSPRGELDEEGYMTPMRDKPKQEYLNPVEENPFVSRRKNGDLQALDNPEYHNASNGPPKAEDEYVNEPLYLNTFANTLGKAEYLKNNILSMPEKAKKAFDNPDYWNHSLPPRSTLQHPDYLQEYSTKYFYKQNGRIRPIVAENPEYLSEFSLKPGTVLPPPPYRHRNTVV

SEQ ID NO: 55 - protein, 335 aa, synthetic construct
  REGION 1..335: note = Description of Artificial Sequence: Synthetic polypeptide
RKVCNGIGIGEFKDSLSINATNIKHFKNCTSISGDLHILPVAFRGDSFTHTPPLDPQELDILKTVKEITGFLLIQAWPENRTDLHAFENLEIIRGRTKQHGQFSLAVVSLNITSLGLRSLKEISDGDVIISGNKNLCYANTINWKKLFGTSGQKTKIISNRGENSCKATGQVCHALCSPEGCWGPEPRDCVSCRNVSRGRECVDKCNLLEGEPREFVENSECIQCHPECLPQAMNITCTGRGPDNCIQCAHYIDGPHCVKTCPAGVMGENNTLVWKYADAGHVCHLCHPNCTYGCTGPGLEGCPTNGPKIPSIATGMVGALLLLLVVALGIGLFM

SEQ ID NO: 56 - DNA, 732 bp, synthetic construct
  misc_feature 1..732: note = Description of Artificial Sequence: Synthetic polynucleotide
  source 1..732: mol_type = other DNA
cgcaaagtgtgtaacggaataggtattggtgaatttaaagactcactctccataaatgctacgaatattaaacacttcaaaaactgcacctccatcagtggcgatctccacatcctgccggtggcatttaggggtgactccttcacacatactcctcctctggatccacaggaactggatattctgaaaaccgtaaaggaaatcacagggtttttgctgattcaggcttggcctgaaaacaggacggacctccatgcctttgagaacctagaaatcatacgcggcaggaccaagcaacatggtcagttttctcttgcagtcgtcagcctgaacataacatccttgggattacgctccctcaaggagataagtgatggagatgtgataatttcaggaaacaaaaatttgtgctatgcaaatacaataaactggaaaaaactgtttgggacctccggtcagaaaaccaaaattataagcaacagaggtgaaaacagctgcaaggccacaggccaggtctgccatgccttgtgctcccccgagggctgctggggcccggagcccagggactgcgtctctggtggcggtggctcgggcggtggtgggtcgggtggcggcggatctggtggcggtggctcgttttgggtgctggtggtggttggtggagtcctggcttgctatagcttgctagtaacagtggcctttattattttctgggtgaggagtaagaggagc

SEQ ID NO: 57 - protein, 244 aa, synthetic construct
  REGION 1..244: note = Description of Artificial Sequence: Synthetic polypeptide
RKVCNGIGIGEFKDSLSINATNIKHFKNCTSISGDLHILPVAFRGDSFTHTPPLDPQELDILKTVKEITGFLLIQAWPENRTDLHAFENLEIIRGRTKQHGQFSLAVVSLNITSLGLRSLKEISDGDVIISGNKNLCYANTINWKKLFGTSGQKTKIISNRGENSCKATGQVCHALCSPEGCWGPEPRDCVSGGGGSGGGGSGGGGSGGGGSFWVLVVVGGVLACYSLLVTVAFIIFWVRSKRS

SEQ ID NO: 58 - DNA, 771 bp, synthetic construct
  misc_feature 1..771: note = Description of Artificial Sequence: Synthetic polynucleotide
  source 1..771: mol_type = other DNA
cgcaaagtgtgtaacggaataggtattggtgaatttaaagactcactctccataaatgctacgaatattaaacacttcaaaaactgcacctccatcagtggcgatctccacatcctgccggtggcatttaggggtgactccttcacacatactcctcctctggatccacaggaactggatattctgaaaaccgtaaaggaaatcacagggtttttgctgattcaggcttggcctgaaaacaggacggacctccatgcctttgagaacctagaaatcatacgcggcaggaccaagcaacatggtcagttttctcttgcagtcgtcagcctgaacataacatccttgggattacgctccctcaaggagataagtgatggagatgtgataatttcaggaaacaaaaatttgtgctatgcaaatacaataaactggaaaaaactgtttgggacctccggtcagaaaaccaaaattataagcaacagaggtgaaaacagctgcaaggccacaggccaggtctgccatgccttgtgctcccccgagggctgctggggcccggagcccagggactgcgtctcttgccggaatgtcagccgaggcagggaatgcgtggacaagggtggcggtggctcgggcggtggtgggtcgggtggcggcggatctggtggcggtggctcgttttgggtgctggtggtggttggtggagtcctggcttgctatagcttgctagtaacagtggcctttattattttctgggtgaggagtaagaggagc

SEQ ID NO: 59 - protein, 257 aa, synthetic construct
  REGION 1..257: note = Description of Artificial Sequence: Synthetic polypeptide
RKVCNGIGIGEFKDSLSINATNIKHFKNCTSISGDLHILPVAFRGDSFTHTPPLDPQELDILKTVKEITGFLLIQAWPENRTDLHAFENLEIIRGRTKQHGQFSLAVVSLNITSLGLRSLKEISDGDVIISGNKNLCYANTINWKKLFGTSGQKTKIISNRGENSCKATGQVCHALCSPEGCWGPEPRDCVSCRNVSRGRECVDKGGGGSGGGGSGGGGSGGGGSFWVLVVVGGVLACYSLLVTVAFIIFWVRSKRS

SEQ ID NO: 60 - DNA, 828 bp, synthetic construct
  misc_feature 1..828: note = Description of Artificial Sequence: Synthetic polynucleotide
  source 1..828: mol_type = other DNA
cgcaaagtgtgtaacggaataggtattggtgaatttaaagactcactctccataaatgctacgaatattaaacacttcaaaaactgcacctccatcagtggcgatctccacatcctgccggtggcatttaggggtgactccttcacacatactcctcctctggatccacaggaactggatattctgaaaaccgtaaaggaaatcacagggtttttgctgattcaggcttggcctgaaaacaggacggacctccatgcctttgagaacctagaaatcatacgcggcaggaccaagcaacatggtcagttttctcttgcagtcgtcagcctgaacataacatccttgggattacgctccctcaaggagataagtgatggagatgtgataatttcaggaaacaaaaatttgtgctatgcaaatacaataaactggaaaaaactgtttgggacctccggtcagaaaaccaaaattataagcaacagaggtgaaaacagctgcaaggccacaggccaggtctgccatgccttgtgctcccccgagggctgctggggcccggagcccagggactgcgtctcttgccggaatgtcagccgaggcagggaatgcgtggacaagtgcaaccttctggagggtgagccaagggagtttgtggagaactctgagtgcatacagggtggcggtggctcgggcggtggtgggtcgggtggcggcggatctggtggcggtggctcgttttgggtgctggtggtggttggtggagtcctggcttgctatagcttgctagtaacagtggcctttattattttctgggtgaggagtaagaggagc

SEQ ID NO: 61 - protein, 276 aa, synthetic construct
  REGION 1..276: note = Description of Artificial Sequence: Synthetic polypeptide
RKVCNGIGIGEFKDSLSINATNIKHFKNCTSISGDLHILPVAFRGDSFTHTPPLDPQELDILKTVKEITGFLLIQAWPENRTDLHAFENLEIIRGRTKQHGQFSLAVVSLNITSLGLRSLKEISDGDVIISGNKNLCYANTINWKKLFGTSGQKTKIISNRGENSCKATGQVCHALCSPEGCWGPEPRDCVSCRNVSRGRECVDKCNLLEGEPREFVENSECIQGGGGSGGGGSGGGGSGGGGSFWVLVVVGGVLACYSLLVTVAFIIFWVRSKRS

SEQ ID NO: 62 - DNA, 885 bp, synthetic construct
  misc_feature 1..885: note = Description of Artificial Sequence: Synthetic polynucleotide
  source 1..885: mol_type = other DNA
cgcaaagtgtgtaacggaataggtattggtgaatttaaagactcactctccataaatgctacgaatattaaacacttcaaaaactgcacctccatcagtggcgatctccacatcctgccggtggcatttaggggtgactccttcacacatactcctcctctggatccacaggaactggatattctgaaaaccgtaaaggaaatcacagggtttttgctgattcaggcttggcctgaaaacaggacggacctccatgcctttgagaacctagaaatcatacgcggcaggaccaagcaacatggtcagttttctcttgcagtcgtcagcctgaacataacatccttgggattacgctccctcaaggagataagtgatggagatgtgataatttcaggaaacaaaaatttgtgctatgcaaatacaataaactggaaaaaactgtttgggacctccggtcagaaaaccaaaattataagcaacagaggtgaaaacagctgcaaggccacaggccaggtctgccatgccttgtgctcccccgagggctgctggggcccggagcccagggactgcgtctcttgccggaatgtcagccgaggcagggaatgcgtggacaagtgcaaccttctggagggtgagccaagggagtttgtggagaactctgagtgcatacagtgccacccagagtgcctgcctcaggccatgaacatcacctgcacaggacggggaccagacaactgtatccagggcggaggcggaagcggaggcggaggctccggcggaggcggaagcttttgggtgctggtggtggttggtggagtcctggcttgctatagcttgctagtaacagtggcctttattattttctgggtgaggagtaagaggagc

SEQ ID NO: 63 - protein, 295 aa, synthetic construct
  REGION 1..295: note = Description of Artificial Sequence: Synthetic polypeptide
RKVCNGIGIGEFKDSLSINATNIKHFKNCTSISGDLHILPVAFRGDSFTHTPPLDPQELDILKTVKEITGFLLIQAWPENRTDLHAFENLEIIRGRTKQHGQFSLAVVSLNITSLGLRSLKEISDGDVIISGNKNLCYANTINWKKLFGTSGQKTKIISNRGENSCKATGQVCHALCSPEGCWGPEPRDCVSCRNVSRGRECVDKCNLLEGEPREFVENSECIQCHPECLPQAMNITCTGRGPDNCIQGGGGSGGGGSGGGGSFWVLVVVGGVLACYSLLVTVAFIIFWVRSKRS

SEQ ID NO: 64 - DNA, 924 bp, synthetic construct
  misc_feature 1..924: note = Description of Artificial Sequence: Synthetic polynucleotide
  source 1..924: mol_type = other DNA
cgcaaagtgtgtaacggaataggtattggtgaatttaaagactcactctccataaatgctacgaatattaaacacttcaaaaactgcacctccatcagtggcgatctccacatcctgccggtggcatttaggggtgactccttcacacatactcctcctctggatccacaggaactggatattctgaaaaccgtaaaggaaatcacagggtttttgctgattcaggcttggcctgaaaacaggacggacctccatgcctttgagaacctagaaatcatacgcggcaggaccaagcaacatggtcagttttctcttgcagtcgtcagcctgaacataacatccttgggattacgctccctcaaggagataagtgatggagatgtgataatttcaggaaacaaaaatttgtgctatgcaaatacaataaactggaaaaaactgtttgggacctccggtcagaaaaccaaaattataagcaacagaggtgaaaacagctgcaaggccacaggccaggtctgccatgccttgtgctcccccgagggctgctggggcccggagcccagggactgcgtctcttgccggaatgtcagccgaggcagggaatgcgtggacaagtgcaaccttctggagggtgagccaagggagtttgtggagaactctgagtgcatacagtgccacccagagtgcctgcctcaggccatgaacatcacctgcacaggacggggaccagacaactgtatccagtgtgcccactacattgacggcccccactgcgtcaagaccggcggaggcggaagcggaggcggaggctccggcggaggcggaagcttttgggtgctggtggtggttggtggagtcctggcttgctatagcttgctagtaacagtggcctttattattttctgggtgaggagtaagaggagc

SEQ ID NO: 65 - protein, 308 aa, synthetic construct
  REGION 1..308: note = Description of Artificial Sequence: Synthetic polypeptide
RKVCNGIGIGEFKDSLSINATNIKHFKNCTSISGDLHILPVAFRGDSFTHTPPLDPQELDILKTVKEITGFLLIQAWPENRTDLHAFENLEIIRGRTKQHGQFSLAVVSLNITSLGLRSLKEISDGDVIISGNKNLCYANTINWKKLFGTSGQKTKIISNRGENSCKATGQVCHALCSPEGCWGPEPRDCVSCRNVSRGRECVDKCNLLEGEPREFVENSECIQCHPECLPQAMNITCTGRGPDNCIQCAHYIDGPHCVKTGGGGSGGGGSGGGGSFWVLVVVGGVLACYSLLVTVAFIIFWVRSKRS

SEQ ID NO: 66 - DNA, 984 bp, synthetic construct
  misc_feature 1..984: note = Description of Artificial Sequence: Synthetic polynucleotide
  source 1..984: mol_type = other DNA
cgcaaagtgtgtaacggaataggtattggtgaatttaaagactcactctccataaatgctacgaatattaaacacttcaaaaactgcacctccatcagtggcgatctccacatcctgccggtggcatttaggggtgactccttcacacatactcctcctctggatccacaggaactggatattctgaaaaccgtaaaggaaatcacagggtttttgctgattcaggcttggcctgaaaacaggacggacctccatgcctttgagaacctagaaatcatacgcggcaggaccaagcaacatggtcagttttctcttgcagtcgtcagcctgaacataacatccttgggattacgctccctcaaggagataagtgatggagatgtgataatttcaggaaacaaaaatttgtgctatgcaaatacaataaactggaaaaaactgtttgggacctccggtcagaaaaccaaaattataagcaacagaggtgaaaacagctgcaaggccacaggccaggtctgccatgccttgtgctcccccgagggctgctggggcccggagcccagggactgcgtctcttgccggaatgtcagccgaggcagggaatgcgtggacaagtgcaaccttctggagggtgagccaagggagtttgtggagaactctgagtgcatacagtgccacccagagtgcctgcctcaggccatgaacatcacctgcacaggacggggaccagacaactgtatccagtgtgcccactacattgacggcccccactgcgtcaagacctgcccggcaggagtcatgggagaaaacaacaccctggtctggaagtacgcagacgccggccatgtgtgccacctgggcggaggcggaagcggaggcggaggctccttttgggtgctggtggtggttggtggagtcctggcttgctatagcttgctagtaacagtggcctttattattttctgggtgaggagtaagaggagc

SEQ ID NO: 67 - protein, 328 aa, synthetic construct
  REGION 1..328: note = Description of Artificial Sequence: Synthetic polypeptide
RKVCNGIGIGEFKDSLSINATNIKHFKNCTSISGDLHILPVAFRGDSFTHTPPLDPQELDILKTVKEITGFLLIQAWPENRTDLHAFENLEIIRGRTKQHGQFSLAVVSLNITSLGLRSLKEISDGDVIISGNKNLCYANTINWKKLFGTSGQKTKIISNRGENSCKATGQVCHALCSPEGCWGPEPRDCVSCRNVSRGRECVDKCNLLEGEPREFVENSECIQCHPECLPQAMNITCTGRGPDNCIQCAHYIDGPHCVKTCPAGVMGENNTLVWKYADAGHVCHLGGGGSGGGGSFWVLVVVGGVLACYSLLVTVAFIIFWVRSKRS

SEQ ID NO: 68 - DNA, 1032 bp, synthetic construct
  misc_feature 1..1032: note = Description of Artificial Sequence: Synthetic polynucleotide
  source 1..1032: mol_type = other DNA
cgcaaagtgtgtaacggaataggtattggtgaatttaaagactcactctccataaatgctacgaatattaaacacttcaaaaactgcacctccatcagtggcgatctccacatcctgccggtggcatttaggggtgactccttcacacatactcctcctctggatccacaggaactggatattctgaaaaccgtaaaggaaatcacagggtttttgctgattcaggcttggcctgaaaacaggacggacctccatgcctttgagaacctagaaatcatacgcggcaggaccaagcaacatggtcagttttctcttgcagtcgtcagcctgaacataacatccttgggattacgctccctcaaggagataagtgatggagatgtgataatttcaggaaacaaaaatttgtgctatgcaaatacaataaactggaaaaaactgtttgggacctccggtcagaaaaccaaaattataagcaacagaggtgaaaacagctgcaaggccacaggccaggtctgccatgccttgtgctcccccgagggctgctggggcccggagcccagggactgcgtctcttgccggaatgtcagccgaggcagggaatgcgtggacaagtgcaaccttctggagggtgagccaagggagtttgtggagaactctgagtgcatacagtgccacccagagtgcctgcctcaggccatgaacatcacctgcacaggacggggaccagacaactgtatccagtgtgcccactacattgacggcccccactgcgtcaagacctgcccggcaggagtcatgggagaaaacaacaccctggtctggaagtacgcagacgccggccatgtgtgccacctgtgccatccaaactgcacctacggatgcactgggccaggtcttgaaggctgtccaggtggcggtggcggcggatctttttgggtgctggtggtggttggtggagtcctggcttgctatagcttgctagtaacagtggcctttattattttctgggtgaggagtaagaggagctaa

SEQ ID NO: 69 - protein, 343 aa, synthetic construct
  REGION 1..343: note = Description of Artificial Sequence: Synthetic polypeptide
RKVCNGIGIGEFKDSLSINATNIKHFKNCTSISGDLHILPVAFRGDSFTHTPPLDPQELDILKTVKEITGFLLIQAWPENRTDLHAFENLEIIRGRTKQHGQFSLAVVSLNITSLGLRSLKEISDGDVIISGNKNLCYANTINWKKLFGTSGQKTKIISNRGENSCKATGQVCHALCSPEGCWGPEPRDCVSCRNVSRGRECVDKCNLLEGEPREFVENSECIQCHPECLPQAMNITCTGRGPDNCIQCAHYIDGPHCVKTCPAGVMGENNTLVWKYADAGHVCHLCHPNCTYGCTGPGLEGCPGGGGGGSFWVLVVVGGVLACYSLLVTVAFIIFWVRSKRS

SEQ ID NO: 70 - DNA, 786 bp, synthetic construct
  misc_feature 1..786: note = Description of Artificial Sequence: Synthetic polynucleotide
  source 1..786: mol_type = other DNA
atgaggctccctgctcagctcctggggctgctaatgctctgggtcccaggatccagtgggcgcaaagtgtgtaacggaataggtattggtgaatttaaagactcactctccataaatgctacgaatattaaacacttcaaaaactgcacctccatcagtggcgatctccacatcctgccggtggcatttaggggtgactccttcacacatactcctcctctggatccacaggaactggatattctgaaaaccgtaaaggaaatcacagggtttttgctgattcaggcttggcctgaaaacaggacggacctccatgcctttgagaacctagaaatcatacgcggcaggaccaagcaacatggtcagttttctcttgcagtcgtcagcctgaacataacatccttgggattacgctccctcaaggagataagtgatggagatgtgataatttcaggaaacaaaaatttgtgctatgcaaatacaataaactggaaaaaactgtttgggacctccggtcagaaaaccaaaattataagcaacagaggtgaaaacagctgcaaggccacaggccaggtctgccatgccttgtgctcccccgagggctgctggggcccggagcccagggactgcgtctctggtggcggtggctcgggcggtggtgggtcgggtggcggcggatctggtggcggtggctcggagataacactcattatttttggggtgatggctggtgttattggaacgatcctcttaatttcttacggtattcgccgaggaggtggaagc

SEQ ID NO: 71 - protein, 262 aa, synthetic construct
  REGION 1..262: note = Description of Artificial Sequence: Synthetic polypeptide
MRLPAQLLGLLMLWVPGSSGRKVCNGIGIGEFKDSLSINATNIKHFKNCTSISGDLHILPVAFRGDSFTHTPPLDPQELDILKTVKEITGFLLIQAWPENRTDLHAFENLEIIRGRTKQHGQFSLAVVSLNITSLGLRSLKEISDGDVIISGNKNLCYANTINWKKLFGTSGQKTKIISNRGENSCKATGQVCHALCSPEGCWGPEPRDCVSGGGGSGGGGSGGGGSGGGGSEITLIIFGVMAGVIGTILLISYGIRRGGGS

SEQ ID NO: 72 - DNA, 726 bp, synthetic construct
  misc_feature 1..726: note = Description of Artificial Sequence: Synthetic polynucleotide
  source 1..726: mol_type = other DNA
cgcaaagtgtgtaacggaataggtattggtgaatttaaagactcactctccataaatgctacgaatattaaacacttcaaaaactgcacctccatcagtggcgatctccacatcctgccggtggcatttaggggtgactccttcacacatactcctcctctggatccacaggaactggatattctgaaaaccgtaaaggaaatcacagggtttttgctgattcaggcttggcctgaaaacaggacggacctccatgcctttgagaacctagaaatcatacgcggcaggaccaagcaacatggtcagttttctcttgcagtcgtcagcctgaacataacatccttgggattacgctccctcaaggagataagtgatggagatgtgataatttcaggaaacaaaaatttgtgctatgcaaatacaataaactggaaaaaactgtttgggacctccggtcagaaaaccaaaattataagcaacagaggtgaaaacagctgcaaggccacaggccaggtctgccatgccttgtgctcccccgagggctgctggggcccggagcccagggactgcgtctctggtggcggtggctcgggcggtggtgggtcgggtggcggcggatctggtggcggtggctcggagataacactcattatttttggggtgatggctggtgttattggaacgatcctcttaatttcttacggtattcgccgaggaggtggaagc

SEQ ID NO: 73 - protein, 242 aa, synthetic construct
  REGION 1..242: note = Description of Artificial Sequence: Synthetic polypeptide
RKVCNGIGIGEFKDSLSINATNIKHFKNCTSISGDLHILPVAFRGDSFTHTPPLDPQELDILKTVKEITGFLLIQAWPENRTDLHAFENLEIIRGRTKQHGQFSLAVVSLNITSLGLRSLKEISDGDVIISGNKNLCYANTINWKKLFGTSGQKTKIISNRGENSCKATGQVCHALCSPEGCWGPEPRDCVSGGGGSGGGGSGGGGSGGGGSEITLIIFGVMAGVIGTILLISYGIRRGGGS

SEQ ID NO: 74 - DNA, 777 bp, synthetic construct
  misc_feature 1..777: note = Description of Artificial Sequence: Synthetic polynucleotide
  source 1..777: mol_type = other DNA
atgaggctccctgctcagctcctggggctgctaatgctctgggtcccaggatccagtgggcgcaaagtgtgtaacggaataggtattggtgaatttaaagactcactctccataaatgctacgaatattaaacacttcaaaaactgcacctccatcagtggcgatctccacatcctgccggtggcatttaggggtgactccttcacacatactcctcctctggatccacaggaactggatattctgaaaaccgtaaaggaaatcacagggtttttgctgattcaggcttggcctgaaaacaggacggacctccatgcctttgagaacctagaaatcatacgcggcaggaccaagcaacatggtcagttttctcttgcagtcgtcagcctgaacataacatccttgggattacgctccctcaaggagataagtgatggagatgtgataatttcaggaaacaaaaatttgtgctatgcaaatacaataaactggaaaaaactgtttgggacctccggtcagaaaaccaaaattataagcaacagaggtgaaaacagctgcaaggccacaggccaggtctgccatgccttgtgctcccccgagggctgctggggcccggagcccagggactgcgtctctggtggcggtggctcgggcggtggtgggtcgggtggcggcggatctggtggcggtggctcgataacactcattatttttggggtgatggctggtgttattggaacgatcctcttaatttcttacggtattggaggtggaagc

SEQ ID NO: 75 - protein, 259 aa, synthetic construct
  REGION 1..259: note = Description of Artificial Sequence: Synthetic polypeptide
MRLPAQLLGLLMLWVPGSSGRKVCNGIGIGEFKDSLSINATNIKHFKNCTSISGDLHILPVAFRGDSFTHTPPLDPQELDILKTVKEITGFLLIQAWPENRTDLHAFENLEIIRGRTKQHGQFSLAVVSLNITSLGLRSLKEISDGDVIISGNKNLCYANTINWKKLFGTSGQKTKIISNRGENSCKATGQVCHALCSPEGCWGPEPRDCVSGGGGSGGGGSGGGGSGGGGSITLIIFGVMAGVIGTILLISYGIGGGS

SEQ ID NO: 76 - DNA, 717 bp, synthetic construct
  misc_feature 1..717: note = Description of Artificial Sequence: Synthetic polynucleotide
  source 1..717: mol_type = other DNA
cgcaaagtgtgtaacggaataggtattggtgaatttaaagactcactctccataaatgctacgaatattaaacacttcaaaaactgcacctccatcagtggcgatctccacatcctgccggtggcatttaggggtgactccttcacacatactcctcctctggatccacaggaactggatattctgaaaaccgtaaaggaaatcacagggtttttgctgattcaggcttggcctgaaaacaggacggacctccatgcctttgagaacctagaaatcatacgcggcaggaccaagcaacatggtcagttttctcttgcagtcgtcagcctgaacataacatccttgggattacgctccctcaaggagataagtgatggagatgtgataatttcaggaaacaaaaatttgtgctatgcaaatacaataaactggaaaaaactgtttgggacctccggtcagaaaaccaaaattataagcaacagaggtgaaaacagctgcaaggccacaggccaggtctgccatgccttgtgctcccccgagggctgctggggcccggagcccagggactgcgtctctggtggcggtggctcgggcggtggtgggtcgggtggcggcggatctggtggcggtggctcgataacactcattatttttggggtgatggctggtgttattggaacgatcctcttaatttcttacggtattggaggtggaagc

SEQ ID NO: 77 - protein, 239 aa, synthetic construct
  REGION 1..239: note = Description of Artificial Sequence: Synthetic polypeptide
RKVCNGIGIGEFKDSLSINATNIKHFKNCTSISGDLHILPVAFRGDSFTHTPPLDPQELDILKTVKEITGFLLIQAWPENRTDLHAFENLEIIRGRTKQHGQFSLAVVSLNITSLGLRSLKEISDGDVIISGNKNLCYANTINWKKLFGTSGQKTKIISNRGENSCKATGQVCHALCSPEGCWGPEPRDCVSGGGGSGGGGSGGGGSGGGGSITLIIFGVMAGVIGTILLISYGIGGGS

SEQ ID NO: 78 - DNA, 777 bp, synthetic construct
  misc_feature 1..777: note = Description of Artificial Sequence: Synthetic polynucleotide
  source 1..777: mol_type = other DNA
atgaggctccctgctcagctcctggggctgctaatgctctgggtcccaggatccagtgggcgcaaagtgtgtaacggaataggtattggtgaatttaaagactcactctccataaatgctacgaatattaaacacttcaaaaactgcacctccatcagtggcgatctccacatcctgccggtggcatttaggggtgactccttcacacatactcctcctctggatccacaggaactggatattctgaaaaccgtaaaggaaatcacagggtttttgctgattcaggcttggcctgaaaacaggacggacctccatgcctttgagaacctagaaatcatacgcggcaggaccaagcaacatggtcagttttctcttgcagtcgtcagcctgaacataacatccttgggattacgctccctcaaggagataagtgatggagatgtgataatttcaggaaacaaaaatttgtgctatgcaaatacaataaactggaaaaaactgtttgggacctccggtcagaaaaccaaaattataagcaacagaggtgaaaacagctgcaaggccacaggccaggtctgccatgccttgtgctcccccgagggctgctggggcccggagcccagggactgcgtctctggtggcggtggctcgggcggtggtgggtcgggtggcggcggatctggtggcggtggctcgataacactcattatttttggggtgatggctggtgttattggaacgatcctcttagccctgctcatctggggaggtggaagc

SEQ ID NO: 79 - protein, 259 aa, synthetic construct
  REGION 1..259: note = Description of Artificial Sequence: Synthetic polypeptide
MRLPAQLLGLLMLWVPGSSGRKVCNGIGIGEFKDSLSINATNIKHFKNCTSISGDLHILPVAFRGDSFTHTPPLDPQELDILKTVKEITGFLLIQAWPENRTDLHAFENLEIIRGRTKQHGQFSLAVVSLNITSLGLRSLKEISDGDVIISGNKNLCYANTINWKKLFGTSGQKTKIISNRGENSCKATGQVCHALCSPEGCWGPEPRDCVSGGGGSGGGGSGGGGSGGGGSITLIIFGVMAGVIGTILLALLIWGGGS

SEQ ID NO: 80 - DNA, 717 bp, synthetic construct
  misc_feature 1..717: note = Description of Artificial Sequence: Synthetic polynucleotide
  source 1..717: mol_type = other DNA
cgcaaagtgtgtaacggaataggtattggtgaatttaaagactcactctccataaatgctacgaatattaaacacttcaaaaactgcacctccatcagtggcgatctccacatcctgccggtggcatttaggggtgactccttcacacatactcctcctctggatccacaggaactggatattctgaaaaccgtaaaggaaatcacagggtttttgctgattcaggcttggcctgaaaacaggacggacctccatgcctttgagaacctagaaatcatacgcggcaggaccaagcaacatggtcagttttctcttgcagtcgtcagcctgaacataacatccttgggattacgctccctcaaggagataagtgatggagatgtgataatttcaggaaacaaaaatttgtgctatgcaaatacaataaactggaaaaaactgtttgggacctccggtcagaaaaccaaaattataagcaacagaggtgaaaacagctgcaaggccacaggccaggtctgccatgccttgtgctcccccgagggctgctggggcccggagcccagggactgcgtctctggtggcggtggctcgggcggtggtgggtcgggtggcggcggatctggtggcggtggctcgataacactcattatttttggggtgatggctggtgttattggaacgatcctcttagccctgctcatctggggaggtggaagc

SEQ ID NO: 81 - protein, 239 aa, synthetic construct
  REGION 1..239: note = Description of Artificial Sequence: Synthetic polypeptide
RKVCNGIGIGEFKDSLSINATNIKHFKNCTSISGDLHILPVAFRGDSFTHTPPLDPQELDILKTVKEITGFLLIQAWPENRTDLHAFENLEIIRGRTKQHGQFSLAVVSLNITSLGLRSLKEISDGDVIISGNKNLCYANTINWKKLFGTSGQKTKIISNRGENSCKATGQVCHALCSPEGCWGPEPRDCVSGGGGSGGGGSGGGGSGGGGSITLIIFGVMAGVIGTILLALLIWGGGS

SEQ ID NO: 82 - DNA, 771 bp, synthetic construct
  misc_feature 1..771: note = Description of Artificial Sequence: Synthetic polynucleotide
  source 1..771: mol_type = other DNA
atgaggctccctgctcagctcctggggctgctaatgctctgggtcccaggatccagtgggcgcaaagtgtgtaacggaataggtattggtgaatttaaagactcactctccataaatgctacgaatattaaacacttcaaaaactgcacctccatcagtggcgatctccacatcctgccggtggcatttaggggtgactccttcacacatactcctcctctggatccacaggaactggatattctgaaaaccgtaaaggaaatcacagggtttttgctgattcaggcttggcctgaaaacaggacggacctccatgcctttgagaacctagaaatcatacgcggcaggaccaagcaacatggtcagttttctcttgcagtcgtcagcctgaacataacatccttgggattacgctccctcaaggagataagtgatggagatgtgataatttcaggaaacaaaaatttgtgctatgcaaatacaataaactggaaaaaactgtttgggacctccggtcagaaaaccaaaattataagcaacagaggtgaaaacagctgcaaggccacaggccaggtctgccatgccttgtgctcccccgagggctgctggggcccggagcccagggactgcgtctctggtggcggtggctcgggcggtggtgggtcgggtggcggcggatctggtggcggtggctcgctctgctacctgctggatggaatcctcttcatctatggtgtcattctcactgccttgttcctgggaggtggaagc

SEQ ID NO: 83 - protein, 257 aa, synthetic construct
  REGION 1..257: note = Description of Artificial Sequence: Synthetic polypeptide
MRLPAQLLGLLMLWVPGSSGRKVCNGIGIGEFKDSLSINATNIKHFKNCTSISGDLHILPVAFRGDSFTHTPPLDPQELDILKTVKEITGFLLIQAWPENRTDLHAFENLEIIRGRTKQHGQFSLAVVSLNITSLGLRSLKEISDGDVIISGNKNLCYANTINWKKLFGTSGQKTKIISNRGENSCKATGQVCHALCSPEGCWGPEPRDCVSGGGGSGGGGSGGGGSGGGGSLCYLLDGILFIYGVILTALFLGGGS

SEQ ID NO: 84 - DNA, 711 bp, synthetic construct
  misc_feature 1..711: note = Description of Artificial Sequence: Synthetic polynucleotide
  source 1..711: mol_type = other DNA
cgcaaagtgtgtaacggaataggtattggtgaatttaaagactcactctccataaatgctacgaatattaaacacttcaaaaactgcacctccatcagtggcgatctccacatcctgccggtggcatttaggggtgactccttcacacatactcctcctctggatccacaggaactggatattctgaaaaccgtaaaggaaatcacagggtttttgctgattcaggcttggcctgaaaacaggacggacctccatgcctttgagaacctagaaatcatacgcggcaggaccaagcaacatggtcagttttctcttgcagtcgtcagcctgaacataacatccttgggattacgctccctcaaggagataagtgatggagatgtgataatttcaggaaacaaaaatttgtgctatgcaaatacaataaactggaaaaaactgtttgggacctccggtcagaaaaccaaaattataagcaacagaggtgaaaacagctgcaaggccacaggccaggtctgccatgccttgtgctcccccgagggctgctggggcccggagcccagggactgcgtctctggtggcggtggctcgggcggtggtgggtcgggtggcggcggatctggtggcggtggctcgctctgctacctgctggatggaatcctcttcatctatggtgtcattctcactgccttgttcctgggaggtggaagc

SEQ ID NO: 85 - protein, 237 aa, synthetic construct
  REGION 1..237: note = Description of Artificial Sequence: Synthetic polypeptide
RKVCNGIGIGEFKDSLSINATNIKHFKNCTSISGDLHILPVAFRGDSFTHTPPLDPQELDILKTVKEITGFLLIQAWPENRTDLHAFENLEIIRGRTKQHGQFSLAVVSLNITSLGLRSLKEISDGDVIISGNKNLCYANTINWKKLFGTSGQKTKIISNRGENSCKATGQVCHALCSPEGCWGPEPRDCVSGGGGSGGGGSGGGGSGGGGSLCYLLDGILFIYGVILTALFLGGGS

SEQ ID NO: 86 - DNA, 1077 bp, synthetic construct
  misc_feature 1..1077: note = Description of Artificial Sequence: Synthetic polynucleotide
  source 1..1077: mol_type = other DNA
atgcttctcctggtgacaagccttctgctctgtgagttaccacacccagcattcctcctgatcccacgcaaagtgtgtaacggaataggtattggtgaatttaaagactcactctccataaatgctacgaatattaaacacttcaaaaactgcacctccatcagtggcgatctccacatcctgccggtggcatttaggggtgactccttcacacatactcctcctctggatccacaggaactggatattctgaaaaccgtaaaggaaatcacagggtttttgctgattcaggcttggcctgaaaacaggacggacctccatgcctttgagaacctagaaatcatacgcggcaggaccaagcaacatggtcagttttctcttgcagtcgtcagcctgaacataacatccttgggattacgctccctcaaggagataagtgatggagatgtgataatttcaggaaacaaaaatttgtgctatgcaaatacaataaactggaaaaaactgtttgggacctccggtcagaaaaccaaaattataagcaacagaggtgaaaacagctgcaaggccacaggccaggcctgccaccagctgtgcgcccgagggcactgctggggtccagggcccacccagtgtgtcaactgcagccagttccttcggggccaggagtgcgtggaggaatgccgagtactgcaggggctccccagggagtatgtgaatgccaggcactgtttgccgtgccaccctgagtgtcagccccagaatggctcagtgacctgttttggaccggaggctgaccagtgtgtggcctgtgcccactataaggaccctcccttctgcgtggcccgctgccccagcggtgtgaaacctgacctctcctacatgcccatctggaagtttccagatgaggagggcgcatgccagccttgccccatcaactgcacccactcctgtgtggacctggatgacaagggctgccccgccgagcagagagccagccctctgacgtccatcatctctgcggtggttggcattctgctggtcgtggtcttgggggtggtctttgggatcctcatc

SEQ ID NO: 87 - protein, 359 aa, synthetic construct
  REGION 1..359: note = Description of Artificial Sequence: Synthetic polypeptide
MLLLVTSLLLCELPHPAFLLIPRKVCNGIGIGEFKDSLSINATNIKHFKNCTSISGDLHILPVAFRGDSFTHTPPLDPQELDILKTVKEITGFLLIQAWPENRTDLHAFENLEIIRGRTKQHGQFSLAVVSLNITSLGLRSLKEISDGDVIISGNKNLCYANTINWKKLFGTSGQKTKIISNRGENSCKATGQACHQLCARGHCWGPGPTQCVNCSQFLRGQECVEECRVLQGLPREYVNARHCLPCHPECQPQNGSVTCFGPEADQCVACAHYKDPPFCVARCPSGVKPDLSYMPIWKFPDEEGACQPCPINCTHSCVDLDDKGCPAEQRASPLTSIISAVVGILLVVVLGVVFGILI

SEQ ID NO: 88 - DNA, 1011 bp, synthetic construct
  misc_feature 1..1011: note = Description of Artificial Sequence: Synthetic polynucleotide
  source 1..1011: mol_type = other DNA
cgcaaagtgtgtaacggaataggtattggtgaatttaaagactcactctccataaatgctacgaatattaaacacttcaaaaactgcacctccatcagtggcgatctccacatcctgccggtggcatttaggggtgactccttcacacatactcctcctctggatccacaggaactggatattctgaaaaccgtaaaggaaatcacagggtttttgctgattcaggcttggcctgaaaacaggacggacctccatgcctttgagaacctagaaatcatacgcggcaggaccaagcaacatggtcagttttctcttgcagtcgtcagcctgaacataacatccttgggattacgctccctcaaggagataagtgatggagatgtgataatttcaggaaacaaaaatttgtgctatgcaaatacaataaactggaaaaaactgtttgggacctccggtcagaaaaccaaaattataagcaacagaggtgaaaacagctgcaaggccacaggccaggcctgccaccagctgtgcgcccgagggcactgctggggtccagggcccacccagtgtgtcaactgcagccagttccttcggggccaggagtgcgtggaggaatgccgagtactgcaggggctccccagggagtatgtgaatgccaggcactgtttgccgtgccaccctgagtgtcagccccagaatggctcagtgacctgttttggaccggaggctgaccagtgtgtggcctgtgcccactataaggaccctcccttctgcgtggcccgctgccccagcggtgtgaaacctgacctctcctacatgcccatctggaagtttccagatgaggagggcgcatgccagccttgccccatcaactgcacccactcctgtgtggacctggatgacaagggctgccccgccgagcagagagccagccctctgacgtccatcatctctgcggtggttggcattctgctggtcgtggtcttgggggtggtctttgggatcctcatc

SEQ ID NO: 89 - protein, 337 aa, synthetic construct
  REGION 1..337: note = Description of Artificial Sequence: Synthetic polypeptide
RKVCNGIGIGEFKDSLSINATNIKHFKNCTSISGDLHILPVAFRGDSFTHTPPLDPQELDILKTVKEITGFLLIQAWPENRTDLHAFENLEIIRGRTKQHGQFSLAVVSLNITSLGLRSLKEISDGDVIISGNKNLCYANTINWKKLFGTSGQKTKIISNRGENSCKATGQACHQLCARGHCWGPGPTQCVNCSQFLRGQECVEECRVLQGLPREYVNARHCLPCHPECQPQNGSVTCFGPEADQCVACAHYKDPPFCVARCPSGVKPDLSYMPIWKFPDEEGACQPCPINCTHSCVDLDDKGCPAEQRASPLTSIISAVVGILLVVVLGVVFGILI

SEQ ID NO: 90 - DNA, 1029 bp, synthetic construct
  misc_feature 1..1029: note = Description of Artificial Sequence: Synthetic polynucleotide
  source 1..1029: mol_type = other DNA
atgcttctcctggtgacaagccttctgctctgtgagttaccacacccagcattcctcctgatcccacgcaaagtgtgtaacggaataggtattggtgaatttaaagactcactctccataaatgctacgaatattaaacacttcaaaaactgcacctccatcagtggcgatctccacatcctgccggtggcatttaggggtgactccttcacacatactcctcctctggatccacaggaactggatattctgaaaaccgtaaaggaaatcacagggtttttgctgattcaggcttggcctgaaaacaggacggacctccatgcctttgagaacctagaaatcatacgcggcaggaccaagcaacatggtcagttttctcttgcagtcgtcagcctgaacataacatccttgggattacgctccctcaaggagataagtgatggagatgtgataatttcaggaaacaaaaatttgtgctatgcaaatacaataaactggaaaaaactgtttgggacctccggtcagaaaaccaaaattataagcaacagaggtgaaaacagctgcaaggccacaggccaggcctgccaccagctgtgcgcccgagggcactgctggggtccagggcccacccagtgtgtcaactgcagccagttccttcggggccaggagtgcgtggaggaatgccgagtactgcaggggctccccagggagtatgtgaatgccaggcactgtttgccgtgccaccctgagtgtcagccccagaatggctcagtgacctgttttggaccggaggctgaccagtgtgtggcctgtgcccactataaggaccctcccttctgcgtggcccgctgccccagcggtgtgaaacctgacctctcctacatgcccatctggaagtttccagatgaggagggcgcatgccagccttgccccatcaactgcacccactcccctctgacgtccatcatctctgcggtggttggcattctgctggtcgtggtcttgggggtggtctttgggatcctcatc

SEQ ID NO: 91 - protein, 343 aa, synthetic construct
  REGION 1..343: note = Description of Artificial Sequence: Synthetic polypeptide
MLLLVTSLLLCELPHPAFLLIPRKVCNGIGIGEFKDSLSINATNIKHFKNCTSISGDLHILPVAFRGDSFTHTPPLDPQELDILKTVKEITGFLLIQAWPENRTDLHAFENLEIIRGRTKQHGQFSLAVVSLNITSLGLRSLKEISDGDVIISGNKNLCYANTINWKKLFGTSGQKTKIISNRGENSCKATGQACHQLCARGHCWGPGPTQCVNCSQFLRGQECVEECRVLQGLPREYVNARHCLPCHPECQPQNGSVTCFGPEADQCVACAHYKDPPFCVARCPSGVKPDLSYMPIWKFPDEEGACQPCPINCTHSPLTSIISAVVGILLVVVLGVVFGILI

SEQ ID NO: 92 - DNA, 963 bp, synthetic construct
  misc_feature 1..963: note = Description of Artificial Sequence: Synthetic polynucleotide
  source 1..963: mol_type = other DNA
cgcaaagtgtgtaacggaataggtattggtgaatttaaagactcactctccataaatgctacgaatattaaacacttcaaaaactgcacctccatcagtggcgatctccacatcctgccggtggcatttaggggtgactccttcacacatactcctcctctggatccacaggaactggatattctgaaaaccgtaaaggaaatcacagggtttttgctgattcaggcttggcctgaaaacaggacggacctccatgcctttgagaacctagaaatcatacgcggcaggaccaagcaacatggtcagttttctcttgcagtcgtcagcctgaacataacatccttgggattacgctccctcaaggagataagtgatggagatgtgataatttcaggaaacaaaaatttgtgctatgcaaatacaataaactggaaaaaactgtttgggacctccggtcagaaaaccaaaattataagcaacagaggtgaaaacagctgcaaggccacaggccaggcctgccaccagctgtgcgcccgagggcactgctggggtccagggcccacccagtgtgtcaactgcagccagttccttcggggccaggagtgcgtggaggaatgccgagtactgcaggggctccccagggagtatgtgaatgccaggcactgtttgccgtgccaccctgagtgtcagccccagaatggctcagtgacctgttttggaccggaggctgaccagtgtgtggcctgtgcccactataaggaccctcccttctgcgtggcccgctgccccagcggtgtgaaacctgacctctcctacatgcccatctggaagtttccagatgaggagggcgcatgccagccttgccccatcaactgcacccactcccctctgacgtccatcatctctgcggtggttggcattctgctggtcgtggtcttgggggtggtctttgggatcctcatc

SEQ ID NO: 93 - protein, 321 aa, synthetic construct
  REGION 1..321: note = Description of Artificial Sequence: Synthetic polypeptide
RKVCNGIGIGEFKDSLSINATNIKHFKNCTSISGDLHILPVAFRGDSFTHTPPLDPQELDILKTVKEITGFLLIQAWPENRTDLHAFENLEIIRGRTKQHGQFSLAVVSLNITSLGLRSLKEISDGDVIISGNKNLCYANTINWKKLFGTSGQKTKIISNRGENSCKATGQACHQLCARGHCWGPGPTQCVNCSQFLRGQECVEECRVLQGLPREYVNARHCLPCHPECQPQNGSVTCFGPEADQCVACAHYKDPPFCVARCPSGVKPDLSYMPIWKFPDEEGACQPCPINCTHSPLTSIISAVVGILLVVVLGVVFGILI

SEQ ID NO: 94 - DNA, 1080 bp, synthetic construct
  misc_feature 1..1080: note = Description of Artificial Sequence: Synthetic polynucleotide
  source 1..1080: mol_type = other DNA
atgcttctcctggtgacaagccttctgctctgtgagttaccacacccagcattcctcctgatcccacgcaaagtgtgtaacggaataggtattggtgaatttaaagactcactctccataaatgctacgaatattaaacacttcaaaaactgcacctccatcagtggcgatctccacatcctgccggtggcatttaggggtgactccttcacacatactcctcctctggatccacaggaactggatattctgaaaaccgtaaaggaaatcacagggtttttgctgattcaggcttggcctgaaaacaggacggacctccatgcctttgagaacctagaaatcatacgcggcaggaccaagcaacatggtcagttttctcttgcagtcgtcagcctgaacataacatccttgggattacgctccctcaaggagataagtgatggagatgtgataatttcaggaaacaaaaatttgtgctatgcaaatacaataaactggaaaaaactgtttgggacctccggtcagaaaaccaaaattataagcaacagaggtgaaaacagctgcaaggccacaggccaggtgtgtgacccactgtgctcctctgggggatgctggggcccaggccctggtcagtgcttgtcctgtcgaaattatagccgaggaggtgtctgtgtgacccactgcaactttctgaatggggagcctcgagaatttgcccatgaggccgaatgcttctcctgccacccggaatgccaacccatggagggcactgccacatgcaatggctcgggctctgatacttgtgctcaatgtgcccattttcgagatgggccccactgtgtgagcagctgcccccatggagtcctaggtgccaagggcccaatctacaagtacccagatgttcagaatgaatgtcggccctgccatgagaactgcacccaggggtgtaaaggaccagagcttcaagactgtttaggacaaacactggtgctgatcggcaaaacccatctgacaatggctttgacagtgatagcaggattggtagtgattttcatgatgctgggcggcacttttctctac

SEQ ID NO: 95 - protein, 360 aa, synthetic construct
  REGION 1..360: note = Description of Artificial Sequence: Synthetic polypeptide
MLLLVTSLLLCELPHPAFLLIPRKVCNGIGIGEFKDSLSINATNIKHFKNCTSISGDLHILPVAFRGDSFTHTPPLDPQELDILKTVKEITGFLLIQAWPENRTDLHAFENLEIIRGRTKQHGQFSLAVVSLNITSLGLRSLKEISDGDVIISGNKNLCYANTINWKKLFGTSGQKTKIISNRGENSCKATGQVCDPLCSSGGCWGPGPGQCLSCRNYSRGGVCVTHCNFLNGEPREFAHEAECFSCHPECQPMEGTATCNGSGSDTCAQCAHFRDGPHCVSSCPHGVLGAKGPIYKYPDVQNECRPCHENCTQGCKGPELQDCLGQTLVLIGKTHLTMALTVIAGLVVIFMMLGGTFLY

SEQ ID NO: 96 - DNA, 1014 bp, synthetic construct
  misc_feature 1..1014: note = Description of Artificial Sequence: Synthetic polynucleotide
  source 1..1014: mol_type = other DNA
cgcaaagtgtgtaacggaataggtattggtgaatttaaagactcactctccataaatgctacgaatattaaacacttcaaaaactgcacctccatcagtggcgatctccacatcctgccggtggcatttaggggtgactccttcacacatactcctcctctggatccacaggaactggatattctgaaaaccgtaaaggaaatcacagggtttttgctgattcaggcttggcctgaaaacaggacggacctccatgcctttgagaacctagaaatcatacgcggcaggaccaagcaacatggtcagttttctcttgcagtcgtcagcctgaacataacatccttgggattacgctccctcaaggagataagtgatggagatgtgataatttcaggaaacaaaaatttgtgctatgcaaatacaataaactggaaaaaactgtttgggacctccggtcagaaaaccaaaattataagcaacagaggtgaaaacagctgcaaggccacaggccaggtgtgtgacccactgtgctcctctgggggatgctggggcccaggccctggtcagtgcttgtcctgtcgaaattatagccgaggaggtgtctgtgtgacccactgcaactttctgaatggggagcctcgagaatttgcccatgaggccgaatgcttctcctgccacccggaatgccaacccatggagggcactgccacatgcaatggctcgggctctgatacttgtgctcaatgtgcccattttcgagatgggccccactgtgtgagcagctgcccccatggagtcctaggtgccaagggcccaatctacaagtacccagatgttcagaatgaatgtcggccctgccatgagaactgcacccaggggtgtaaaggaccagagcttcaagactgtttaggacaaacactggtgctgatcggcaaaacccatctgacaatggctttgacagtgatagcaggattggtagtgattttcatgatgctgggcggcacttttctctac

SEQ ID NO: 97 - protein, 338 aa, synthetic construct
  REGION 1..338: note = Description of Artificial Sequence: Synthetic polypeptide
RKVCNGIGIGEFKDSLSINATNIKHFKNCTSISGDLHILPVAFRGDSFTHTPPLDPQELDILKTVKEITGFLLIQAWPENRTDLHAFENLEIIRGRTKQHGQFSLAVVSLNITSLGLRSLKEISDGDVIISGNKNLCYANTINWKKLFGTSGQKTKIISNRGENSCKATGQVCDPLCSSGGCWGPGPGQCLSCRNYSRGGVCVTHCNFLNGEPREFAHEAECFSCHPECQPMEGTATCNGSGSDTCAQCAHFRDGPHCVSSCPHGVLGAKGPIYKYPDVQNECRPCHENCTQGCKGPELQDCLGQTLVLIGKTHLTMALTVIAGLVVIFMMLGGTFLY

SEQ ID NO: 98 - DNA, 1101 bp, synthetic construct
  misc_feature 1..1101: note = Description of Artificial Sequence: Synthetic polynucleotide
  source 1..1101: mol_type = other DNA
atgcttctcctggtgacaagccttctgctctgtgagttaccacacccagcattcctcctgatcccacgcaaagtgtgtaacggaataggtattggtgaatttaaagactcactctccataaatgctacgaatattaaacacttcaaaaactgcacctccatcagtggcgatctccacatcctgccggtggcatttaggggtgactccttcacacatactcctcctctggatccacaggaactggatattctgaaaaccgtaaaggaaatcacagggtttttgctgattcaggcttggcctgaaaacaggacggacctccatgcctttgagaacctagaaatcatacgcggcaggaccaagcaacatggtcagttttctcttgcagtcgtcagcctgaacataacatccttgggattacgctccctcaaggagataagtgatggagatgtgataatttcaggaaacaaaaatttgtgctatgcaaatacaataaactggaaaaaactgtttgggacctccggtcagaaaaccaaaattataagcaacagaggtgaaaacagctgcaaggccacaggccaggtgtgcaaccatctgtgttccagtgatggctgttggggacctgggccagaccaatgtctgtcgtgtcgccgcttcagtagaggaaggatctgcatagagtcttgtaacctctatgatggtgaatttcgggagtttgagaatggctccatctgtgtggagtgtgacccccagtgtgagaagatggaagatggcctcctcacatgccatggaccgggtcctgacaactgtacaaagtgctctcattttaaagatggcccaaactgtgtggaaaaatgtccagatggcttacagggggcaaacagtttcattttcaagtatgctgatccagatcgggagtgccacccatgccatccaaactgcacccaagggtgtaacggtcccactagtcatgactgcatttactacccatggacgggccattccactttaccacaacatgctagaactcccctgattgcagctggagtaattggtgggctcttcattctggtcattgtgggtctgacatttgctgtttatgtt

SEQ ID NO: 99 - protein, 367 aa, synthetic construct
  REGION 1..367: note = Description of Artificial Sequence: Synthetic polypeptide
MLLLVTSLLLCELPHPAFLLIPRKVCNGIGIGEFKDSLSINATNIKHFKNCTSISGDLHILPVAFRGDSFTHTPPLDPQELDILKTVKEITGFLLIQAWPENRTDLHAFENLEIIRGRTKQHGQFSLAVVSLNITSLGLRSLKEISDGDVIISGNKNLCYANTINWKKLFGTSGQKTKIISNRGENSCKATGQVCNHLCSSDGCWGPGPDQCLSCRRFSRGRICIESCNLYDGEFREFENGSICVECDPQCEKMEDGLLTCHGPGPDNCTKCSHFKDGPNCVEKCPDGLQGANSFIFKYADPDRECHPCHPNCTQGCNGPTSHDCIYYPWTGHSTLPQHARTPLIAAGVIGGLFILVIVGLTFAVYV

SEQ ID NO: 100 - DNA, 1035 bp, synthetic construct
  misc_feature 1..1035: note = Description of Artificial Sequence: Synthetic polynucleotide
  source 1..1035: mol_type = other DNA
cgcaaagtgtgtaacggaataggtattggtgaatttaaagactcactctccataaatgctacgaatattaaacacttcaaaaactgcacctccatcagtggcgatctccacatcctgccggtggcatttaggggtgactccttcacacatactcctcctctggatccacaggaactggatattctgaaaaccgtaaaggaaatcacagggtttttgctgattcaggcttggcctgaaaacaggacggacctccatgcctttgagaacctagaaatcatacgcggcaggaccaagcaacatggtcagttttctcttgcagtcgtcagcctgaacataacatccttgggattacgctccctcaaggagataagtgatggagatgtgataatttcaggaaacaaaaatttgtgctatgcaaatacaataaactggaaaaaactgtttgggacctccggtcagaaaaccaaaattataagcaacagaggtgaaaacagctgcaaggccacaggccaggtgtgcaaccatctgtgttccagtgatggctgttggggacctgggccagaccaatgtctgtcgtgtcgccgcttcagtagaggaaggatctgcatagagtcttgtaacctctatgatggtgaatttcgggagtttgagaatggctccatctgtgtggagtgtgacccccagtgtgagaagatggaagatggcctcctcacatgccatggaccgggtcctgacaactgtacaaagtgctctcattttaaagatggcccaaactgtgtggaaaaatgtccagatggcttacagggggcaaacagtttcattttcaagtatgctgatccagatcgggagtgccacccatgccatccaaactgcacccaagggtgtaacggtcccactagtcatgactgcatttactacccatggacgggccattccactttaccacaacatgctagaactcccctgattgcagctggagtaattggtgggctcttcattctggtcattgtgggtctgacatttgctgtttatgtt

SEQ ID NO: 101 - protein, 345 aa, synthetic construct
  REGION 1..345: note = Description of Artificial Sequence: Synthetic polypeptide
RKVCNGIGIGEFKDSLSINATNIKHFKNCTSISGDLHILPVAFRGDSFTHTPPLDPQELDILKTVKEITGFLLIQAWPENRTDLHAFENLEIIRGRTKQHGQFSLAVVSLNITSLGLRSLKEISDGDVIISGNKNLCYANTINWKKLFGTSGQKTKIISNRGENSCKATGQVCNHLCSSDGCWGPGPDQCLSCRRFSRGRICIESCNLYDGEFREFENGSICVECDPQCEKMEDGLLTCHGPGPDNCTKCSHFKDGPNCVEKCPDGLQGANSFIFKYADPDRECHPCHPNCTQGCNGPTSHDCIYYPWTGHSTLPQHARTPLIAAGVIGGLFILVIVGLTFAVYV

SEQ ID NO: 102 - DNA, 1071 bp, synthetic construct
  misc_feature 1..1071: note = Description of Artificial Sequence: Synthetic polynucleotide
  source 1..1071: mol_type = other DNA
atgcttctcctggtgacaagccttctgctctgtgagttaccacacccagcattcctcctgatcccacgcaaagtgtgtaacggaataggtattggtgaatttaaagactcactctccataaatgctacgaatattaaacacttcaaaaactgcacctccatcagtggcgatctccacatcctgccggtggcatttaggggtgactccttcacacatactcctcctctggatccacaggaactggatattctgaaaaccgtaaaggaaatcacagggtttttgctgattcaggcttggcctgaaaacaggacggacctccatgcctttgagaacctagaaatcatacgcggcaggaccaagcaacatggtcagttttctcttgcagtcgtcagcctgaacataacatccttgggattacgctccctcaaggagataagtgatggagatgtgataatttcaggaaacaaaaatttgtgctatgcaaatacaataaactggaaaaaactgtttgggacctccggtcagaaaaccaaaattataagcaacagaggtgaaaacagctgcaaggccacaggccaggtgtgcaaccatctgtgttccagtgatggctgttggggacctgggccagaccaatgtctgtcgtgtcgccgcttcagtagaggaaggatctgcatagagtcttgtaacctctatgatggtgaatttcgggagtttgagaatggctccatctgtgtggagtgtgacccccagtgtgagaagatggaagatggcctcctcacatgccatggaccgggtcctgacaactgtacaaagtgctctcattttaaagatggcccaaactgtgtggaaaaatgtccagatggcttacagggggcaaacagtttcattttcaagtatgctgatccagatcgggagtgccacccatgccatccaaactgcacccaagggtgcataggctcaagtattgaagactgcatcggcctgatggatagaactcccctgattgcagctggagtaattggtgggctcttcattctggtcattgtgggtctgacatttgctgtttatgtt

SEQ ID NO: 103 - protein, 357 aa, synthetic construct
  REGION 1..357: note = Description of Artificial Sequence: Synthetic polypeptide
MLLLVTSLLLCELPHPAFLLIPRKVCNGIGIGEFKDSLSINATNIKHFKNCTSISGDLHILPVAFRGDSFTHTPPLDPQELDILKTVKEITGFLLIQAWPENRTDLHAFENLEIIRGRTKQHGQFSLAVVSLNITSLGLRSLKEISDGDVIISGNKNLCYANTINWKKLFGTSGQKTKIISNRGENSCKATGQVCNHLCSSDGCWGPGPDQCLSCRRFSRGRICIESCNLYDGEFREFENGSICVECDPQCEKMEDGLLTCHGPGPDNCTKCSHFKDGPNCVEKCPDGLQGANSFIFKYADPDRECHPCHPNCTQGCIGSSIEDCIGLMDRTPLIAAGVIGGLFILVIVGLTFAVYV

SEQ ID NO: 104 - DNA, 1005 bp, synthetic construct
  misc_feature 1..1005: note = Description of Artificial Sequence: Synthetic polynucleotide
  source 1..1005: mol_type = other DNA
cgcaaagtgtgtaacggaataggtattggtgaatttaaagactcactctccataaatgctacgaatattaaacacttcaaaaactgcacctccatcagtggcgatctccacatcctgccggtggcatttaggggtgactccttcacacatactcctcctctggatccacaggaactggatattctgaaaaccgtaaaggaaatcacagggtttttgctgattcaggcttggcctgaaaacaggacggacctccatgcctttgagaacctagaaatcatacgcggcaggaccaagcaacatggtcagttttctcttgcagtcgtcagcctgaacataacatccttgggattacgctccctcaaggagataagtgatggagatgtgataatttcaggaaacaaaaatttgtgctatgcaaatacaataaactggaaaaaactgtttgggacctccggtcagaaaaccaaaattataagcaacagaggtgaaaacagctgcaaggccacaggccaggtgtgcaaccatctgtgttccagtgatggctgttggggacctgggccagaccaatgtctgtcgtgtcgccgcttcagtagaggaaggatctgcatagagtcttgtaacctctatgatggtgaatttcgggagtttgagaatggctccatctgtgtggagtgtgacccccagtgtgagaagatggaagatggcctcctcacatgccatggaccgggtcctgacaactgtacaaagtgctctcattttaaagatggcccaaactgtgtggaaaaatgtccagatggcttacagggggcaaacagtttcattttcaagtatgctgatccagatcgggagtgccacccatgccatccaaactgcacccaagggtgcataggctcaagtattgaagactgcatcggcctgatggatagaactcccctgattgcagctggagtaattggtgggctcttcattctggtcattgtgggtctgacatttgctgtttatgtt

SEQ ID NO: 105 - protein, 335 aa, synthetic construct
  REGION 1..335: note = Description of Artificial Sequence: Synthetic polypeptide
RKVCNGIGIGEFKDSLSINATNIKHFKNCTSISGDLHILPVAFRGDSFTHTPPLDPQELDILKTVKEITGFLLIQAWPENRTDLHAFENLEIIRGRTKQHGQFSLAVVSLNITSLGLRSLKEISDGDVIISGNKNLCYANTINWKKLFGTSGQKTKIISNRGENSCKATGQVCNHLCSSDGCWGPGPDQCLSCRRFSRGRICIESCNLYDGEFREFENGSICVECDPQCEKMEDGLLTCHGPGPDNCTKCSHFKDGPNCVEKCPDGLQGANSFIFKYADPDRECHPCHPNCTQGCIGSSIEDCIGLMDRTPLIAAGVIGGLFILVIVGLTFAVYV

SEQ ID NO: 106 - DNA, 891 bp, unidentified
  misc_feature 1..891: note = Description of Unknown: Full length CD20 sequence
  source 1..891: mol_type = genomic DNA
atgacaacacccagaaattcagtaaatgggactttcccggcagagccaatgaaaggccctattgctatgcaatctggtccaaaaccactcttcaggaggatgtcttcactggtgggccccacgcaaagcttcttcatgagggaatctaagactttgggggctgtccagattatgaatgggctcttccacattgccctggggggtcttctgatgatcccagcagggatctatgcacccatctgtgtgactgtgtggtaccctctctggggaggcattatgtatattatttccggatcactcctggcagcaacggagaaaaactccaggaagtgtttggtcaaaggaaaaatgataatgaattcattgagcctctttgctgccatttctggaatgattctttcaatcatggacatacttaatattaaaatttcccattttttaaaaatggagagtctgaattttattagagctcacacaccatatattaacatatacaactgtgaaccagctaatccctctgagaaaaactccccatctacccaatactgttacagcatacaatctctgttcttgggcattttgtcagtgatgctgatctttgccttcttccaggaacttgtaatagctggcatcgttgagaatgaatggaaaagaacgtgctccagacccaaatctaacatagttctcctgtcagcagaagaaaaaaaagaacagactattgaaataaaagaagaagtggttgggctaactgaaacatcttcccaaccaaagaatgaagaagacattgaaattattccaatccaagaagaggaagaagaagaaacagagacgaactttccagaacctccccaagatcaggaatcctcaccaatagaaaatgacagctctcct

SEQ ID NO: 107 - protein, 297 aa, unidentified
  REGION 1..297: note = Description of Unknown: Full length CD20 sequence
MTTPRNSVNGTFPAEPMKGPIAMQSGPKPLFRRMSSLVGPTQSFFMRESKTLGAVQIMNGLFHIALGGLLMIPAGIYAPICVTVWYPLWGGIMYIISGSLLAATEKNSRKCLVKGKMIMNSLSLFAAISGMILSIMDILNIKISHFLKMESLNFIRAHTPYINIYNCEPANPSEKNSPSTQYCYSIQSLFLGILSVMLIFAFFQELVIAGIVENEWKRTCSRPKSNIVLLSAEEKKEQTIEIKEEVVGLTETSSQPKNEEDIEIIPIQEEEEEETETNFPEPPQDQESSPIENDSSP

SEQ ID NO: 108 - DNA, 789 bp, synthetic construct
  misc_feature 1..789: note = Description of Artificial Sequence: Synthetic polynucleotide
  source 1..789: mol_type = other DNA
atgaccacaccacggaactctgtgaatggcaccttcccagcagagccaatgaagggaccaatcgcaatgcagagcggacccaagcctctgtttcggagaatgagctccctggtgggcccaacccagtccttctttatgagagagtctaagacactgggcgccgtgcagatcatgaacggactgttccacatcgccctgggaggactgctgatgatcccagccggcatctacgcccctatctgcgtgaccgtgtggtaccctctgtggggcggcatcatgtatatcatctccggctctctgctggccgccacagagaagaacagcaggaagtgtctggtgaagggcaagatgatcatgaatagcctgtccctgtttgccgccatctctggcatgatcctgagcatcatggacatcctgaacatcaagatcagccacttcctgaagatggagagcctgaacttcatcagagcccacaccccttacatcaacatctataattgcgagcctgccaacccatccgagaagaattctccaagcacacagtactgttattccatccagtctctgttcctgggcatcctgtctgtgatgctgatctttgccttctttcaggagctggtcatcgccggcatcgtggagaacgagtggaagaggacctgcagccgccccaagtccaatatcgtgctgctgtccgccgaggagaagaaggagcagacaatcgagatcaaggaggaggtggtgggcctgaccgagacatctagccagcctaagaatgaggaggatatcgag

SEQ ID NO: 109 - protein, 263 aa, synthetic construct
  REGION 1..263: note = Description of Artificial Sequence: Synthetic polypeptide
MTTPRNSVNGTFPAEPMKGPIAMQSGPKPLFRRMSSLVGPTQSFFMRESKTLGAVQIMNGLFHIALGGLLMIPAGIYAPICVTVWYPLWGGIMYIISGSLLAATEKNSRKCLVKGKMIMNSLSLFAAISGMILSIMDILNIKISHFLKMESLNFIRAHTPYINIYNCEPANPSEKNSPSTQYCYSIQSLFLGILSVMLIFAFFQELVIAGIVENEWKRTCSRPKSNIVLLSAEEKKEQTIEIKEEVVGLTETSSQPKNEEDIE

SEQ ID NO: 110 - DNA, 294 bp, synthetic construct
  misc_feature 1..294: note = Description of Artificial Sequence: Synthetic polynucleotide
  source 1..294: mol_type = other DNA
atgataatgaattcattgagcctctttgctgccatttctggaatgattctttcaatcatggacatacttaatattaaaatttcccattttttaaaaatggagagtctgaattttattagagctcacacaccatatattaacatatacaactgtgaaccagctaatccctctgagaaaaactccccatctacccaatactgttacagcatacaatctctgttcttgggcattttgtcagtgatgctgatctttgccttcttccaggaacttgtaatagctggcatcgttgagaat

SEQ ID NO: 111 - protein, 98 aa, synthetic construct
  REGION 1..98: note = Description of Artificial Sequence: Synthetic polypeptide
MIMNSLSLFAAISGMILSIMDILNIKISHFLKMESLNFIRAHTPYINIYNCEPANPSEKNSPSTQYCYSIQSLFLGILSVMLIFAFFQELVIAGIVEN

SEQ ID NO: 112 - DNA, 267 bp, synthetic construct
  misc_feature 1..267: note = Description of Artificial Sequence: Synthetic polynucleotide
  source 1..267: mol_type = other DNA
atggccttaccagtgaccgccttgctcctgccgctggccttgctgctccacgccgccaggccgaaaatttcccattttttaaaaatggagagtctgaattttattagagctcacacaccatatattaacatatacaactgtgaaccagctaatccctctgagaaaaactccccatctacccaatactgttacagcatacaatctatctacatctgggcgcccttggccgggacttgtggggtccttctcctgtcactggttatcacc

SEQ ID NO: 113 - protein, 89 aa, synthetic construct
  REGION 1..89: note = Description of Artificial Sequence: Synthetic polypeptide
MALPVTALLLPLALLLHAARPKISHFLKMESLNFIRAHTPYINIYNCEPANPSEKNSPSTQYCYSIQSIYIWAPLAGTCGVLLLSLVIT

SEQ ID NO: 114 - DNA, 642 bp, synthetic construct
  misc_feature 1..642: note = Description of Artificial Sequence: Synthetic polynucleotide
  source 1..642: mol_type = other DNA
atgacaacacccagaaattcagtaaatgggactttcccggcagagccaatgaaaggccctattgctatgcaatctggtccaaaaccactcttcaggaggatgtcttcactggtgggccccacgcaaagcttcttcatgagggaatctaagactttgggggctgtccagattatgaatgggctcttccacattgccctggggggtcttctgatgatcccagcagggatctatgcacccatctgtgtgactgtgtggtaccctctctggggaggcattatgtatattatttccggatcactcctggcagcaacggagaaaaactccaggaagtgtttggtcaaaggaaaaatgataatgaattcattgagcctctttgctgccatttctggaatgattctttcaatcatggacatacttaatattaaaatttcccattttttaaaaatggagagtctgaattttattagagctcacacaccatatattaacatatacaactgtgaaccagctaatccctctgagaaaaactccccatctacccaatactgttacagcatacaatctctgttcttgggcattttgtcagtgatgctgatctttgccttcttccaggaacttgtaatagctggcatcgttgagaat

SEQ ID NO: 115 - protein, 214 aa, synthetic construct
  REGION 1..214: note = Description of Artificial Sequence: Synthetic polypeptide
MTTPRNSVNGTFPAEPMKGPIAMQSGPKPLFRRMSSLVGPTQSFFMRESKTLGAVQIMNGLFHIALGGLLMIPAGIYAPICVTVWYPLWGGIMYIISGSLLAATEKNSRKCLVKGKMIMNSLSLFAAISGMILSIMDILNIKISHFLKMESLNFIRAHTPYINIYNCEPANPSEKNSPSTQYCYSIQSLFLGILSVMLIFAFFQELVIAGIVEN

SEQ ID NO: 116 - DNA, 399 bp, synthetic construct
  misc_feature 1..399: note = Description of Artificial Sequence: Synthetic polynucleotide
  source 1..399: mol_type = other DNA
gtgactgtgtggtaccctctctggggaggcattatgtatattatttccggatcactcctggcagcaacggagaaaaactccaggaagtgtttggtcaaaggaaaaatgataatgaattcattgagcctctttgctgccatttctggaatgattctttcaatcatggacatacttaatattaaaatttcccattttttaaaaatggagagtctgaattttattagagctcacacaccatatattaacatatacaactgtgaaccagctaatccctctgagaaaaactccccatctacccaatactgttacagcatacaatctctgttcttgggcattttgtcagtgatgctgatctttgccttcttccaggaacttgtaatagctggcatcgttgagaat

SEQ ID NO: 117 - protein, 133 aa, synthetic construct
  REGION 1..133: note = Description of Artificial Sequence: Synthetic polypeptide
VTVWYPLWGGIMYIISGSLLAATEKNSRKCLVKGKMIMNSLSLFAAISGMILSIMDILNIKISHFLKMESLNFIRAHTPYINIYNCEPANPSEKNSPSTQYCYSIQSLFLGILSVMLIFAFFQELVIAGIVEN

SEQ ID NO: 118 - DNA, 315 bp, synthetic construct
  misc_feature 1..315: note = Description of Artificial Sequence: Synthetic polynucleotide
  source 1..315: mol_type = other DNA
gtgactgtgtggtaccctctctggggaggcattatgtatattatttccggatcactcctggcagcaacggagaaaaactccaggaagtgtttggtcaaaggaaaaatgataatgaattcattgagcctctttgctgccatttctggaatgattctttcaatcatggacatacttaatattaaaatttcccattttttaaaaatggagagtctgaattttattagagctcacacaccatatattaacatatacaactgtgaaccagctaatccctctgagaaaaactccccatctacccaatactgttacagcata

SEQ ID NO: 119 - protein, 133 aa, synthetic construct; identical to SEQ ID NO: 117
  REGION 1..133: note = Description of Artificial Sequence: Synthetic polypeptide

SEQ ID NO: 120 - DNA, 333 bp, synthetic construct
  misc_feature 1..333: note = Description of Artificial Sequence: Synthetic polynucleotide
  source 1..333: mol_type = other DNA
ccatatattaacatatacaactgtgaaccagctaatccctctgagaaaaactccccatctacccaatactgttacagcatacaatcgggtggcggcggatctattgaagttatgtatcctcctccttacctagacaatgagaagagcaatggaaccattatccatgtgaaagggaaacacctttgtccaagtcccctatttcccggaccttctaagcccttttgggtgctggtggtggttggtggagtcctggcttgctatagcttgctagtaacagtggcctttattattttctgggtgaggagtaagaggagcaggctcctgcacagtgac

SEQ ID NO: 121 - protein, 111 aa, synthetic construct
  REGION 1..111: note = Description of Artificial Sequence: Synthetic polypeptide
PYINIYNCEPANPSEKNSPSTQYCYSIQSGGGGSIEVMYPPPYLDNEKSNGTIIHVKGKHLCPSPLFPGPSKPFWVLVVVGGVLACYSLLVTVAFIIFWVRSKRSRLLHSD

SEQ ID NO: 122 - DNA, 435 bp, synthetic construct
  misc_feature 1..435: note = Description of Artificial Sequence: Synthetic polynucleotide
  source 1..435: mol_type = other DNA
ccatatattaacatatacaactgtgaaccagctaatccctctgagaaaaactccccatctacccaatactgttacagcatacaatcgggtggcggcggatctccatatattaacatatacaactgtgaaccagctaatccctctgagaaaaactccccatctacccaatactgttacagcatacaatcgggtggcggcggatctattgaagttatgtatcctcctccttacctagacaatgagaagagcaatggaaccattatccatgtgaaagggaaacacctttgtccaagtcccctatttcccggaccttctaagcccttttgggtgctggtggtggttggtggagtcctggcttgctatagcttgctagtaacagtggcctttattattttctgggtgaggagtaagaggagcaggctcctgcacagtgac

SEQ ID NO: 123 - protein, 145 aa, synthetic construct
  REGION 1..145: note = Description of Artificial Sequence: Synthetic polypeptide
PYINIYNCEPANPSEKNSPSTQYCYSIQSGGGGSPYINIYNCEPANPSEKNSPSTQYCYSIQSGGGGSIEVMYPPPYLDNEKSNGTIIHVKGKHLCPSPLFPGPSKPFWVLVVVGGVLACYSLLVTVAFIIFWVRSKRSRLLHSD

SEQ ID NO: 124 - DNA, 348 bp, synthetic construct
  misc_feature 1..348: note = Description of Artificial Sequence: Synthetic polynucleotide
  source 1..348: mol_type = other DNA
ccatatattaacatatacaactgtgaaccagctaatccctctgagaaaaactccccatctacccaatactgttacagcatacaatcgggtggcggcggatctccagcgccgcgaccaccaacaccggcgcccaccatcgcgtcgcagcccctgtccctgcgcccagaggcgtgccggccagcggcggggggcgcagtgcacacgagggggctggacttcgcctgtgatatctacatctgggcgcccttggccgggacttgtggggtccttctcctgtcactggttatcaccctttactgcaaccacaggaaccgaagacgtgtttgcaaatgtccccggcctgtggtc

SEQ ID NO: 125 - protein, 116 aa, synthetic construct
  REGION 1..116: note = Description of Artificial Sequence: Synthetic polypeptide
PYINIYNCEPANPSEKNSPSTQYCYSIQSGGGGSPAPRPPTPAPTIASQPLSLRPEACRPAAGGAVHTRGLDFACDIYIWAPLAGTCGVLLLSLVITLYCNHRNRRRVCKCPRPVV

SEQ ID NO: 126 - DNA, 300 bp, synthetic construct
  misc_feature 1..300: note = Description of Artificial Sequence: Synthetic polynucleotide
  source 1..300: mol_type = other DNA
tgtgaaccagctaatccctctgagaaaaactccccatctacccaatactgttcgggtggcggcggatctattgaagttatgtatcctcctccttacctagacaatgagaagagcaatggaaccattatccatgtgaaagggaaacacctttgtccaagtcccctatttcccggaccttctaagcccttttgggtgctggtggtggttggtggagtcctggcttgctatagcttgctagtaacagtggcctttattattttctgggtgaggagtaagaggagcaggctcctgcacagtgac

SEQ ID NO: 127 - protein, 100 aa, synthetic construct
  REGION 1..100: note = Description of Artificial Sequence: Synthetic polypeptide
CEPANPSEKNSPSTQYCSGGGGSIEVMYPPPYLDNEKSNGTIIHVKGKHLCPSPLFPGPSKPFWVLVVVGGVLACYSLLVTVAFIIFWVRSKRSRLLHSD

SEQ ID NO: 128 - DNA, 369 bp, synthetic construct
  misc_feature 1..369: note = Description of Artificial Sequence: Synthetic polynucleotide
  source 1..369: mol_type = other DNA
tgtgaaccagctaatccctctgagaaaaactccccatctacccaatactgttcgggtggcggcggatcttgtgaaccagctaatccctctgagaaaaactccccatctacccaatactgttcgggtggcggcggatctattgaagttatgtatcctcctccttacctagacaatgagaagagcaatggaaccattatccatgtgaaagggaaacacctttgtccaagtcccctatttcccggaccttctaagcccttttgggtgctggtggtggttggtggagtcctggcttgctatagcttgctagtaacagtggcctttattattttctgggtgaggagtaagaggagcaggctcctgcacagtgac

SEQ ID NO: 129 - protein, 123 aa, synthetic construct
  REGION 1..123: note = Description of Artificial Sequence: Synthetic polypeptide
CEPANPSEKNSPSTQYCSGGGGSCEPANPSEKNSPSTQYCSGGGGSIEVMYPPPYLDNEKSNGTIIHVKGKHLCPSPLFPGPSKPFWVLVVVGGVLACYSLLVTVAFIIFWVRSKRSRLLHSD

SEQ ID NO: 130 - DNA, 315 bp, synthetic construct
  misc_feature 1..315: note = Description of Artificial Sequence: Synthetic polynucleotide
  source 1..315: mol_type = other DNA
tgtgaaccagctaatccctctgagaaaaactccccatctacccaatactgttcgggtggcggcggatctccagcgccgcgaccaccaacaccggcgcccaccatcgcgtcgcagcccctgtccctgcgcccagaggcgtgccggccagcggcggggggcgcagtgcacacgagggggctggacttcgcctgtgatatctacatctgggcgcccttggccgggacttgtggggtccttctcctgtcactggttatcaccctttactgcaaccacaggaaccgaagacgtgtttgcaaatgtccccggcctgtggtc

SEQ ID NO: 131 - protein, 105 aa, synthetic construct
  REGION 1..105: note = Description of Artificial Sequence: Synthetic polypeptide
CEPANPSEKNSPSTQYCSGGGGSPAPRPPTPAPTIASQPLSLRPEACRPAAGGAVHTRGLDFACDIYIWAPLAGTCGVLLLSLVITLYCNHRNRRRVCKCPRPVV

SEQ ID NO: 132 - DNA, 729 bp, synthetic construct
  misc_feature 1..729: note = Description of Artificial Sequence: Synthetic polynucleotide
  source 1..729: mol_type = other DNA
atgaccacaccccggaactccgtgaatggcaccttccctgccgagccaatgaagggccctatcgccatgcagtctggcccaaagcccctgtttcggagaatgagctccctggtgggccccacccagagcttctttatgagggagtccaagacactgggcgcctgcctggtgaagggcaagatgatcatgaactctctgagcctgttcgccgccatctccggcatgatcctgtctatcatggacatcctgaacatcaagatctctcacttcctgaagatggagagcctgaacttcatccgggcccacaccccatacatcaacatctataattgcgagcccgccaaccctagcgagaagaattccccctctacacagtactgttatagcatccagtccctgttcctgggcatcctgtccgtgatgctgatctttgccttctttcaggagctggtcatcgccggcatcgtggagaacgagtggaagaggacctgttctcgccctaagagcaatatcgtgctgctgagcgccgaggagaagaaggagcagacaatcgagatcaaggaggaggtggtgggcctgaccgagacatctagccagcctaagaatgaggaggatatcgagatcatcccaatccaggaggaggaggaggaggagaccgagacaaactttccagagccccctcaggaccaggagtcctctccaatcgagaatgatagctccccctgataa

SEQ ID NO: 133 - protein, 240 aa, synthetic construct
  REGION 1..240: note = Description of Artificial Sequence: Synthetic polypeptide
MTTPRNSVNGTFPAEPMKGPIAMQSGPKPLFRRMSSLVGPTQSFFMRESKTLGACLVKGKMIMNSLSLFAAISGMILSIMDILNIKISHFLKMESLNFIRAHTPYINIYNCEPANPSEKNSPSTQYCYSIQSLFLGILSVMLIFAFFQELVIAGIVENEWKRTCSRPKSNIVLLSAEEKKEQTIEIKEEVVGLTETSSQPKNEEDIEIIPIQEEEEEETETNFPEPPQDQESSPIENDSS

SEQ ID NO: 134 - DNA, 681 bp, synthetic construct
  misc_feature 1..681: note = Description of Artificial Sequence: Synthetic polynucleotide
  source 1..681: mol_type = other DNA
atgaccacaccacggaacagcgtgaatggcaccttcccagcagagccaatgaagggaccaatcgcaatgcagtccggacccaagcctctgtttcggagaatgagctccctggtgggccccacccagtctttctttatgagggagagcaagacactgggcgcctgcctggtgaagggcaagatgatcatgaactccctgtctctgttcgccgccatcagcggcatgatcctgtccatcatggacatcctgaacatcaagatctcccacttcctgaagatggagagcctgaacttcatccgggcccacaccccttacatcaacatctataattgcgagcctgccaacccatctgagaagaatagcccatccacacagtactgttattctatccagagcctgttcctgggcatcctgtccgtgatgctgatctttgccttctttcaggagctggtcatcgccggcatcgtggagaacgagtggaagaggacctgttcccgccccaagtctaatatcgtgctgctgagcgccgaggagaagaaggagcagacaatcgagatcaaggaggaggtggtgggcctgaccgagacatctagccagcccaagaacgaggaggatatcgagatcatccctatccaggaggaggaggaggaggagaccgagacaaattttcctgagtgataa

SEQ ID NO: 135 - protein, 225 aa, synthetic construct
  REGION 1..225: note = Description of Artificial Sequence: Synthetic polypeptide
MTTPRNSVNGTFPAEPMKGPIAMQSGPKPLFRRMSSLVGPTQSFFMRESKTLGACLVKGKMIMNSLSLFAAISGMILSIMDILNIKISHFLKMESLNFIRAHTPYINIYNCEPANPSEKNSPSTQYCYSIQSLFLGILSVMLIFAFFQELVIAGIVENEWKRTCSRPKSNIVLLSAEEKKEQTIEIKEEVVGLTETSSQPKNEEDIEIIPIQEEEEEETETNFPE

SEQ ID NO: 136 - DNA, 627 bp, synthetic construct
  misc_feature 1..627: note = Description of Artificial Sequence: Synthetic polynucleotide
  source 1..627: mol_type = other DNA
atgaccacaccccggaacagcgtgaatggcaccttcccagccgagcccatgaagggccctatcgccatgcagtccggccccaagcctctgtttcggagaatgagctccctggtgggccccacccagtctttctttatgagggagagcaagacactgggcgcctgcctggtgaagggcaagatgatcatgaactccctgtctctgttcgccgccatcagcggcatgatcctgtccatcatggacatcctgaacatcaagatctcccacttcctgaagatggagagcctgaacttcatccgggcccacaccccatacatcaacatctataattgcgagcctgccaacccatctgagaagaatagcccctccacacagtactgttattctatccagagcctgttcctgggcatcctgtccgtgatgctgatctttgccttctttcaggagctggtcatcgccggcatcgtggagaacgagtggaagaggacctgttcccgccctaagtctaatatcgtgctgctgagcgccgaggagaagaaggagcagacaatcgagatcaaggaggaggtggtgggcctgaccgagacatctagccagccaaagaatgaggaggatatcgagtgataa

SEQ ID NO: 137 - protein, 207 aa, synthetic construct
  REGION 1..207: note = Description of Artificial Sequence: Synthetic polypeptide
MTTPRNSVNGTFPAEPMKGPIAMQSGPKPLFRRMSSLVGPTQSFFMRESKTLGACLVKGKMIMNSLSLFAAISGMILSIMDILNIKISHFLKMESLNFIRAHTPYINIYNCEPANPSEKNSPSTQYCYSIQSLFLGILSVMLIFAFFQELVIAGIVENEWKRTCSRPKSNIVLLSAEEKKEQTIEIKEEVVGLTETSSQPKNEEDIE

SEQ ID NO: 138 - DNA, 522 bp, synthetic construct
  misc_feature 1..522: note = Description of Artificial Sequence: Synthetic polynucleotide
  source 1..522: mol_type = other DNA
atgaccacaccccggaactccgtgaatggcaccttcccagccgagcccatgaagggccctatcgccatgcagtctggccccaagcctctgtttcggagaatgagctccctggtgggccctacccagagcttctttatgagggagtccaagacactgggcgcctgcctggtgaagggcaagatgatcatgaactctctgagcctgttcgccgccatctccggcatgatcctgtctatcatggacatcctgaacatcaagatctctcacttcctgaagatggagagcctgaacttcatccgggcccacaccccatacatcaacatctataattgcgagcctgccaacccaagcgagaagaattccccctctacacagtactgttatagcatccagtccctgttcctgggcatcctgtccgtgatgctgatctttgccttctttcaggagctggtcatcgccggcatcgtggagaacgagtggaagaggacatgttctcgccccaagagcaatatcgtgtgataa

SEQ ID NO: 139 - protein, 172 aa, synthetic construct
  REGION 1..172: note = Description of Artificial Sequence: Synthetic polypeptide
MTTPRNSVNGTFPAEPMKGPIAMQSGPKPLFRRMSSLVGPTQSFFMRESKTLGACLVKGKMIMNSLSLFAAISGMILSIMDILNIKISHFLKMESLNFIRAHTPYINIYNCEPANPSEKNSPSTQYCYSIQSLFLGILSVMLIFAFFQELVIAGIVENEWKRTCSRPKSNIV

SEQ ID NO: 140 - DNA, 591 bp, synthetic construct
  misc_feature 1..591: note = Description of Artificial Sequence: Synthetic polynucleotide
  source 1..591: mol_type = other DNA
atgaccacacccaggaacagcgtgtgcctggtgaagggcaagatgatcatgaatagcctgtccctgttcgccgccatctctggcatgatcctgagcatcatggacatcctgaacatcaagatctcccacttcctgaagatggagagcctgaacttcatccgggcccacaccccatacatcaacatctataattgcgagccagccaaccccagcgagaagaattctcccagcacacagtactgttattccatccagtctctgttcctgggcatcctgtccgtgatgctgatctttgccttctttcaggagctggtcatcgccggcatcgtggagaacgagtggaagcggacctgtagcagacctaagtccaatatcgtgctgctgtccgccgaggagaagaaggagcagacaatcgagatcaaggaggaggtggtgggcctgaccgagacaagctcccagcccaagaacgaggaggatatcgagatcatccctatccaggaggaggaggaggaggagaccgagacaaactttccagagccccctcaggaccaggagtctagccctatcgagaatgattcctctccatgataa

SEQ ID NO: 141 - protein, 195 aa, synthetic construct
  REGION 1..195: note = Description of Artificial Sequence: Synthetic polypeptide
MTTPRNSVCLVKGKMIMNSLSLFAAISGMILSIMDILNIKISHFLKMESLNFIRAHTPYINIYNCEPANPSEKNSPSTQYCYSIQSLFLGILSVMLIFAFFQELVIAGIVENEWKRTCSRPKSNIVLLSAEEKKEQTIEIKEEVVGLTETSSQPKNEEDIEIIPIQEEEEEETETNFPEPPQDQESSPIENDSSP

SEQ ID NO: 142 - DNA, 36 bp, synthetic construct
  misc_feature 1..36: note = Description of Artificial Sequence: Synthetic oligonucleotide
  source 1..36: mol_type = other DNA
ggacaaaacgacaccagccaaaccagcagcccctca

SEQ ID NO: 143 - protein, 12 aa, synthetic construct
  REGION 1..12: note = Description of Artificial Sequence: Synthetic peptide
GQNDTSQTSSPS

SEQ ID NO: 144 - DNA, 279 bp, synthetic construct
  misc_feature 1..279: note = Description of Artificial Sequence: Synthetic polynucleotide
  source 1..279: mol_type = other DNA
atgaagcgcttcctcttcctcctactcaccatcagcctcctggttatggtacagatacaaactggactctcaggacaaaacgacaccagccaaaccagcagcccctcaggcagcacctccggcagcggcaagcctggcagcggcgagggcagcaccaagggcggcggaggcggaagcggaggcggaggctccaagcccttctgggtgctggtcgtggtcggcggagtgctggcctgttacagcctgctggtcaccgtggccttcatcatcttttgggtc

SEQ ID NO: 145 - protein, 93 aa, synthetic construct
  REGION 1..93: note = Description of Artificial Sequence: Synthetic polypeptide
MKRFLFLLLTISLLVMVQIQTGLSGQNDTSQTSSPSGSTSGSGKPGSGEGSTKGGGGGSGGGGSKPFWVLVVVGGVLACYSLLVTVAFIIFWV

SEQ ID NO: 146 - DNA, 369 bp, synthetic construct
  misc_feature 1..369: note = Description of Artificial Sequence: Synthetic polynucleotide
  source 1..369: mol_type = other DNA
atgaagcgcttcctcttcctcctactcaccatcagcctcctggttatggtacagatacaaactggactctcaggacaaaacgacaccagccaaaccagcagcccctcaggcagcacctccggcagcggcaagcctggcagcggcgagggcagcaccaagggcggccagaatgatacatctcagacttcatctcctagcggatccacttctggttccggtaaaccaggttctggggaaggtagtacaaaaggaggcggaggcggaagcggaggcggaggctccaagcccttctgggtgctggtcgtggtcggcggagtgctggcctgttacagcctgctggtcaccgtggccttcatcatcttttgggtc

SEQ ID NO: 147 - protein, 123 aa, synthetic construct
  REGION 1..123: note = Description of Artificial Sequence: Synthetic polypeptide
MKRFLFLLLTISLLVMVQIQTGLSGQNDTSQTSSPSGSTSGSGKPGSGEGSTKGGQNDTSQTSSPSGSTSGSGKPGSGEGSTKGGGGGSGGGGSKPFWVLVVVGGVLACYSLLVTVAFIIFWV

SEQ ID NO: 148 - DNA, 459 bp, synthetic construct
  misc_feature 1..459: note = Description of Artificial Sequence: Synthetic polynucleotide
  source 1..459: mol_type = other DNA
atgaagcgcttcctcttcctcctactcaccatcagcctcctggttatggtacagatacaaactggactctcaggacaaaacgacaccagccaaaccagcagcccctcaggcagcacctccggcagcggcaagcctggcagcggcgagggcagcaccaagggcggccagaatgatacatctcagacttcatctcctagcggatccacttctggttccggtaaaccaggttctggggaaggtagtacaaaaggaggtcagaacgacacttcacagacatctagtccatccggcagtacaagcggaagtggaaagcccggaagtggtgagggatcaactaagggtggcggaggcggaagcggaggcggaggctccaagcccttctgggtgctggtcgtggtcggcggagtgctggcctgttacagcctgctggtcaccgtggccttcatcatcttttgggtc

SEQ ID NO: 149 - protein, 153 aa, synthetic construct
  REGION 1..153: note = Description of Artificial Sequence: Synthetic polypeptide
MKRFLFLLLTISLLVMVQIQTGLSGQNDTSQTSSPSGSTSGSGKPGSGEGSTKGGQNDTSQTSSPSGSTSGSGKPGSGEGSTKGGQNDTSQTSSPSGSTSGSGKPGSGEGSTKGGGGGSGGGGSKPFWVLVVVGGVLACYSLLVTVAFIIFWV

SEQ ID NO: 150 - protein, 163 aa, synthetic construct
  REGION 1..163: note = Description of Artificial Sequence: Synthetic polypeptide
MKRFLFLLLTISLLVMVQIQTGLSGQNDTSQTSSPSGSTSGSGKPGSGEGSTKGGQNDTSQTSSPSGSTSGSGKPGSGEGSTKGGQNDTSQTSSPSGSTSGSGKPGSGEGSTKGGGGSGGGGSGGGGSGGGGSEITLIIFGVMAGVIGTILLISYGIRRGGGS

SEQ ID NO: 151 - protein, 160 aa, synthetic construct
  REGION 1..160: note = Description of Artificial Sequence: Synthetic polypeptide
MKRFLFLLLTISLLVMVQIQTGLSGQNDTSQTSSPSGSTSGSGKPGSGEGSTKGGQNDTSQTSSPSGSTSGSGKPGSGEGSTKGGQNDTSQTSSPSGSTSGSGKPGSGEGSTKGGGGSGGGGSGGGGSGGGGSITLIIFGVMAGVIGTILLALLIWGGGS

SEQ ID NO: 152 - protein, 160 aa, synthetic construct; identical to SEQ ID NO: 151
  REGION 1..160: note = Description of Artificial Sequence: Synthetic polypeptide

SEQ ID NO: 153 - DNA, 1284 bp, unidentified
  misc_feature 1..1284: note = Description of Unknown: Low-affinity nerve growth factor receptor (LNGFR, TNFRSF16) sequence
  source 1..1284: mol_type = genomic DNA
atgggggcaggtgccaccggccgcgccatggacgggccgcgcctgctgctgttgctgcttctgggggtgtcccttggaggtgccaaggaggcatgccccacaggcctgtacacacacagcggtgagtgctgcaaagcctgcaacctgggcgagggtgtggcccagccttgtggagccaaccagaccgtgtgtgagccctgcctggacagcgtgacgttctccgacgtggtgagcgcgaccgagccgtgcaagccgtgcaccgagtgcgtggggctccagagcatgtcggcgccgtgcgtggaggccgacgacgccgtgtgccgctgcgcctacggctactaccaggatgagacgactgggcgctgcgaggcgtgccgcgtgtgcgaggcgggctcgggcctcgtgttctcctgccaggacaagcagaacaccgtgtgcgaggagtgccccgacggcacgtattccgacgaggccaaccacgtggacccgtgcctgccctgcaccgtgtgcgaggacaccgagcgccagctccgcgagtgcacacgctgggccgacgccgagtgcgaggagatccctggccgttggattacacggtccacacccccagagggctcggacagcacagcccccagcacccaggagcctgaggcacctccagaacaagacctcatagccagcacggtggcaggtgtggtgaccacagtgatgggcagctcccagcccgtggtgacccgaggcaccaccgacaacctcatccctgtctattgctccatcctggctgctgtggttgtgggccttgtggcctacatagccttcaagaggtggaacagctgcaagcagaacaagcaaggagccaacagccggccagtgaaccagacgcccccaccagagggagaaaaactccacagcgacagtggcatctccgtggacagccagagcctgcatgaccagcagccccacacgcagacagcctcgggccaggccctcaagggtgacggaggcctctacagcagcctgcccccagccaagcgggaggaggtggagaagcttctcaacggctctgcgggggacacctggcggcacctggcgggcgagctgggctaccagcccgagcacatagactcctttacccatgaggcctgccccgttcgcgccctgcttgcaagctgggccacccaggacagcgccacactggacgccctcctggccgccctgcgccgcatccagcgagccgacctcgtggagagtctgtgcagtgagtccactgccacatccccggtgtga

SEQ ID NO: 154 - protein, 427 aa, unidentified
  REGION 1..427: note = Description of Unknown: Low-affinity nerve growth factor receptor (LNGFR, TNFRSF16) sequence
MGAGATGRAMDGPRLLLLLLLGVSLGGAKEACPTGLYTHSGECCKACNLGEGVAQPCGANQTVCEPCLDSVTFSDVVSATEPCKPCTECVGLQSMSAPCVEADDAVCRCAYGYYQDETTGRCEACRVCEAGSGLVFSCQDKQNTVCEECPDGTYSDEANHVDPCLPCTVCEDTERQLRECTRWADAECEEIPGRWITRSTPPEGSDSTAPSTQEPEAPPEQDLIASTVAGVVTTVMGSSQPVVTRGTTDNLIPVYCSILAAVVVGLVAYIAFKRWNSCKQNKQGANSRPVNQTPPPEGEKLHSDSGISVDSQSLHDQQPHTQTASGQALKGDGGLYSSLPPAKREEVEKLLNGSAGDTWRHLAGELGYQPEHIDSFTHEACPVRALLASWATQDSATLDALLAALRRIQRADLVESLCSESTATSPV

SEQ ID NO: 155 - DNA, 666 bp, unidentified
  misc_feature 1..666: note = Description of Unknown: LNGFR Extracellular Domain (K29-N250) sequence
  source 1..666: mol_type = genomic DNA
aaggaggcatgccccacaggcctgtacacacacagcggtgagtgctgcaaagcctgcaacctgggcgagggtgtggcccagccttgtggagccaaccagaccgtgtgtgagccctgcctggacagcgtgacgttctccgacgtggtgagcgcgaccgagccgtgcaagccgtgcaccgagtgcgtggggctccagagcatgtcggcgccgtgcgtggaggccgacgacgccgtgtgccgctgcgcctacggctactaccaggatgagacgactgggcgctgcgaggcgtgccgcgtgtgcgaggcgggctcgggcctcgtgttctcctgccaggacaagcagaacaccgtgtgcgaggagtgccccgacggcacgtattccgacgaggccaaccacgtggacccgtgcctgccctgcaccgtgtgcgaggacaccgagcgccagctccgcgagtgcacacgctgggccgacgccgagtgcgaggagatccctggccgttggattacacggtccacacccccagagggctcggacagcacagcccccagcacccaggagcctgaggcacctccagaacaagacctcatagccagcacggtggcaggtgtggtgaccacagtgatgggcagctcccagcccgtggtgacccgaggcaccaccgacaac

SEQ ID NO: 156 - protein, 222 aa, unidentified
  REGION 1..222: note = Description of Unknown: LNGFR Extracellular Domain (K29-N250) sequence
KEACPTGLYTHSGECCKACNLGEGVAQPCGANQTVCEPCLDSVTFSDVVSATEPCKPCTECVGLQSMSAPCVEADDAVCRCAYGYYQDETTGRCEACRVCEAGSGLVFSCQDKQNTVCEECPDGTYSDEANHVDPCLPCTVCEDTERQLRECTRWADAECEEIPGRWITRSTPPEGSDSTAPSTQEPEAPPEQDLIASTVAGVVTTVMGSSQPVVTRGTTDN

SEQ ID NO: 157 - DNA, 558 bp, synthetic construct
  misc_feature 1..558: note = Description of Artificial Sequence: Synthetic polynucleotide
  source 1..558: mol_type = other DNA
gagccctgcctggacagcgtgacgttctccgacgtggtgagcgcgaccgagccgtgcaagccgtgcaccgagtgcgtggggctccagagcatgtcggcgccgtgcgtggaggccgacgacgccgtgtgccgctgcgcctacggctactaccaggatgagacgactgggcgctgcgaggcgtgccgcgtgtgcgaggcgggctcgggcctcgtgttctcctgccaggacaagcagaacaccgtgtgcgaggagtgccccgacggcacgtattccgacgaggccaaccacgtggacccgtgcctgccctgcaccgtgtgcgaggacaccgagcgccagctccgcgagtgcacacgctgggccgacgccgagtgcgaggagatccctggccgttggattacacggtccacacccccagagggctcggacagcacagcccccagcacccaggagcctgaggcacctccagaacaagacctcatagccagcacggtggcaggtgtggtgaccacagtgatgggcagctcccagcccgtggtgacccgaggcaccaccgacaac

SEQ ID NO: 158 - protein, 186 aa, synthetic construct
  REGION 1..186: note = Description of Artificial Sequence: Synthetic polypeptide
EPCLDSVTFSDVVSATEPCKPCTECVGLQSMSAPCVEADDAVCRCAYGYYQDETTGRCEACRVCEAGSGLVFSCQDKQNTVCEECPDGTYSDEANHVDPCLPCTVCEDTERQLRECTRWADAECEEIPGRWITRSTPPEGSDSTAPSTQEPEAPPEQDLIASTVAGVVTTVMGSSQPVVTRGTTDN

SEQ ID NO: 159 - DNA, 429 bp, synthetic construct
  misc_feature 1..429: note = Description of Artificial Sequence: Synthetic polynucleotide
  source 1..429: mol_type = other DNA
cgctgcgcctacggctactaccaggatgagacgactgggcgctgcgaggcgtgccgcgtgtgcgaggcgggctcgggcctcgtgttctcctgccaggacaagcagaacaccgtgtgcgaggagtgccccgacggcacgtattccgacgaggccaaccacgtggacccgtgcctgccctgcaccgtgtgcgaggacaccgagcgccagctccgcgagtgcacacgctgggccgacgccgagtgcgaggagatccctggccgttggattacacggtccacacccccagagggctcggacagcacagcccccagcacccaggagcctgaggcacctccagaacaagacctcatagccagcacggtggcaggtgtggtgaccacagtgatgggcagctcccagcccgtggtgacccgaggcaccaccgacaac

SEQ ID NO: 160 - protein, 143 aa, synthetic construct
  REGION 1..143: note = Description of Artificial Sequence: Synthetic polypeptide
RCAYGYYQDETTGRCEACRVCEAGSGLVFSCQDKQNTVCEECPDGTYSDEANHVDPCLPCTVCEDTERQLRECTRWADAECEEIPGRWITRSTPPEGSDSTAPSTQEPEAPPEQDLIASTVAGVVTTVMGSSQPVVTRGTTDN

SEQ ID NO: 161 - DNA, 732 bp, synthetic construct
  misc_feature 1..732: note = Description of Artificial Sequence: Synthetic polynucleotide
  source 1..732: mol_type = other DNA
aaggaggcatgccccacaggcctgtacacacacagcggtgagtgctgcaaagcctgcaacctgggcgagggtgtggcccagccttgtggagccaaccagaccgtgtgtgagccctgcctggacagcgtgacgttctccgacgtggtgagcgcgaccgagccgtgcaagccgtgcaccgagtgcgtggggctccagagcatgtcggcgccgtgcgtggaggccgacgacgccgtgtgccgctgcgcctacggctactaccaggatgagacgactgggcgctgcgaggcgtgccgcgtgtgcgaggcgggctcgggcctcgtgttctcctgccaggacaagcagaacaccgtgtgcgaggagtgccccgacggcacgtattccgacgaggccaaccacgtggacccgtgcctgccctgcaccgtgtgcgaggacaccgagcgccagctccgcgagtgcacacgctgggccgacgccgagtgcgaggagatccctggccgttggattacacggtccacacccccagagggctcggacagcacagcccccagcacccaggagcctgaggcacctccagaacaagacctcatagccagcacggtggcaggtgtggtgaccacagtgatgggcagctcccagcccgtggtgacccgaggcaccaccgacaacctcatccctgtctattgctccatcctggctgctgtggttgtgggccttgtggcctacatagccttc

SEQ ID NO: 162 - protein, 244 aa, synthetic construct
  REGION 1..244: note = Description of Artificial Sequence: Synthetic polypeptide
KEACPTGLYTHSGECCKACNLGEGVAQPCGANQTVCEPCLDSVTFSDVVSATEPCKPCTECVGLQSMSAPCVEADDAVCRCAYGYYQDETTGRCEACRVCEAGSGLVFSCQDKQNTVCEECPDGTYSDEANHVDPCLPCTVCEDTERQLRECTRWADAECEEIPGRWITRSTPPEGSDSTAPSTQEPEAPPEQDLIASTVAGVVTTVMGSSQPVVTRGTTDNLIPVYCSILAAVVVGLVAYIAF

SEQ ID NO: 163 - protein, 274 aa, synthetic construct
  REGION 1..274: note = Description of Artificial Sequence: Synthetic polypeptide
KEACPTGLYTHSGECCKACNLGEGVAQPCGANQTVCEPCLDSVTFSDVVSATEPCKPCTECVGLQSMSAPCVEADDAVCRCAYGYYQDETTGRCEACRVCEAGSGLVFSCQDKQNTVCEECPDGTYSDEANHVDPCLPCTVCEDTERQLRECTRWADAECEEIPGRWITRSTPPEGSDSTAPSTQEPEAPPEQDLIASTVAGVVTTVMGSSQPVVTRGTTDNGGGGSGGGGSGGGGSGGGGSFWVLVVVGGVLACYSLLVTVAFIIFWVRSKRS

SEQ ID NO: 164 - protein, 238 aa, synthetic construct
  REGION 1..238: note = Description of Artificial Sequence: Synthetic polypeptide
EPCLDSVTFSDVVSATEPCKPCTECVGLQSMSAPCVEADDAVCRCAYGYYQDETTGRCEACRVCEAGSGLVFSCQDKQNTVCEECPDGTYSDEANHVDPCLPCTVCEDTERQLRECTRWADAECEEIPGRWITRSTPPEGSDSTAPSTQEPEAPPEQDLIASTVAGVVTTVMGSSQPVVTRGTTDNGGGGSGGGGSGGGGSGGGGSFWVLVVVGGVLACYSLLVTVAFIIFWVRSKRS

SEQ ID NO: 165 - protein, 195 aa, synthetic construct
  REGION 1..195: note = Description of Artificial Sequence: Synthetic polypeptide
RCAYGYYQDETTGRCEACRVCEAGSGLVFSCQDKQNTVCEECPDGTYSDEANHVDPCLPCTVCEDTERQLRECTRWADAECEEIPGRWITRSTPPEGSDSTAPSTQEPEAPPEQDLIASTVAGVVTTVMGSSQPVVTRGTTDNGGGGSGGGGSGGGGSGGGGSFWVLVVVGGVLACYSLLVTVAFIIFWVRSKRS

SEQ ID NO: 166 - protein, 193 aa, synthetic construct
  REGION 1..193: note = Description of Artificial Sequence: Synthetic polypeptide
RCAYGYYQDETTGRCEACRVCEAGSGLVFSCQDKQNTVCEECPDGTYSDEANHVDPCLPCTVCEDTERQLRECTRWADAECEEIPGRWITRSTPPEGSDSTAPSTQEPEAPPEQDLIASTVAGVVTTVMGSSQPVVTRGTTDNGGGGSGGGGSGGGGSGGGGSEITLIIFGVMAGVIGTILLISYGIRRGGGS

SEQ ID NO: 167 - protein, 190 aa, synthetic construct
  REGION 1..190: note = Description of Artificial Sequence: Synthetic polypeptide
RCAYGYYQDETTGRCEACRVCEAGSGLVFSCQDKQNTVCEECPDGTYSDEANHVDPCLPCTVCEDTERQLRECTRWADAECEEIPGRWITRSTPPEGSDSTAPSTQEPEAPPEQDLIASTVAGVVTTVMGSSQPVVTRGTTDNGGGGSGGGGSGGGGSGGGGSITLIIFGVMAGVIGTILLALLIWGGGS

SEQ ID NO: 168 - protein, 190 aa, synthetic construct; identical to SEQ ID NO: 167
  REGION 1..190: note = Description of Artificial Sequence: Synthetic polypeptide

SEQ ID NO: 169 - DNA, 1332 bp, synthetic construct
  misc_feature 1..1332: note = Description of Artificial Sequence: Synthetic polynucleotide
  source 1..1332: mol_type = other DNA
atggcgctgcccgtgaccgccttgctcctgccgctggccttgctgctccacgccgccaggccggacatccagatgacacagactacatcctccctgtctgcctctctgggagacagagtcaccatcagttgcagggcaagtcaggacattagtaaatatttaaattggtatcagcagaaaccagatggaactgttaaactcctgatctaccatacatcaagattacactcaggagtcccatcaaggttcagtggcagtgggtctggaacagattattctctcaccattagcaatttggagcaggaagatattgccacttacttttgccaacagggtaatacgcttccgtacacgttcggaggggggaccaagctggagatcacaggtggcggtggctcgggcggtggtgggtcgggtggcggcggatctgaggtgaaactgcaggagtcaggacctggcctggtggcgccctcacagagcctgtccgtcacatgcactgtctcaggggtctcattacccgactatggtgtaagctggattcgccagcctccacgaaagggtctggagtggctgggagtaatatggggtagtgaaaccacatactataattcagctctcaaatccagactgaccatcatcaaggacaactccaagagccaagttttcttaaaaatgaacagtctgcaaactgatgacacagccatttactactgtgccaaacattattactacggtggtagctatgctatggactactggggccaaggaacctcagtcaccgtctcctcaaccacgacgccagcgccgcgaccaccaacaccggcgcccaccatcgcgtcgcagcccctgtccctgcgcccagaggcgtgtagaccggctgcaggtggagcagtgcacacgagggggctggacttcgcctgtgatatctacatctgggcgcccttggccgggacttgtggggtccttctcctgtcactggttatcaccctttactgccgcgtcaagttcagcaggagcgcagacgcccccgcgtacaagcagggccagaaccagctctataacgagctcaatctaggacgaagagaggagtacgatgttttggacaagagacgtggccgggaccctgagatggggggaaagccgagaaggaagaaccctcaggaaggcctgtacaatgaactgcagaaagataagatggcggaggcctacagtgagattgggatgaaaggcgagcgccggaggggcaaggggcacgatggcctttaccagggtctcagtacagccaccaaggacacctacgacgcccttcacatgcaggccctgccccctcgc

SEQ ID NO: 170 - protein, 444 aa, synthetic construct
  REGION 1..444: note = Description of Artificial Sequence: Synthetic polypeptide
MALPVTALLLPLALLLHAARPDIQMTQTTSSLSASLGDRVTISCRASQDISKYLNWYQQKPDGTVKLLIYHTSRLHSGVPSRFSGSGSGTDYSLTISNLEQEDIATYFCQQGNTLPYTFGGGTKLEITGGGGSGGGGSGGGGSEVKLQESGPGLVAPSQSLSVTCTVSGVSLPDYGVSWIRQPPRKGLEWLGVIWGSETTYYNSALKSRLTIIKDNSKSQVFLKMNSLQTDDTAIYYCAKHYYYGGSYAMDYWGQGTSVTVSSTTTPAPRPPTPAPTIASQPLSLRPEACRPAAGGAVHTRGLDFACDIYIWAPLAGTCGVLLLSLVITLYCRVKFSRSADAPAYKQGQNQLYNELNLGRREEYDVLDKRRGRDPEMGGKPRRKNPQEGLYNELQKDKMAEAYSEIGMKGERRRGKGHDGLYQGLSTATKDTYDALHMQALPPR

SEQ ID NO: 171 - DNA, 1467 bp, synthetic construct
  misc_feature 1..1467: note = Description of Artificial Sequence: Synthetic polynucleotide
  source 1..1467: mol_type = other DNA
atggccttaccagtgaccgccttgctcctgccgctggccttgctgctccacgccgccaggccggacatccagatgacacagactacatcctccctgtctgcctctctgggagacagagtcaccatcagttgcagggcaagtcaggacattagtaaatatttaaattggtatcagcagaaaccagatggaactgttaaactcctgatctaccatacatcaagattacactcaggagtcccatcaaggttcagtggcagtgggtctggaacagattattctctcaccattagcaacctggagcaagaagatattgccacttacttttgccaacagggtaatacgcttccgtacacgttcggaggggggaccaagctggagatcacaggcagcacctccggcagcggcaagcctggcagcggcgagggcagcaccaagggcgaggtgaaactgcaggagtcaggacctggcctggtggcgccctcacagagcctgtccgtcacatgcactgtctcaggggtctcattacccgactatggtgtaagctggattcgccagcctccacgaaagggtctggagtggctgggagtaatatggggtagtgaaaccacatactataattcagctctcaaatccagactgaccatcatcaaggacaactccaagagccaagttttcttaaaaatgaacagtctgcaaactgatgacacagccatttactactgtgccaaacattattactacggtggtagctatgctatggactactggggccaaggaacctcagtcaccgtctcctcaaccacgacgccagcgccgcgaccaccaacaccggcgcccaccatcgcgtcgcagcccctgtccctgcgcccagaggcgtgccggccagcggcggggggcgcagtgcacacgagggggctggacttcgcctgtgatatctacatctgggcgcccttggccgggacttgtggggtccttctcctgtcactggttatcaccctttactgcaaacggggcagaaagaaactcctgtatatattcaaacaaccatttatgagaccagtacaaactactcaagaggaagatggctgtagctgccgatttccagaagaagaagaaggaggatgtgaactgagagtgaagttcagcaggagcgcagacgcccccgcgtacaagcagggccagaaccagctctataacgagctcaatctaggacgaagagaggagtacgatgttttggacaagagacgtggccgggaccctgagatggggggaaagccgagaaggaagaaccctcaggaaggcctgtacaatgaactgcagaaagataagatggcggaggcctacagtgagattgggatgaaaggcgagcgccggaggggcaaggggcacgatggcctttaccagggtctcagtacagccaccaaggacacctacgacgcccttcacatgcaggccctgccccctcgc

SEQ ID NO: 172 - protein, 489 aa, synthetic construct
  REGION 1..489: note = Description of Artificial Sequence: Synthetic polypeptide
MALPVTALLLPLALLLHAARPDIQMTQTTSSLSASLGDRVTISCRASQDISKYLNWYQQKPDGTVKLLIYHTSRLHSGVPSRFSGSGSGTDYSLTISNLEQEDIATYFCQQGNTLPYTFGGGTKLEITGSTSGSGKPGSGEGSTKGEVKLQESGPGLVAPSQSLSVTCTVSGVSLPDYGVSWIRQPPRKGLEWLGVIWGSETTYYNSALKSRLTIIKDNSKSQVFLKMNSLQTDDTAIYYCAKHYYYGGSYAMDYWGQGTSVTVSSTTTPAPRPPTPAPTIASQPLSLRPEACRPAAGGAVHTRGLDFACDIYIWAPLAGTCGVLLLSLVITLYCKRGRKKLLYIFKQPFMRPVQTTQEEDGCSCRFPEEEEGGCELRVKFSRSADAPAYKQGQNQLYNELNLGRREEYDVLDKRRGRDPEMGGKPRRKNPQEGLYNELQKDKMAEAYSEIGMKGERRRGKGHDGLYQGLSTATKDTYDALHMQALPPR

SEQ ID NO: 173 - DNA, 1455 bp, synthetic construct
  misc_feature 1..1455: note = Description of Artificial Sequence: Synthetic polynucleotide
  source 1..1455: mol_type = other DNA
atggcgctgcccgtgaccgccttgctcctgccgctggccttgctgctccacgccgccaggccggacatccagatgacacagactacatcctccctgtctgcctctctgggagacagagtcaccatcagttgcagggcaagtcaggacattagtaaatatttaaattggtatcagcagaaaccagatggaactgttaaactcctgatctaccatacatcaagattacactcaggagtcccatcaaggttcagtggcagtgggtctggaacagattattctctcaccattagcaatttggagcaggaagatattgccacttacttttgccaacagggtaatacgcttccgtacacgttcggaggggggaccaagctggagatcacaggtggcggtggctcgggcggtggtgggtcgggtggcggcggatctgaggtgaaactgcaggagtcaggacctggcctggtggcgccctcacagagcctgtccgtcacatgcactgtctcaggggtctcattacccgactatggtgtaagctggattcgccagcctccacgaaagggtctggagtggctgggagtaatatggggtagtgaaaccacatactataattcagctctcaaatccagactgaccatcatcaaggacaactccaagagccaagttttcttaaaaatgaacagtctgcaaactgatgacacagccatttactactgtgccaaacattattactacggtggtagctatgctatggactactggggccaaggaacctcagtcaccgtctcctcaaccacgacgccagcgccgcgaccaccaacaccggcgcccaccatcgcgtcgcagcccctgtccctgcgcccagaggcgtgtagaccggctgcaggtggagcagtgcacacgagggggctggacttcgcctgtgatatctacatctgggcgcccttggccgggacttgtggggtccttctcctgtcactggttatcaccctttactgcaggagtaagaggagcaggctcctgcacagtgactacatgaacatgactccccgccgccccgggcccacccgcaagcattaccagccctatgccccaccacgcgacttcgcagcctatcgctcccgcgtcaagttcagcaggagcgcagacgcccccgcgtacaagcagggccagaaccagctctataacgagctcaatctaggacgaagagaggagtacgatgttttggacaagagacgtggccgggaccctgagatggggggaaagccgagaaggaagaaccctcaggaaggcctgtacaatgaactgcagaaagataagatggcggaggcctacagtgagattgggatgaaaggcgagcgccggaggggcaaggggcacgatggcctttaccagggtctcagtacagccaccaaggacacctacgacgcccttcacatgcaggccctgccccctcgc

SEQ ID NO: 174 - protein, 485 aa, synthetic construct
  REGION 1..485: note = Description of Artificial Sequence: Synthetic polypeptide
MALPVTALLLPLALLLHAARPDIQMTQTTSSLSASLGDRVTISCRASQDISKYLNWYQQKPDGTVKLLIYHTSRLHSGVPSRFSGSGSGTDYSLTISNLEQEDIATYFCQQGNTLPYTFGGGTKLEITGGGGSGGGGSGGGGSEVKLQESGPGLVAPSQSLSVTCTVSGVSLPDYGVSWIRQPPRKGLEWLGVIWGSETTYYNSALKSRLTIIKDNSKSQVFLKMNSLQTDDTAIYYCAKHYYYGGSYAMDYWGQGTSVTVSSTTTPAPRPPTPAPTIASQPLSLRPEACRPAAGGAVHTRGLDFACDIYIWAPLAGTCGVLLLSLVITLYCRSKRSRLLHSDYMNMTPRRPGPTRKHYQPYAPPRDFAAYRSRVKFSRSADAPAYKQGQNQLYNELNLGRREEYDVLDKRRGRDPEMGGKPRRKNPQEGLYNELQKDKMAEAYSEIGMKGERRRGKGHDGLYQGLSTATKDTYDALHMQALPPR

SEQ ID NO: 175 - DNA, 2031 bp, synthetic construct
  misc_feature 1..2031: note = Description of Artificial Sequence: Synthetic polynucleotide
  source 1..2031: mol_type = other DNA
atgctgctgctggtgaccagcctgctgctgtgtgagctgccccaccccgcctttctgctgatccccgacatccagatgacccagaccacctccagcctgagcgccagcctgggcgaccgggtgaccatcagctgccgggccagccaggacatcagcaagtacctgaactggtatcagcagaagcccgacggcaccgtcaagctgctgatctaccacaccagccggctgcacagcggcgtgcccagccggtttagcggcagcggctccggcaccgactacagcctgaccatctccaacctggagcaggaggacatcgccacctacttttgccagcagggcaacacactgccctacacctttggcggcggaacaaagctggagatcaccggcagcacctccggcagcggcaagcctggcagcggcgagggcagcaccaagggcgaggtgaagctgcaggagagcggccctggcctggtggcccccagccagagcctgagcgtgacctgtaccgtgtccggcgtgtccctgcccgactacggcgtgtcctggatccggcagccccctaggaagggcctggagtggctgggcgtgatctggggcagcgagaccacctactacaacagcgccctgaagagccggctgaccatcatcaaggacaacagcaagagccaggtgttcctgaagatgaacagcctgcagaccgacgacaccgccatctactactgtgccaagcactactactacggcggcagctacgccatggactactggggccagggcaccagcgtgaccgtgtccagcgagagcaagtacggccctccctgccccccttgccctgcccccgagttcctgggcggacccagcgtgttcctgttcccccccaagcccaaggacaccctgatgatcagccggacccccgaggtgacctgtgtggtggtggacgtgtcccaggaggaccccgaggtccagttcaactggtacgtggacggcgtggaggtgcacaacgccaagaccaagccccgggaggagcagttcaatagcacctaccgggtggtgtccgtgctgaccgtgctgcaccaggactggctgaacggcaaggaatacaagtgtaaggtgtccaacaagggcctgcccagcagcatcgagaaaaccatcagcaaggccaagggccagcctcgggagccccaggtgtacaccctgccccctagccaagaggagatgaccaagaatcaggtgtccctgacctgcctggtgaagggcttctaccccagcgacatcgccgtggagtgggagagcaacggccagcccgagaacaactacaagaccaccccccctgtgctggacagcgacggcagcttcttcctgtacagcaggctgaccgtggacaagagccggtggcaggagggcaacgtctttagctgctccgtgatgcacgaggccctgcacaaccactacacccagaagagcctgtccctgagcctgggcaagatgttctgggtgctggtcgtggtgggtggcgtgctggcctgctacagcctgctggtgacagtggccttcatcatcttttgggtgaggagcaagcggagcagaggcggccacagcgactacatgaacatgaccccccggaggcctggccccacccggaagcactaccagccctacgcccctcccagggacttcgccgcctaccggagccgggtgaagttcagccggagcgccgacgcccctgcctaccagcagggccagaaccagctgtacaacgagctgaacctgggccggagggaggagtacgacgtgctggacaagcggagaggccgggaccctgagatgggcggcaagccccggagaaagaaccctcaggagggcctgtataacgaactgcagaaagacaagatggccgaggcctacagcgagatcggcatgaagggcgagcggcggaggggcaagggccacgacggcctgtaccagggcctgagcaccgccaccaaggatacctacgacgccctgcacatgcaggccctgccccccaga

SEQ ID NO: 176 - protein, 677 aa, synthetic construct
  REGION 1..677: note = Description of Artificial Sequence: Synthetic polypeptide
MLLLVTSLLLCELPHPAFLLIPDIQMTQTTSSLSASLGDRVTISCRASQDISKYLNWYQQKPDGTVKLLIYHTSRLHSGVPSRFSGSGSGTDYSLTISNLEQEDIATYFCQQGNTLPYTFGGGTKLEITGSTSGSGKPGSGEGSTKGEVKLQESGPGLVAPSQSLSVTCTVSGVSLPDYGVSWIRQPPRKGLEWLGVIWGSETTYYNSALKSRLTIIKDNSKSQVFLKMNSLQTDDTAIYYCAKHYYYGGSYAMDYWGQGTSVTVSSESKYGPPCPPCPAPEFLGGPSVFLFPPKPKDTLMISRTPEVTCVVVDVSQEDPEVQFNWYVDGVEVHNAKTKPREEQFNSTYRVVSVLTVLHQDWLNGKEYKCKVSNKGLPSSIEKTISKAKGQPREPQVYTLPPSQEEMTKNQVSLTCLVKGFYPSDIAVEWESNGQPENNYKTTPPVLDSDGSFFLYSRLTVDKSRWQEGNVFSCSVMHEALHNHYTQKSLSLSLGKMFWVLVVVGGVLACYSLLVTVAFIIFWVRSKRSRGGHSDYMNMTPRRPGPTRKHYQPYAPPRDFAAYRSRVKFSRSADAPAYQQGQNQLYNELNLGRREEYDVLDKRRGRDPEMGGKPRRKNPQEGLYNELQKDKMAEAYSEIGMKGERRRGKGHDGLYQGLSTATKDTYDALHMQALPPR

SEQ ID NO: 177 - DNA, 1131 bp, synthetic construct
  misc_feature 1..1131: note = Description of Artificial Sequence: Synthetic polynucleotide
  source 1..1131: mol_type = other DNA
aactgggtgaatgtgatcagcgacctgaagaagatcgaggatctgatccagagcatgcacattgatgccaccctgtacacagaatctgatgtgcaccctagctgtaaagtgaccgccatgaagtgttttctgctggagctgcaggtgatttctctggaaagcggagatgcctctatccacgacacagtggagaatctgatcatcctggccaacaatagcctgagcagcaatggcaatgtgacagagtctggctgtaaggagtgtgaggagctggaggagaagaacatcaaggagtttctgcagagctttgtgcacatcgtgcagatgttcatcaatacaagctctggcggaggatctggaggaggcggatctggaggaggaggcagtggaggcggaggatctggcggaggatctctgcagattacatgccctcctccaatgtctgtggagcacgccgatatttgggtgaagtcctacagcctgtacagcagagagagatacatctgcaacagcggctttaagagaaaggccggcacctcttctctgacagagtgcgtgctgaataaggccacaaatgtggcccactggacaacacctagcctgaagtgcattagagatcctgccctggtccaccagaggcctgcccctccatctacagtgacaacagccggagtgacacctcagcctgaatctctgagcccttctggaaaagaacctgccgccagctctcctagctctaataataccgccgccacaacagccgccattgtgcctggatctcagctgatgcctagcaagtctcctagcacaggcacaacagagatcagcagccacgaatcttctcacggaacaccttctcagaccaccgccaagaattgggagctgacagcctctgcctctcaccagcctccaggagtgtatcctcagggccactctgatacaacagtggccatcagcacatctacagtgctgctgtgtggactgtctgccgtgtctctgctggcctgttacctgaagtctagacagacacctcctctggcctctgtggagatggaggccatggaagccctgcctgtgacatggggaacaagcagcagagatgaggacctggagaattgttctcaccacctg

SEQ ID NO: 178 - protein, 377 aa, synthetic construct
  REGION 1..377: note = Description of Artificial Sequence: Synthetic polypeptide
NWVNVISDLKKIEDLIQSMHIDATLYTESDVHPSCKVTAMKCFLLELQVISLESGDASIHDTVENLIILANNSLSSNGNVTESGCKECEELEEKNIKEFLQSFVHIVQMFINTSSGGGSGGGGSGGGGSGGGGSGGGSLQITCPPPMSVEHADIWVKSYSLYSRERYICNSGFKRKAGTSSLTECVLNKATNVAHWTTPSLKCIRDPALVHQRPAPPSTVTTAGVTPQPESLSPSGKEPAASSPSSNNTAATTAAIVPGSQLMPSKSPSTGTTEISSHESSHGTPSQTTAKNWELTASASHQPPGVYPQGHSDTTVAISTSTVLLCGLSAVSLLACYLKSRQTPPLASVEMEAMEALPVTWGTSSRDEDLENCSHHL

SEQ ID NO: 179 - protein, 841 aa, synthetic construct
  REGION 1..841: note = Description of Artificial Sequence: Synthetic polypeptide
DIQMTQTTSSLSASLGDRVTISCRASQDISKYLNWYQQKPDGTVKLLIYHTSRLHSGVPSRFSGSGSGTDYSLTISNLEQEDIATYFCQQGNTLPYTFGGGTKLEITGSTSGSGKPGSGEGSTKGEVKLQESGPGLVAPSQSLSVTCTVSGVSLPDYGVSWIRQPPRKGLEWLGVIWGSETTYYNSALKSRLTIIKDNSKSQVFLKMNSLQTDDTAIYYCAKHYYYGGSYAMDYWGQGTSVTVSSTTTPAPRPPTPAPTIASQPLSLRPEACRPAAGGAVHTRGLDFACDIYIWAPLAGTCGVLLLSLVITLYCKRGRKKLLYIFKQPFMRPVQTTQEEDGCSCRFPEEEEGGCELRVKFSRSADAPAYKQGQNQLYNELNLGRREEYDVLDKRRGRDPEMGGKPRRKNPQEGLYNELQKDKMAEAYSEIGMKGERRRGKGHDGLYQGLSTATKDTYDALHMQALPPREGRGSLLTCGDVEENPGPMRLPAQLLGLLMLWVPGSSGRKVCNGIGIGEFKDSLSINATNIKHFKNCTSISGDLHILPVAFRGDSFTHTPPLDPQELDILKTVKEITGFLLIQAWPENRTDLHAFENLEIIRGRTKQHGQFSLAVVSLNITSLGLRSLKEISDGDVIISGNKNLCYANTINWKKLFGTSGQKTKIISNRGENSCKATGQVCHALCSPEGCWGPEPRDCVSCRNVSRGRECVDKCNLLEGEPREFVENSECIQCHPECLPQAMNITCTGRGPDNCIQCAHYIDGPHCVKTCPAGVMGENNTLVWKYADAGHVCHLCHPNCTYGCTGPGLEGCPTNGPKIPSIATGMVGALLLLLVVALGIGLFM

SEQ ID NO: 180 - protein, 750 aa, synthetic construct
  REGION 1..750: note = Description of Artificial Sequence: Synthetic polypeptide
DIQMTQTTSSLSASLGDRVTISCRASQDISKYLNWYQQKPDGTVKLLIYHTSRLHSGVPSRFSGSGSGTDYSLTISNLEQEDIATYFCQQGNTLPYTFGGGTKLEITGSTSGSGKPGSGEGSTKGEVKLQESGPGLVAPSQSLSVTCTVSGVSLPDYGVSWIRQPPRKGLEWLGVIWGSETTYYNSALKSRLTIIKDNSKSQVFLKMNSLQTDDTAIYYCAKHYYYGGSYAMDYWGQGTSVTVSSTTTPAPRPPTPAPTIASQPLSLRPEACRPAAGGAVHTRGLDFACDIYIWAPLAGTCGVLLLSLVITLYCKRGRKKLLYIFKQPFMRPVQTTQEEDGCSCRFPEEEEGGCELRVKFSRSADAPAYKQGQNQLYNELNLGRREEYDVLDKRRGRDPEMGGKPRRKNPQEGLYNELQKDKMAEAYSEIGMKGERRRGKGHDGLYQGLSTATKDTYDALHMQALPPREGRGSLLTCGDVEENPGPMRLPAQLLGLLMLWVPGSSGRKVCNGIGIGEFKDSLSINATNIKHFKNCTSISGDLHILPVAFRGDSFTHTPPLDPQELDILKTVKEITGFLLIQAWPENRTDLHAFENLEIIRGRTKQHGQFSLAVVSLNITSLGLRSLKEISDGDVIISGNKNLCYANTINWKKLFGTSGQKTKIISNRGENSCKATGQVCHALCSPEGCWGPEPRDCVSGGGGSGGGGSGGGGSGGGGSFWVLVVVGGVLACYSLLVTVAFIIFWVRSKRS

SEQ ID NO: 181 - DNA, 2814 bp, synthetic construct
  misc_feature 1..2814: note = Description of Artificial Sequence: Synthetic polynucleotide
  source 1..2814: mol_type = other DNA
gacatccaaatgacacagacaaccagcagcctctctgccagtctgggagatcgtgtgaccatcagttgtagagcctcacaagatatttccaaatacctaaactggtatcagcaaaaaccagatggtacagtgaagttactgatctaccatactagccgtcttcattccggtgtgccttctcgctttagcgggtctggatcaggaacagattacagtctcaccatcagcaacctcgaacaagaagatatagctacctatttctgccagcagggtaacactttgccatataccttcggaggaggcacaaaactggagatcactggttctaccagtggaagcggcaagcctggctccggtgaaggaagtaccaaaggcgaagtgaagctgcaagagtcaggtccaggtttggtagctcccagccaatccctatctgttacctgtacagtgtctggtgtgtcacttccagattatggcgtgtcatggataaggcagcccccacgaaaaggcctggaatggttgggggtgatctggggatctgagaccacctactacaacagcgccctgaaaagtcggctcaccatcatcaaagacaactccaagtcacaagtgtttcttaagatgaactcacttcagaccgacgacacagccatatactactgtgctaaacattactactatggcggtagctatgccatggattactggggtcaaggtactagtgtgacagtatcatctgaatcaaagtatggcccaccctgccccccttgtcccgctcctgagttcctgggtggtccctccgtattcctgtttccacctaagccaaaagacactctcatgatcagcagaacacctgaggtgacatgcgtcgtagttgatgttagccaggaggaccccgaagtgcaatttaactggtacgtagacggtgtggaagtgcataacgcaaagaccaagccacgtgaagagcagtttaactccacctaccgagtggtgtctgtgctcacagtcttacatcaagattggctgaacggaaaagagtataaatgtaaagtatccaataagggccttccctctagcatcgaaaagactatctccaaagccaagggacagccacgcgaaccacaggtgtatactttacctccttctcaagaagagatgaccaagaaccaagtatctctgacgtgtttggtgaaggggttctacccctctgacatcgcagtggaatgggaatcaaacggtcaacctgagaacaattacaaaaccaccccacctgtgctggatagcgacggcagcttctttctgtatagcaggctcacagtggataaaagtcggtggcaggaaggaaacgtatttagttgcagtgtgatgcacgaggccctccataaccattatacccagaagtcactctcacttagtctgggtaagatgttctgggtgctcgtggtcgtaggtggagtgctggcttgctactccctcttagtgaccgtggcttttatcatcttctgggtacgttccaaaaggtcccgtggtggccattcagattacatgaatatgacccccagacgaccaggcccaacaaggaagcattatcaaccttacgcccctccccgagattttgcagcttatcgaagtagggtgaagttcagccggtctgctgacgctcctgcataccagcaaggtcagaatcagttatacaatgagctaaatctaggacgacgcgaagaatatgatgtgctggacaaacgacgtggcagggaccctgaaatgggtggcaagccaagaaggaagaacccacaagagggtctgtacaacgagttgcagaaagacaagatggcagaggcctactccgagatcggaatgaaaggagagaggcggaggggtaaaggacatgacggtctttaccagggcctgagcacagctactaaagatacctacgacgccctccacatgcaggctttgcccccacgagctaccaattttagtctgttgaaacaagctggagatgtcgaggaaaatccaggcccaatgcgacttcctgctcaactgctgggtctgctcatgctgtgggttcctggaagcagtggccgaaaggtctgcaacggcatcggtatcggcgaatttaaggatagtctatctatcaacgctaccaatattaagcattttaagaactgcacgtctatttccggcgacttgcacatcctccctgttgcatttcggggtgatagtttcacccataccccccctctcgatccacaagaactggacattcttaaaaccgttaaagaaataacaggttttctcctcatccaggcatggcccgagaataggacagatcttcacgcatttgaaaacctcgaaatcatcagagggaggaccaaacagcatggtcagtttagtctcgcagtggtgtctctgaacatcacttctttagggcttcgatcacttaaggaaatctctgacggtgatgtaatcatcagcggtaacaagaacctgtgctacgctaacacgatcaactggaagaagctgtttggcacaagcggccagaaaaccaagatcattagtaataggggcgagaatagctgtaaagcaaccgggcaagtgtgtcacgctctgtgttctcccgagggatgttggggacctgaaccaagagactgcgttagtggaggggggggctctggtggcggaggatctggcggaggcggaagcggaggcggggggagcttctgggtgctcgtggtcgtaggaggggtgctggcctgttactctctactcgtaactgttgctttcatcatattctgggtccgaagtaagcgtagc

SEQ ID NO: 182 - protein, 938 aa, synthetic construct
  REGION 1..938: note = Description of Artificial Sequence: Synthetic polypeptide
DIQMTQTTSSLSASLGDRVTISCRASQDISKYLNWYQQKPDGTVKLLIYHTSRLHSGVPSRFSGSGSGTDYSLTISNLEQEDIATYFCQQGNTLPYTFGGGTKLEITGSTSGSGKPGSGEGSTKGEVKLQESGPGLVAPSQSLSVTCTVSGVSLPDYGVSWIRQPPRKGLEWLGVIWGSETTYYNSALKSRLTIIKDNSKSQVFLKMNSLQTDDTAIYYCAKHYYYGGSYAMDYWGQGTSVTVSSESKYGPPCPPCPAPEFLGGPSVFLFPPKPKDTLMISRTPEVTCVVVDVSQEDPEVQFNWYVDGVEVHNAKTKPREEQFNSTYRVVSVLTVLHQDWLNGKEYKCKVSNKGLPSSIEKTISKAKGQPREPQVYTLPPSQEEMTKNQVSLTCLVKGFYPSDIAVEWESNGQPENNYKTTPPVLDSDGSFFLYSRLTVDKSRWQEGNVFSCSVMHEALHNHYTQKSLSLSLGKMFWVLVVVGGVLACYSLLVTVAFIIFWVRSKRSRGGHSDYMNMTPRRPGPTRKHYQPYAPPRDFAAYRSRVKFSRSADAPAYQQGQNQLYNELNLGRREEYDVLDKRRGRDPEMGGKPRRKNPQEGLYNELQKDKMAEAYSEIGMKGERRRGKGHDGLYQGLSTATKDTYDALHMQALPPRATNFSLLKQAGDVEENPGPMRLPAQLLGLLMLWVPGSSGRKVCNGIGIGEFKDSLSINATNIKHFKNCTSISGDLHILPVAFRGDSFTHTPPLDPQELDILKTVKEITGFLLIQAWPENRTDLHAFENLEIIRGRTKQHGQFSLAVVSLNITSLGLRSLKEISDGDVIISGNKNLCYANTINWKKLFGTSGQKTKIISNRGENSCKATGQVCHALCSPEGCWGPEPRDCVSGGGGSGGGGSGGGGSGGGGSFWVLVVVGGVLACYSLLVTVAFIIFWVRSKRS

SEQ ID NO: 183 - protein, 959 aa, synthetic construct
  REGION 1..959: note = Description of Artificial Sequence: Synthetic polypeptide
MRLPAQLLGLLMLWVPGSSGRKVCNGIGIGEFKDSLSINATNIKHFKNCTSISGDLHILPVAFRGDSFTHTPPLDPQELDILKTVKEITGFLLIQAWPENRTDLHAFENLEIIRGRTKQHGQFSLAVVSLNITSLGLRSLKEISDGDVIISGNKNLCYANTINWKKLFGTSGQKTKIISNRGENSCKATGQVCHALCSPEGCWGPEPRDCVSGGGGSGGGGSGGGGSGGGGSFWVLVVVGGVLACYSLLVTVAFIIFWVRSKRSATNFSLLKQAGDVEENPGPMALPVTALLLPLALLLHAARPDIQMTQTTSSLSASLGDRVTISCRASQDISKYLNWYQQKPDGTVKLLIYHTSRLHSGVPSRFSGSGSGTDYSLTISNLEQEDIATYFCQQGNTLPYTFGGGTKLEITGSTSGSGKPGSGEGSTKGEVKLQESGPGLVAPSQSLSVTCTVSGVSLPDYGVSWIRQPPRKGLEWLGVIWGSETTYYNSALKSRLTIIKDNSKSQVFLKMNSLQTDDTAIYYCAKHYYYGGSYAMDYWGQGTSVTVSSESKYGPPCPPCPAPEFLGGPSVFLFPPKPKDTLMISRTPEVTCVVVDVSQEDPEVQFNWYVDGVEVHNAKTKPREEQFNSTYRVVSVLTVLHQDWLNGKEYKCKVSNKGLPSSIEKTISKAKGQPREPQVYTLPPSQEEMTKNQVSLTCLVKGFYPSDIAVEWESNGQPENNYKTTPPVLDSDGSFFLYSRLTVDKSRWQEGNVFSCSVMHEALHNHYTQKSLSLSLGKMFWVLVVVGGVLACYSLLVTVAFIIFWVRSKRSRGGHSDYMNMTPRRPGPTRKHYQPYAPPRDFAAYRSRVKFSRSADAPAYQQGQNQLYNELNLGRREEYDVLDKRRGRDPEMGGKPRRKNPQEGLYNELQKDKMAEAYSEIGMKGERRRGKGHDGLYQGLSTATKDTYDALHMQALPPR

SEQ ID NO: 184 - protein, 763 aa, synthetic construct
  REGION 1..763: note = Description of Artificial Sequence: Synthetic polypeptide
DIQMTQTTSSLSASLGDRVTISCRASQDISKYLNWYQQKPDGTVKLLIYHTSRLHSGVPSRFSGSGSGTDYSLTISNLEQEDIATYFCQQGNTLPYTFGGGTKLEITGSTSGSGKPGSGEGSTKGEVKLQESGPGLVAPSQSLSVTCTVSGVSLPDYGVSWIRQPPRKGLEWLGVIWGSETTYYNSALKSRLTIIKDNSKSQVFLKMNSLQTDDTAIYYCAKHYYYGGSYAMDYWGQGTSVTVSSKPTTTPAPRPPTPAPTIASQPLSLRPEACRPAAGGAVHTRGLDFACDIYIWAPLAGTCGVLLLSLVITLYCNHRNRSKRSRGGHSDYMNMTPRRPGPTRKHYQPYAPPRDFAAYRSRVKFSRSADAPAYQQGQNQLYNELNLGRREEYDVLDKRRGRDPEMGGKPRRKNPQEGLYNELQKDKMAEAYSEIGMKGERRRGKGHDGLYQGLSTATKDTYDALHMQALPPRRAKRSGSGEGRGSLLTCGDVEENPGPMRLPAQLLGLLMLWVPGSSGRKVCNGIGIGEFKDSLSINATNIKHFKNCTSISGDLHILPVAFRGDSFTHTPPLDPQELDILKTVKEITGFLLIQAWPENRTDLHAFENLEIIRGRTKQHGQFSLAVVSLNITSLGLRSLKEISDGDVIISGNKNLCYANTINWKKLFGTSGQKTKIISNRGENSCKATGQVCHALCSPEGCWGPEPRDCVSGGGGSGGGGSGGGGSGGGGSFWVLVVVGGVLACYSLLVTVAFIIFWVRSKRS

SEQ ID NO: 185 - DNA, 2553 bp, synthetic construct
  misc_feature 1..2553: note = Description of Artificial Sequence: Synthetic polynucleotide
  source 1..2553: mol_type = other DNA
gacatacagatgactcagacaacaagtagcttgtccgcatccctgggcgatagagtgaccatcagttgtcgagcatcccaagatatatccaagtacttaaactggtatcagcagaagccagatggcaccgtcaagctgctaatctaccacacaagtaggctccacagcggagtgcctagccgattctctggttctggttctggcacagactattccctaaccatcagcaacctggagcaagaggacattgcaacatatttttgccagcagggcaacacactgccatatacctttggaggcgggaccaagctggaaatcaccggtagtacgagtggttctggaaaacctggttctggcgaaggtagtactaaaggagaggtgaaacttcaagagagtggccctggcttggtggccccttctcaaagtttgagcgtgacctgcacagtaagtggcgtcagcctgccagattacggagtcagttggattcgccagcctccaaggaagggccttgaatggctgggcgtaatctgggggtccgaaaccacctattacaactccgcacttaagagccgtttaaccatcatcaaagacaacagcaagagtcaggtctttctcaaaatgaatagtctgcaaacggacgacaccgctatctactattgtgccaagcactactactatggtggctcctacgctatggattactggggacaaggaacaagcgtgacagtgtcaagtactaccacacctgctccccgtcctccaacccccgctcctactattgccagtcaaccactgtctcttaggcccgaggcatgtaggccagcagcaggcggggctgtgcatacccgaggtctcgacttcgcctgcgacatatatatctgggcccctctggctggcacttgtggggtcctcctcctgagtctcgtgatcactctgtattgtaaacgtgggcgaaagaagctcctttacatcttcaagcaacccttcatgaggcctgtacagaccacgcaggaggaggacgggtgtagttgccgattccccgaagaggaagaaggcggttgcgagcttcgagtgaaattcagtaggagtgctgacgcaccagcatataagcagggccagaaccaattatacaacgagctgaacctcggacgaagggaagagtatgatgtgctggataagcgcagaggccgtgatccagaaatgggcggcaaacctcgtcggaaaaatccacaagaggggctatacaacgaattgcagaaagacaaaatggcagaggcctattctgaaatcggcatgaagggcgaacgacgaagaggtaagggtcatgacggcctgtatcaaggtctctctaccgccacaaaggacacttacgatgctttacacatgcaggctctccctcccagacaatgcaccaactacgctctattgaagttggcaggagatgtggaatccaaccccggtcctatgcgtctacctgcccagctgcttgggctcctgatgctgtgggtccccggcagcagtggtagaaaagtatgtaacggcataggtatcggtgaatttaaggactcactaagcatcaacgccacaaacatcaagcactttaagaactgtacctctattagcggagacttacacatcctgccagtcgcatttcgaggagacagtttcacccacactccacctctcgatcctcaggaattagacattcttaaaacagttaaggaaatcactggatttcttcttatccaggcctggccagaaaatagaacagacctgcacgctttcgagaaccttgaaataatacgaggcaggaccaaacagcatggccaatttagtttggctgtagtctccttgaacatcacttcccttggcctaaggtctttgaaggaaatcagtgacggagacgtgattatcagcgggaacaagaacctctgttacgcaaacacaatcaactggaagaagctctttggcaccagcggccagaagacaaagatcatttctaaccgaggagagaacagttgtaaggcaacaggacaagtgtgccacgctttgtgcagccccgagggatgttggggtcctgagccacgtgattgtgtctcttgccggaacgtcagcagaggtagagaatgtgtggataagtgcaacctcctggaaggggagcctcgtgagttcgtggagaactccgaatgtatccagtgtcatccagaatgcctgccccaggccatgaacataacatgtacaggacgcggcccagacaactgcatacagtgcgcccactacattgatggcccccattgcgtaaagacttgtcctgctggagtcatgggcgaaaataacaccctggtgtggaagtacgccgacgctggccatgtatgtcatctgtgtcatcctaattgcacctatggctgcactggccccggccttgaaggatgccccggcggtggaggaggaggctctttctgggtcctcgtggtggtgggaggcgtgctggcctgctattccttgctggtcacggtcgccttcattattttctgggtgagatctaaaagaagc

SEQ ID NO: 186 - protein, 851 aa, synthetic construct
  REGION 1..851: note = Description of Artificial Sequence: Synthetic polypeptide
DIQMTQTTSSLSASLGDRVTISCRASQDISKYLNWYQQKPDGTVKLLIYHTSRLHSGVPSRFSGSGSGTDYSLTISNLEQEDIATYFCQQGNTLPYTFGGGTKLEITGSTSGSGKPGSGEGSTKGEVKLQESGPGLVAPSQSLSVTCTVSGVSLPDYGVSWIRQPPRKGLEWLGVIWGSETTYYNSALKSRLTIIKDNSKSQVFLKMNSLQTDDTAIYYCAKHYYYGGSYAMDYWGQGTSVTVSSTTTPAPRPPTPAPTIASQPLSLRPEACRPAAGGAVHTRGLDFACDIYIWAPLAGTCGVLLLSLVITLYCKRGRKKLLYIFKQPFMRPVQTTQEEDGCSCRFPEEEEGGCELRVKFSRSADAPAYKQGQNQLYNELNLGRREEYDVLDKRRGRDPEMGGKPRRKNPQEGLYNELQKDKMAEAYSEIGMKGERRRGKGHDGLYQGLSTATKDTYDALHMQALPPRQCTNYALLKLAGDVESNPGPMRLPAQLLGLLMLWVPGSSGRKVCNGIGIGEFKDSLSINATNIKHFKNCTSISGDLHILPVAFRGDSFTHTPPLDPQELDILKTVKEITGFLLIQAWPENRTDLHAFENLEIIRGRTKQHGQFSLAVVSLNITSLGLRSLKEISDGDVIISGNKNLCYANTINWKKLFGTSGQKTKIISNRGENSCKATGQVCHALCSPEGCWGPEPRDCVSCRNVSRGRECVDKCNLLEGEPREFVENSECIQCHPECLPQAMNITCTGRGPDNCIQCAHYIDGPHCVKTCPAGVMGENNTLVWKYADAGHVCHLCHPNCTYGCTGPGLEGCPGGGGGGSFWVLVVVGGVLACYSLLVTVAFIIFWVRSKRS

SEQ ID NO: 187 - protein, 761 aa, synthetic construct
  REGION 1..761: note = Description of Artificial Sequence: Synthetic polypeptide
DIQMTQTTSSLSASLGDRVTISCRASQDISKYLNWYQQKPDGTVKLLIYHTSRLHSGVPSRFSGSGSGTDYSLTISNLEQEDIATYFCQQGNTLPYTFGGGTKLEITGSTSGSGKPGSGEGSTKGEVKLQESGPGLVAPSQSLSVTCTVSGVSLPDYGVSWIRQPPRKGLEWLGVIWGSETTYYNSALKSRLTIIKDNSKSQVFLKMNSLQTDDTAIYYCAKHYYYGGSYAMDYWGQGTSVTVSSKPTTTPAPRPPTPAPTIASQPLSLRPEACRPAAGGAVHTRGLDFACDIYIWAPLAGTCGVLLLSLVITLYCNHRNRSKRSRGGHSDYMNMTPRRPGPTRKHYQPYAPPRDFAAYRSRVKFSRSADAPAYQQGQNQLYNELNLGRREEYDVLDKRRGRDPEMGGKPRRKNPQEGLYNELQKDKMAEAYSEIGMKGERRRGKGHDGLYQGLSTATKDTYDALHMQALPPRRAKRSGSGEGRGSLLTCGDVEENPGPMRLPAQLLGLLMLWVPGSSGRKVCNGIGIGEFKDSLSINATNIKHFKNCTSISGDLHILPVAFRGDSFTHTPPLDPQELDILKTVKEITGFLLIQAWPENRTDLHAFENLEIIRGRTKQHGQFSLAVVSLNITSLGLRSLKEISDGDVIISGNKNLCYANTINWKKLFGTSGQKTKIISNRGENSCKATGQVCHALCSPEGCWGPEPRDCVSGGGGSGGGGSGGGGSGGGGSEITLIIFGVMAGVIGTILLISYGIRRGGGS

SEQ ID NO: 188 - protein, 750 aa, synthetic construct
  REGION 1..750: note = Description of Artificial Sequence: Synthetic polypeptide
DIQMTQTTSSLSASLGDRVTISCRASQDISKYLNWYQQKPDGTVKLLIYHTSRLHSGVPSRFSGSGSGTDYSLTISNLEQEDIATYFCQQGNTLPYTFGGGTKLEITGSTSGSGKPGSGEGSTKGEVKLQESGPGLVAPSQSLSVTCTVSGVSLPDYGVSWIRQPPRKGLEWLGVIWGSETTYYNSALKSRLTIIKDNSKSQVFLKMNSLQTDDTAIYYCAKHYYYGGSYAMDYWGQGTSVTVSSTTTPAPRPPTPAPTIASQPLSLRPEACRPAAGGAVHTRGLDFACDIYIWAPLAGTCGVLLLSLVITLYCKRGRKKLLYIFKQPFMRPVQTTQEEDGCSCRFPEEEEGGCELRVKFSRSADAPAYKQGQNQLYNELNLGRREEYDVLDKRRGRDPEMGGKPRRKNPQEGLYNELQKDKMAEAYSEIGMKGERRRGKGHDGLYQGLSTATKDTYDALHMQALPPRQCTNYALLKLAGDVESNPGPMRLPAQLLGLLMLWVPGSSGRKVCNGIGIGEFKDSLSINATNIKHFKNCTSISGDLHILPVAFRGDSFTHTPPLDPQELDILKTVKEITGFLLIQAWPENRTDLHAFENLEIIRGRTKQHGQFSLAVVSLNITSLGLRSLKEISDGDVIISGNKNLCYANTINWKKLFGTSGQKTKIISNRGENSCKATGQVCHALCSPEGCWGPEPRDCVSGGGGSGGGGSGGGGSGGGGSEITLIIFGVMAGVIGTILLISYGIRRGGGS

SEQ ID NO: 189 - protein, 758 aa, synthetic construct
  REGION 1..758: note = Description of Artificial Sequence: Synthetic polypeptide
DIQMTQTTSSLSASLGDRVTISCRASQDISKYLNWYQQKPDGTVKLLIYHTSRLHSGVPSRFSGSGSGTDYSLTISNLEQEDIATYFCQQGNTLPYTFGGGTKLEITGSTSGSGKPGSGEGSTKGEVKLQESGPGLVAPSQSLSVTCTVSGVSLPDYGVSWIRQPPRKGLEWLGVIWGSETTYYNSALKSRLTIIKDNSKSQVFLKMNSLQTDDTAIYYCAKHYYYGGSYAMDYWGQGTSVTVSSKPTTTPAPRPPTPAPTIASQPLSLRPEACRPAAGGAVHTRGLDFACDIYIWAPLAGTCGVLLLSLVITLYCNHRNRSKRSRGGHSDYMNMTPRRPGPTRKHYQPYAPPRDFAAYRSRVKFSRSADAPAYQQGQNQLYNELNLGRREEYDVLDKRRGRDPEMGGKPRRKNPQEGLYNELQKDKMAEAYSEIGMKGERRRGKGHDGLYQGLSTATKDTYDALHMQALPPRRAKRSGSGEGRGSLLTCGDVEENPGPMRLPAQLLGLLMLWVPGSSGRKVCNGIGIGEFKDSLSINATNIKHFKNCTSISGDLHILPVAFRGDSFTHTPPLDPQELDILKTVKEITGFLLIQAWPENRTDLHAFENLEIIRGRTKQHGQFSLAVVSLNITSLGLRSLKEISDGDVIISGNKNLCYANTINWKKLFGTSGQKTKIISNRGENSCKATGQVCHALCSPEGCWGPEPRDCVSGGGGSGGGGSGGGGSGGGGSITLIIFGVMAGVIGTILLISYGIGGGS

SEQ ID NO: 190 - protein, 747 aa, synthetic construct
  REGION 1..747: note = Description of Artificial Sequence: Synthetic polypeptide
DIQMTQTTSSLSASLGDRVTISCRASQDISKYLNWYQQKPDGTVKLLIYHTSRLHSGVPSRFSGSGSGTDYSLTISNLEQEDIATYFCQQGNTLPYTFGGGTKLEITGSTSGSGKPGSGEGSTKGEVKLQESGPGLVAPSQSLSVTCTVSGVSLPDYGVSWIRQPPRKGLEWLGVIWGSETTYYNSALKSRLTIIKDNSKSQVFLKMNSLQTDDTAIYYCAKHYYYGGSYAMDYWGQGTSVTVSSTTTPAPRPPTPAPTIASQPLSLRPEACRPAAGGAVHTRGLDFACDIYIWAPLAGTCGVLLLSLVITLYCKRGRKKLLYIFKQPFMRPVQTTQEEDGCSCRFPEEEEGGCELRVKFSRSADAPAYKQGQNQLYNELNLGRREEYDVLDKRRGRDPEMGGKPRRKNPQEGLYNELQKDKMAEAYSEIGMKGERRRGKGHDGLYQGLSTATKDTYDALHMQALPPRQCTNYALLKLAGDVESNPGPMRLPAQLLGLLMLWVPGSSGRKVCNGIGIGEFKDSLSINATNIKHFKNCTSISGDLHILPVAFRGDSFTHTPPLDPQELDILKTVKEITGFLLIQAWPENRTDLHAFENLEIIRGRTKQHGQFSLAVVSLNITSLGLRSLKEISDGDVIISGNKNLCYANTINWKKLFGTSGQKTKIISNRGENSCKATGQVCHALCSPEGCWGPEPRDCVSGGGGSGGGGSGGGGSGGGGSITLIIFGVMAGVIGTILLISYGIGGGS

SEQ ID NO: 191 - protein, 758 aa, synthetic construct
  REGION 1..758: note = Description of Artificial Sequence: Synthetic polypeptide
DIQMTQTTSSLSASLGDRVTISCRASQDISKYLNWYQQKPDGTVKLLIYHTSRLHSGVPSRFSGSGSGTDYSLTISNLEQEDIATYFCQQGNTLPYTFGGGTKLEITGSTSGSGKPGSGEGSTKGEVKLQESGPGLVAPSQSLSVTCTVSGVSLPDYGVSWIRQPPRKGLEWLGVIWGSETTYYNSALKSRLTIIKDNSKSQVFLKMNSLQTDDTAIYYCAKHYYYGGSYAMDYWGQGTSVTVSSKPTTTPAPRPPTPAPTIASQPLSLRPEACRPAAGGAVHTRGLDFACDIYIWAPLAGTCGVLLLSLVITLYCNHRNRSKRSRGGHSDYMNMTPRRPGPTRKHYQPYAPPRDFAAYRSRVKFSRSADAPAYQQGQNQLYNELNLGRREEYDVLDKRRGRDPEMGGKPRRKNPQEGLYNELQKDKMAEAYSEIGMKGERRRGKGHDGLYQGLSTATKDTYDALHMQALPPRRAKRSGSGEGRGSLLTCGDVEENPGPMRLPAQLLGLLMLWVPGSSGRKVCNGIGIGEFKDSLSINATNIKHFKNCTSISGDLHILPVAFRGDSFTHTPPLDPQELDILKTVKEITGFLLIQAWPENRTDLHAFENLEIIRGRTKQHGQFSLAVVSLNITSLGLRSLKEISDGDVIISGNKNLCYANTINWKKLFGTSGQKTKIISNRGENSCKATGQVCHALCSPEGCWGPEPRDCVSGGGGSGGGGSGGGGSGGGGSITLIIFGVMAGVIGTILLALLIWGGGS

SEQ ID NO: 192 - protein, 747 aa, synthetic construct
  REGION 1..747: note = Description of Artificial Sequence: Synthetic polypeptide
DIQMTQTTSSLSASLGDRVTISCRASQDISKYLNWYQQKPDGTVKLLIYHTSRLHSGVPSRFSGSGSGTDYSLTISNLEQEDIATYFCQQGNTLPYTFGGGTKLEITGSTSGSGKPGSGEGSTKGEVKLQESGPGLVAPSQSLSVTCTVSGVSLPDYGVSWIRQPPRKGLEWLGVIWGSETTYYNSALKSRLTIIKDNSKSQVFLKMNSLQTDDTAIYYCAKHYYYGGSYAMDYWGQGTSVTVSSTTTPAPRPPTPAPTIASQPLSLRPEACRPAAGGAVHTRGLDFACDIYIWAPLAGTCGVLLLSLVITLYCKRGRKKLLYIFKQPFMRPVQTTQEEDGCSCRFPEEEEGGCELRVKFSRSADAPAYKQGQNQLYNELNLGRREEYDVLDKRRGRDPEMGGKPRRKNPQEGLYNELQKDKMAEAYSEIGMKGERRRGKGHDGLYQGLSTATKDTYDALHMQALPPRQCTNYALLKLAGDVESNPGPMRLPAQLLGLLMLWVPGSSGRKVCNGIGIGEFKDSLSINATNIKHFKNCTSISGDLHILPVAFRGDSFTHTPPLDPQELDILKTVKEITGFLLIQAWPENRTDLHAFENLEIIRGRTKQHGQFSLAVVSLNITSLGLRSLKEISDGDVIISGNKNLCYANTINWKKLFGTSGQKTKIISNRGENSCKATGQVCHALCSPEGCWGPEPRDCVSGGGGSGGGGSGGGGSGGGGSITLIIFGVMAGVIGTILLALLIWGGGS

SEQ ID NO: 193 - protein, 666 aa, synthetic construct
  REGION 1..666: note = Description of Artificial Sequence: Synthetic polypeptide
NWVNVISDLKKIEDLIQSMHIDATLYTESDVHPSCKVTAMKCFLLELQVISLESGDASIHDTVENLIILANNSLSSNGNVTESGCKECEELEEKNIKEFLQSFVHIVQMFINTSSGGGSGGGGSGGGGSGGGGSGGGSLQITCPPPMSVEHADIWVKSYSLYSRERYICNSGFKRKAGTSSLTECVLNKATNVAHWTTPSLKCIRDPALVHQRPAPPSTVTTAGVTPQPESLSPSGKEPAASSPSSNNTAATTAAIVPGSQLMPSKSPSTGTTEISSHESSHGTPSQTTAKNWELTASASHQPPGVYPQGHSDTTVAISTSTVLLCGLSAVSLLACYLKSRQTPPLASVEMEAMEALPVTWGTSSRDEDLENCSHHLRAKRGSGEGRGSLLTCGDVEENPGPMRLPAQLLGLLMLWVPGSSGRKVCNGIGIGEFKDSLSINATNIKHFKNCTSISGDLHILPVAFRGDSFTHTPPLDPQELDILKTVKEITGFLLIQAWPENRTDLHAFENLEIIRGRTKQHGQFSLAVVSLNITSLGLRSLKEISDGDVIISGNKNLCYANTINWKKLFGTSGQKTKIISNRGENSCKATGQVCHALCSPEGCWGPEPRDCVSGGGGSGGGGSGGGGSGGGGSFWVLVVVGGVLACYSLLVTVAFIIFWVRSKRS

SEQ ID NO: 194 - protein, 971 aa, synthetic construct
  REGION 1..971: note = Description of Artificial Sequence: Synthetic polypeptide
DIQMTQTTSSLSASLGDRVTISCRASQDISKYLNWYQQKPDGTVKLLIYHTSRLHSGVPSRFSGSGSGTDYSLTISNLEQEDIATYFCQQGNTLPYTFGGGTKLEITGSTSGSGKPGSGEGSTKGEVKLQESGPGLVAPSQSLSVTCTVSGVSLPDYGVSWIRQPPRKGLEWLGVIWGSETTYYNSALKSRLTIIKDNSKSQVFLKMNSLQTDDTAIYYCAKHYYYGGSYAMDYWGQGTSVTVSSESKYGPPCPPCPAPEFLGGPSVFLFPPKPKDTLMISRTPEVTCVVVDVSQEDPEVQFNWYVDGVEVHNAKTKPREEQFNSTYRVVSVLTVLHQDWLNGKEYKCKVSNKGLPSSIEKTISKAKGQPREPQVYTLPPSQEEMTKNQVSLTCLVKGFYPSDIAVEWESNGQPENNYKTTPPVLDSDGSFFLYSRLTVDKSRWQEGNVFSCSVMHEALHNHYTQKSLSLSLGKMFWVLVVVGGVLACYSLLVTVAFIIFWVRSKRSRGGHSDYMNMTPRRPGPTRKHYQPYAPPRDFAAYRSRVKFSRSADAPAYQQGQNQLYNELNLGRREEYDVLDKRRGRDPEMGGKPRRKNPQEGLYNELQKDKMAEAYSEIGMKGERRRGKGHDGLYQGLSTATKDTYDALHMQALPPRATNFSLLKQAGDVEENPGPMTTPRNSVNGTFPAEPMKGPIAMQSGPKPLFRRMSSLVGPTQSFFMRESKTLGAVQIMNGLFHIALGGLLMIPAGIYAPICVTVWYPLWGGIMYIISGSLLAATEKNSRKCLVKGKMIMNSLSLFAAISGMILSIMDILNIKISHFLKMESLNFIRAHTPYINIYNCEPANPSEKNSPSTQYCYSIQSLFLGILSVMLIFAFFQELVIAGIVENEWKRTCSRPKSNIVLLSAEEKKEQTIEIKEEVVGLTETSSQPKNEEDIEIIPIQEEEEEETETNFPEPPQDQESSPIENDSSP

SEQ ID NO: 195 - protein, 937 aa, synthetic construct
  REGION 1..937: note = Description of Artificial Sequence: Synthetic polypeptide
DIQMTQTTSSLSASLGDRVTISCRASQDISKYLNWYQQKPDGTVKLLIYHTSRLHSGVPSRFSGSGSGTDYSLTISNLEQEDIATYFCQQGNTLPYTFGGGTKLEITGSTSGSGKPGSGEGSTKGEVKLQESGPGLVAPSQSLSVTCTVSGVSLPDYGVSWIRQPPRKGLEWLGVIWGSETTYYNSALKSRLTIIKDNSKSQVFLKMNSLQTDDTAIYYCAKHYYYGGSYAMDYWGQGTSVTVSSESKYGPPCPPCPAPEFLGGPSVFLFPPKPKDTLMISRTPEVTCVVVDVSQEDPEVQFNWYVDGVEVHNAKTKPREEQFNSTYRVVSVLTVLHQDWLNGKEYKCKVSNKGLPSSIEKTISKAKGQPREPQVYTLPPSQEEMTKNQVSLTCLVKGFYPSDIAVEWESNGQPENNYKTTPPVLDSDGSFFLYSRLTVDKSRWQEGNVFSCSVMHEALHNHYTQKSLSLSLGKMFWVLVVVGGVLACYSLLVTVAFIIFWVRSKRSRGGHSDYMNMTPRRPGPTRKHYQPYAPPRDFAAYRSRVKFSRSADAPAYQQGQNQLYNELNLGRREEYDVLDKRRGRDPEMGGKPRRKNPQEGLYNELQKDKMAEAYSEIGMKGERRRGKGHDGLYQGLSTATKDTYDALHMQALPPRATNFSLLKQAGDVEENPGPMTTPRNSVNGTFPAEPMKGPIAMQSGPKPLFRRMSSLVGPTQSFFMRESKTLGAVQIMNGLFHIALGGLLMIPAGIYAPICVTVWYPLWGGIMYIISGSLLAATEKNSRKCLVKGKMIMNSLSLFAAISGMILSIMDILNIKISHFLKMESLNFIRAHTPYINIYNCEPANPSEKNSPSTQYCYSIQSLFLGILSVMLIFAFFQELVIAGIVENEWKRTCSRPKSNIVLLSAEEKKEQTIEIKEEVVGLTETSSQPKNEEDIE

SEQ ID NO: 196 - protein, 888 aa, synthetic construct
  REGION 1..888: note = Description of Artificial Sequence: Synthetic polypeptide
DIQMTQTTSSLSASLGDRVTISCRASQDISKYLNWYQQKPDGTVKLLIYHTSRLHSGVPSRFSGSGSGTDYSLTISNLEQEDIATYFCQQGNTLPYTFGGGTKLEITGSTSGSGKPGSGEGSTKGEVKLQESGPGLVAPSQSLSVTCTVSGVSLPDYGVSWIRQPPRKGLEWLGVIWGSETTYYNSALKSRLTIIKDNSKSQVFLKMNSLQTDDTAIYYCAKHYYYGGSYAMDYWGQGTSVTVSSESKYGPPCPPCPAPEFLGGPSVFLFPPKPKDTLMISRTPEVTCVVVDVSQEDPEVQFNWYVDGVEVHNAKTKPREEQFNSTYRVVSVLTVLHQDWLNGKEYKCKVSNKGLPSSIEKTISKAKGQPREPQVYTLPPSQEEMTKNQVSLTCLVKGFYPSDIAVEWESNGQPENNYKTTPPVLDSDGSFFLYSRLTVDKSRWQEGNVFSCSVMHEALHNHYTQKSLSLSLGKMFWVLVVVGGVLACYSLLVTVAFIIFWVRSKRSRGGHSDYMNMTPRRPGPTRKHYQPYAPPRDFAAYRSRVKFSRSADAPAYQQGQNQLYNELNLGRREEYDVLDKRRGRDPEMGGKPRRKNPQEGLYNELQKDKMAEAYSEIGMKGERRRGKGHDGLYQGLSTATKDTYDALHMQALPPRATNFSLLKQAGDVEENPGPMTTPRNSVNGTFPAEPMKGPIAMQSGPKPLFRRMSSLVGPTQSFFMRESKTLGAVQIMNGLFHIALGGLLMIPAGIYAPICVTVWYPLWGGIMYIISGSLLAATEKNSRKCLVKGKMIMNSLSLFAAISGMILSIMDILNIKISHFLKMESLNFIRAHTPYINIYNCEPANPSEKNSPSTQYCYSIQSLFLGILSVMLIFAFFQELVIAGIVEN

SEQ ID NO: 197 - protein, 848 aa, synthetic construct
  REGION 1..848: note = Description of Artificial Sequence: Synthetic polypeptide
MKRFLFLLLTISLLVMVQIQTGLSGQNDTSQTSSPSGSTSGSGKPGSGEGSTKGGQNDTSQTSSPSGSTSGSGKPGSGEGSTKGGQNDTSQTSSPSGSTSGSGKPGSGEGSTKGGGGGSGGGGSKPFWVLVVVGGVLACYSLLVTVAFIIFWVATNFSLLKQAGDVEENPGPMALPVTALLLPLALLLHAARPDIQMTQTTSSLSASLGDRVTISCRASQDISKYLNWYQQKPDGTVKLLIYHTSRLHSGVPSRFSGSGSGTDYSLTISNLEQEDIATYFCQQGNTLPYTFGGGTKLEITGSTSGSGKPGSGEGSTKGEVKLQESGPGLVAPSQSLSVTCTVSGVSLPDYGVSWIRQPPRKGLEWLGVIWGSETTYYNSALKSRLTIIKDNSKSQVFLKMNSLQTDDTAIYYCAKHYYYGGSYAMDYWGQGTSVTVSSESKYGPPCPPCPAPEFLGGPSVFLFPPKPKDTLMISRTPEVTCVVVDVSQEDPEVQFNWYVDGVEVHNAKTKPREEQFNSTYRVVSVLTVLHQDWLNGKEYKCKVSNKGLPSSIEKTISKAKGQPREPQVYTLPPSQEEMTKNQVSLTCLVKGFYPSDIAVEWESNGQPENNYKTTPPVLDSDGSFFLYSRLTVDKSRWQEGNVFSCSVMHEALHNHYTQKSLSLSLGKMFWVLVVVGGVLACYSLLVTVAFIIFWVRSKRSRGGHSDYMNMTPRRPGPTRKHYQPYAPPRDFAAYRSRVKFSRSADAPAYQQGQNQLYNELNLGRREEYDVLDKRRGRDPEMGGKPRRKNPQEGLYNELQKDKMAEAYSEIGMKGERRRGKGHDGLYQGLSTATKDTYDALHMQALPPR

SEQ ID NO: 198 - protein, 910 aa, synthetic construct
  REGION 1..910: note = Description of Artificial Sequence: Synthetic polypeptide
MRLPAQLLGLLMLWVPGSSGRCAYGYYQDETTGRCEACRVCEAGSGLVFSCQDKQNTVCEECPDGTYSDEANHVDPCLPCTVCEDTERQLRECTRWADAECEEIPGRWITRSTPPEGSDSTAPSTQEPEAPPEQDLIASTVAGVVTTVMGSSQPVVTRGTTDNGGGGSGGGGSGGGGSGGGGSFWVLVVVGGVLACYSLLVTVAFIIFWVRSKRSATNFSLLKQAGDVEENPGPMALPVTALLLPLALLLHAARPDIQMTQTTSSLSASLGDRVTISCRASQDISKYLNWYQQKPDGTVKLLIYHTSRLHSGVPSRFSGSGSGTDYSLTISNLEQEDIATYFCQQGNTLPYTFGGGTKLEITGSTSGSGKPGSGEGSTKGEVKLQESGPGLVAPSQSLSVTCTVSGVSLPDYGVSWIRQPPRKGLEWLGVIWGSETTYYNSALKSRLTIIKDNSKSQVFLKMNSLQTDDTAIYYCAKHYYYGGSYAMDYWGQGTSVTVSSESKYGPPCPPCPAPEFLGGPSVFLFPPKPKDTLMISRTPEVTCVVVDVSQEDPEVQFNWYVDGVEVHNAKTKPREEQFNSTYRVVSVLTVLHQDWLNGKEYKCKVSNKGLPSSIEKTISKAKGQPREPQVYTLPPSQEEMTKNQVSLTCLVKGFYPSDIAVEWESNGQPENNYKTTPPVLDSDGSFFLYSRLTVDKSRWQEGNVFSCSVMHEALHNHYTQKSLSLSLGKMFWVLVVVGGVLACYSLLVTVAFIIFWVRSKRSRGGHSDYMNMTPRRPGPTRKHYQPYAPPRDFAAYRSRVKFSRSADAPAYQQGQNQLYNELNLGRREEYDVLDKRRGRDPEMGGKPRRKNPQEGLYNELQKDKMAEAYSEIGMKGERRRGKGHDGLYQGLSTATKDTYDALHMQALPPR

SEQ ID NO: 199 - DNA, 513 bp, synthetic construct
  misc_feature 1..513: note = Description of Artificial Sequence: Synthetic polynucleotide
  source 1..513: mol_type = other DNA
cgcaaagtgtgtaacggaataggtattggtgaatttaaagactcactctccataaatgctacgaatattaaacacttcaaaaactgcacctccatcagtggcgatctccacatcctgccggtggcatttaggggtgactccttcacacatactcctcctctggatccacaggaactggatattctgaaaaccgtaaaggaaatcacagggtttttgctgattcaggcttggcctgaaaacaggacggacctccatgcctttgagaacctagaaatcatacgcggcaggaccaagcaacatggtcagttttctcttgcagtcgtcagcctgaacataacatccttgggattacgctccctcaaggagataagtgatggagatgtgataatttcaggaaacaaaaatttgtgctatgcaaatacaataaactggaaaaaactgtttgggacctccggtcagaaaaccaaaattataagcaacagaggtgaaaacagctgcaaggccacaggccag

SEQ ID NO: 200 - protein, 171 aa, synthetic construct
  REGION 1..171: note = Description of Artificial Sequence: Synthetic polypeptide
RKVCNGIGIGEFKDSLSINATNIKHFKNCTSISGDLHILPVAFRGDSFTHTPPLDPQELDILKTVKEITGFLLIQAWPENRTDLHAFENLEIIRGRTKQHGQFSLAVVSLNITSLGLRSLKEISDGDVIISGNKNLCYANTINWKKLFGTSGQKTKIISNRGENSCKATGQ

SEQ ID NO: 201 - DNA, 423 bp, synthetic construct
  misc_feature 1..423: note = Description of Artificial Sequence: Synthetic polynucleotide
  source 1..423: mol_type = other DNA
gtctgccatgccttgtgctcccccgagggctgctggggcccggagcccagggactgcgtctcttgccggaatgtcagccgaggcagggaatgcgtggacaagtgcaaccttctggagggtgagccaagggagtttgtggagaactctgagtgcatacagtgccacccagagtgcctgcctcaggccatgaacatcacctgcacaggacggggaccagacaactgtatccagtgtgcccactacattgacggcccccactgcgtcaagacctgcccggcaggagtcatgggagaaaacaacaccctggtctggaagtacgcagacgccggccatgtgtgccacctgtgccatccaaactgcacctacggatgcactgggccaggtcttgaaggctgtccaacgaatgggcctaagatcccgtcc

SEQ ID NO: 202 - protein, 141 aa, synthetic construct
  REGION 1..141: note = Description of Artificial Sequence: Synthetic polypeptide
VCHALCSPEGCWGPEPRDCVSCRNVSRGRECVDKCNLLEGEPREFVENSECIQCHPECLPQAMNITCTGRGPDNCIQCAHYIDGPHCVKTCPAGVMGENNTLVWKYADAGHVCHLCHPNCTYGCTGPGLEGCPTNGPKIPS

SEQ ID NO: 203 - protein, 21 aa, synthetic construct
  REGION 1..21: note = Description of Artificial Sequence: Synthetic peptide
VCHALCSPEGCWGPEPRDCVS

SEQ ID NO: 204 - protein, 34 aa, synthetic construct
  REGION 1..34: note = Description of Artificial Sequence: Synthetic polypeptide
VCHALCSPEGCWGPEPRDCVSCRNVSRGRECVDK

SEQ ID NO: 205 - protein, 53 aa, synthetic construct
  REGION 1..53: note = Description of Artificial Sequence: Synthetic polypeptide
VCHALCSPEGCWGPEPRDCVSCRNVSRGRECVDKCNLLEGEPREFVENSECIQ

SEQ ID NO: 206 - protein, 77 aa, synthetic construct
  REGION 1..77: note = Description of Artificial Sequence: Synthetic polypeptide
VCHALCSPEGCWGPEPRDCVSCRNVSRGRECVDKCNLLEGEPREFVENSECIQCHPECLPQAMNITCTGRGPDNCIQ

SEQ ID NO: 207 - protein, 90 aa, synthetic construct
  REGION 1..90: note = Description of Artificial Sequence: Synthetic polypeptide
VCHALCSPEGCWGPEPRDCVSCRNVSRGRECVDKCNLLEGEPREFVENSECIQCHPECLPQAMNITCTGRGPDNCIQCAHYIDGPHCVKT

SEQ ID NO: 208 - protein, 115 aa, synthetic construct
  REGION 1..115: note = Description of Artificial Sequence: Synthetic polypeptide
VCHALCSPEGCWGPEPRDCVSCRNVSRGRECVDKCNLLEGEPREFVENSECIQCHPECLPQAMNITCTGRGPDNCIQCAHYIDGPHCVKTCPAGVMGENNTLVWKYADAGHVCHL

SEQ ID NO: 209 - protein, 133 aa, synthetic construct
  REGION 1..133: note = Description of Artificial Sequence: Synthetic polypeptide
VCHALCSPEGCWGPEPRDCVSCRNVSRGRECVDKCNLLEGEPREFVENSECIQCHPECLPQAMNITCTGRGPDNCIQCAHYIDGPHCVKTCPAGVMGENNTLVWKYADAGHVCHLCHPNCTYGCTGPGLEGCP

SEQ ID NO: 210 - protein, 312 aa, synthetic construct
  REGION 1..312: note = Description of Artificial Sequence: Synthetic polypeptide
RKVCNGIGIGEFKDSLSINATNIKHFKNCTSISGDLHILPVAFRGDSFTHTPPLDPQELDILKTVKEITGFLLIQAWPENRTDLHAFENLEIIRGRTKQHGQFSLAVVSLNITSLGLRSLKEISDGDVIISGNKNLCYANTINWKKLFGTSGQKTKIISNRGENSCKATGQVCHALCSPEGCWGPEPRDCVSCRNVSRGRECVDKCNLLEGEPREFVENSECIQCHPECLPQAMNITCTGRGPDNCIQCAHYIDGPHCVKTCPAGVMGENNTLVWKYADAGHVCHLCHPNCTYGCTGPGLEGCPTNGPKIPS

SEQ ID NO: 211 - protein, 192 aa, synthetic construct
  REGION 1..192: note = Description of Artificial Sequence: Synthetic polypeptide
RKVCNGIGIGEFKDSLSINATNIKHFKNCTSISGDLHILPVAFRGDSFTHTPPLDPQELDILKTVKEITGFLLIQAWPENRTDLHAFENLEIIRGRTKQHGQFSLAVVSLNITSLGLRSLKEISDGDVIISGNKNLCYANTINWKKLFGTSGQKTKIISNRGENSCKATGQVCHALCSPEGCWGPEPRDCVS

SEQ ID NO: 212 - protein, 205 aa, synthetic construct
  REGION 1..205: note = Description of Artificial Sequence: Synthetic polypeptide
RKVCNGIGIGEFKDSLSINATNIKHFKNCTSISGDLHILPVAFRGDSFTHTPPLDPQELDILKTVKEITGFLLIQAWPENRTDLHAFENLEIIRGRTKQHGQFSLAVVSLNITSLGLRSLKEISDGDVIISGNKNLCYANTINWKKLFGTSGQKTKIISNRGENSCKATGQVCHALCSPEGCWGPEPRDCVSCRNVSRGRECVDK

SEQ ID NO: 213 - protein, 224 aa, synthetic construct
  REGION 1..224: note = Description of Artificial Sequence: Synthetic polypeptide
RKVCNGIGIGEFKDSLSINATNIKHFKNCTSISGDLHILPVAFRGDSFTHTPPLDPQELDILKTVKEITGFLLIQAWPENRTDLHAFENLEIIRGRTKQHGQFSLAVVSLNITSLGLRSLKEISDGDVIISGNKNLCYANTINWKKLFGTSGQKTKIISNRGENSCKATGQVCHALCSPEGCWGPEPRDCVSCRNVSRGRECVDKCNLLEGEPREFVENSECIQ

SEQ ID NO: 214 - protein, 248 aa, synthetic construct
  REGION 1..248: note = Description of Artificial Sequence: Synthetic polypeptide
RKVCNGIGIGEFKDSLSINATNIKHFKNCTSISGDLHILPVAFRGDSFTHTPPLDPQELDILKTVKEITGFLLIQAWPENRTDLHAFENLEIIRGRTKQHGQFSLAVVSLNITSLGLRSLKEISDGDVIISGNKNLCYANTINWKKLFGTSGQKTKIISNRGENSCKATGQVCHALCSPEGCWGPEPRDCVSCRNVSRGRECVDKCNLLEGEPREFVENSECIQCHPECLPQAMNITCTGRGPDNCIQ

SEQ ID NO: 215 - protein, 261 aa, synthetic construct
  REGION 1..261: note = Description of Artificial Sequence: Synthetic polypeptide
RKVCNGIGIGEFKDSLSINATNIKHFKNCTSISGDLHILPVAFRGDSFTHTPPLDPQELDILKTVKEITGFLLIQAWPENRTDLHAFENLEIIRGRTKQHGQFSLAVVSLNITSLGLRSLKEISDGDVIISGNKNLCYANTINWKKLFGTSGQKTKIISNRGENSCKATGQVCHALCSPEGCWGPEPRDCVSCRNVSRGRECVDKCNLLEGEPREFVENSECIQCHPECLPQAMNITCTGRGPDNCIQCAHYIDGPHCVKT

SEQ ID NO: 216 - protein, 286 aa, synthetic construct
  REGION 1..286: note = Description of Artificial Sequence: Synthetic polypeptide
RKVCNGIGIGEFKDSLSINATNIKHFKNCTSISGDLHILPVAFRGDSFTHTPPLDPQELDILKTVKEITGFLLIQAWPENRTDLHAFENLEIIRGRTKQHGQFSLAVVSLNITSLGLRSLKEISDGDVIISGNKNLCYANTINWKKLFGTSGQKTKIISNRGENSCKATGQVCHALCSPEGCWGPEPRDCVSCRNVSRGRECVDKCNLLEGEPREFVENSECIQCHPECLPQAMNITCTGRGPDNCIQCAHYIDGPHCVKTCPAGVMGENNTLVWKYADAGHVCHL

SEQ ID NO: 217 - protein, 304 aa, synthetic construct
  REGION 1..304: note = Description of Artificial Sequence: Synthetic polypeptide
RKVCNGIGIGEFKDSLSINATNIKHFKNCTSISGDLHILPVAFRGDSFTHTPPLDPQELDILKTVKEITGFLLIQAWPENRTDLHAFENLEIIRGRTKQHGQFSLAVVSLNITSLGLRSLKEISDGDVIISGNKNLCYANTINWKKLFGTSGQKTKIISNRGENSCKATGQVCHALCSPEGCWGPEPRDCVSCRNVSRGRECVDKCNLLEGEPREFVENSECIQCHPECLPQAMNITCTGRGPDNCIQCAHYIDGPHCVKTCPAGVMGENNTLVWKYADAGHVCHLCHPNCTYGCTGPGLEGCP

SEQ ID NO: 218 - protein, 47 aa, synthetic construct
  REGION 1..47: note = Description of Artificial Sequence: Synthetic polypeptide
KISHFLKMESLNFIRAHTPYINIYNCEPANPSEKNSPSTQYCYSIQS

SEQ ID NO: 219 - protein, 29 aa, synthetic construct
  REGION 1..29: note = Description of Artificial Sequence: Synthetic peptide
PYINIYNCEPANPSEKNSPSTQYCYSIQS

SEQ ID NO: 220 - protein, 17 aa, synthetic construct
  REGION 1..17: note = Description of Artificial Sequence: Synthetic peptide
CEPANPSEKNSPSTQYC

SEQ ID NO: 221 - protein, 5 aa, synthetic construct
  REGION 1..5: note = Description of Artificial Sequence: Synthetic peptide
GGGGS

SEQ ID NO: 222 - protein, 25 aa, synthetic construct
  REGION 1..25: note = Description of Artificial Sequence: Synthetic peptide
  REGION 1..25: note = MISC_FEATURE - This sequence may encompass 1-5 "Gly Gly Gly Gly Ser" repeating units
GGGGSGGGGSGGGGSGGGGSGGGGS

SEQ ID NO: 223 - protein, 6 aa, synthetic construct
  REGION 1..6: note = Description of Artificial Sequence: Synthetic peptide
SGGGGS

SEQ ID NO: 224 - protein, 4 aa, synthetic construct
  REGION 1..4: note = Description of Artificial Sequence: Synthetic peptide
GGGS

SEQ ID NO: 225 - protein, 12 aa, synthetic construct
  REGION 1..12: note = Description of Artificial Sequence: Synthetic peptide
ESKYGPPCPPCP

SEQ ID NO: 226 - protein, 26 aa, synthetic construct
  REGION 1..26: note = Description of Artificial Sequence: Synthetic peptide
SGGGSGGGGSGGGGSGGGGSGGGSLQ

SEQ ID NO: 227 - protein, 25 aa, synthetic construct
  REGION 1..25: note = Description of Artificial Sequence: Synthetic peptide
RAKRGSGEGRGSLLTCGDVEENPGP

SEQ ID NO: 228 - protein, 26 aa, synthetic construct
  REGION 1..26: note = Description of Artificial Sequence: Synthetic peptide
RAKRSGSGEGRGSLLTCGDVEENPGP

SEQ ID NO: 229 - protein, 8 aa, synthetic construct
  REGION 1..8: note = Description of Artificial Sequence: Synthetic peptide
  MOD_RES 2: note = Val or Ile
  MOD_RES 4: note = Any amino acid
DXEXNPGP

SEQ ID NO: 230 - protein, 4 aa, synthetic construct
  REGION 1..4: note = Description of Artificial Sequence: Synthetic peptide
RAKR

SEQ ID NO: 231 - DNA, 12 bp, synthetic construct
  misc_feature 1..12: note = Description of Artificial Sequence: Synthetic oligonucleotide
  source 1..12: mol_type = other DNA
agagctaagagg

SEQ ID NO: 232 - DNA, 12 bp, synthetic construct
  misc_feature 1..12: note = Description of Artificial Sequence: Synthetic oligonucleotide
  source 1..12: mol_type = other DNA
cgtgcaaagcgt

SEQ ID NO: 233 - protein, 28 aa, synthetic construct
  REGION 1..28: note = Description of Artificial Sequence: Synthetic peptide
RAKRAPVKQTLNFDLLKLAGDVESNPGP

SEQ ID NO: 234 - DNA, 84 bp, synthetic construct
  misc_feature 1..84: note = Description of Artificial Sequence: Synthetic oligonucleotide
  source 1..84: mol_type = other DNA
agagccaagagggcaccggtgaaacagactttgaattttgaccttctgaagttggcaggagacgttgagtccaaccctgggccc

SEQ ID NO: 235 - protein, 22 aa, synthetic construct
  REGION 1..22: note = Description of Artificial Sequence: Synthetic peptide
GSGATNFSLLKQAGDVEENPGP

SEQ ID NO: 236 - DNA, 66 bp, synthetic construct
  misc_feature 1..66: note = Description of Artificial Sequence: Synthetic oligonucleotide
  source 1..66: mol_type = other DNA
ggaagcggagctactaacttcagcctgctgaagcaggctggagacgtggaggagaaccctggacct

SEQ ID NO: 237 - protein, 31 aa, synthetic construct
  REGION 1..31: note = Description of Artificial Sequence: Synthetic polypeptide
RAKRAPVKQGSGATNFSLLKQAGDVEENPGP

SEQ ID NO: 238 - DNA, 93 bp, synthetic construct
  misc_feature 1..93: note = Description of Artificial Sequence: Synthetic oligonucleotide
  source 1..93: mol_type = other DNA
cgtgcaaagcgtgcaccggtgaaacagggaagcggagctactaacttcagcctgctgaagcaggctggagacgtggaggagaaccctggacct

SEQ ID NO: 239 - protein, 10 aa, synthetic construct
  REGION 1..10: note = Description of Artificial Sequence: Synthetic peptide
  MOD_RES 1: note = Any amino acid
  MOD_RES 3: note = Any amino acid
  MOD_RES 5: note = Any amino acid
  MOD_RES 7: note = Any amino acid
  MOD_RES 9: note = Any amino acid
  REGION 1..10: note = MISC_FEATURE - This sequence may encompass 2-5 "Xaa Pro" repeating units
XPXPXPXPXP

SEQ ID NO: 240 - protein, 27 aa, synthetic construct
  REGION 1..27: note = Description of Artificial Sequence: Synthetic peptide
  REGION 2..26: note = MISC_FEATURE - This region may encompass 2-5 "Glu Ala Ala Ala Lys" repeating units
AEAAAKEAAAKEAAAKEAAAKEAAAKA